European Patent Specification EP 3 405 583 B1, published April 3, 2024. Title: COMPOSITIONS AND METHODS FOR SCREENING AND IDENTIFYING CLINICALLY AGGRESSIVE PROSTATE CANCER. Applicant: Dana-Farber Cancer Institute, Inc. The sequence listing filed with the application follows.

SEQUENCE LISTING (17 sequences)

SEQ ID NO: 1 - DNA, 2566 bp, Homo sapiens
agcctgacttcagcgctcccactctcggccgacacccctcatggccaaccgttacaccatggatctgactgccatctacgaggtgagtccccgccgcacggcatccccggtacctgcatgcctgagtccgagtccccacctctctagcgccgcaaactccagcccgggacgcttgcctcccttctccaactggggctccctagcgccgcgccctccagcctggggcccctgcctcccgctcagaccagcttggtgatttggaggtgaaaatggaacccgcgacacccggctcttcgctcaaacatgggtggggcggcccatgcaagtggaaagtcggagaacttttctcagaccgaggctgcctggaggcggaagtggcccccatacctggctcacccctagtcgttgctgagggcgtggttttgcgcggaggcgtctctggggctgaagtctcagggtggggggatccgacttctgtctctccagtccctgaccgtagagacagagaaccctaaaaccgaagcaatccggacttccaggtcaactttgcccggtttctccagttgtgaaactggagatcccgacgcgtgggtcatatccggggaggacaagagacccaaaattgggaaacagtggtgcgccctgacttcggggtccccctcttggtccagccggggaagccgggattcctgggtccctcgggataaggcctcggtggtgggtaaactcagaacctccaactctgggttcctggcatccggaacccaggggtttctgcgggcgggtggggctcaggcggggagcccacaaaccggcctggcaagctctagttccctgcagctggggtggggcgtcgccctgcattttcaggtgccttaaccgacccatttccgcagagcctcctgtcgctgagccctgacgtgcccgtgccatccgaccatggagggactgagtccagcccaggctggggctcctcgggaccctggagcctgagcccctccgactccagcccgtctggggtcacctcccgcctgcctggccgctccaccagcctagtggagggccgcagctgtggctgggtgcccccaccccctggcttcgcaccgctggctccccgcctgggccctgagctgtcaccctcacccacttcgcccactgcaacctccaccaccccctcgcgctacaagactgagctatgtcggaccttctcagagagtgggcgctgccgctacggggccaagtgccagtttgcccatggcctgggcgagctgcgccaggccaatcgccaccccaaatacaagacggaactctgtcacaagttctacctccagggccgctgcccctacggctctcgctgccacttcatccacaaccctagcgaagacctggcggccccgggccaccctcctgtgcttcgccagagcatcagcttctccggcctgccctctggccgccggacctcaccaccaccaccaggcctggccggcccttccctgtcctccagctccttctcgccctccagctccccaccaccacctggggaccttccactgtcaccctctgccttctctgctgcccctggcacccccctggctcgaagagaccccaccccagtctgttgcccctcctgccgaagggccactcctatcagcgtctgggggcccttgggtggcctggttcggaccccctctgtacagtccctgggatccgaccctgatgaatatgccagcagcggcagcagcctggggggctctgactctcccgtcttcgaggcgggagtttttgcaccaccccagcccgtggcagccccccggcgactccccatcttcaatcgcatctctgtttctgagtgacaaagtgactgcccggtcagatcagctggatctcagcggggagccacgtctcttgcactgtggtctctgcatggaccccagggctgtggggacttgggggacagtaatcaagtaatccccttttccagaatgcattaacccactcccctgacctcacgctggggcaggtccccaagtgtgcaagctcagtattcatgatggtgggggatggagtgtcttccgaggttcttgggggaaaaaaaattgtagcatatttaagggaggcaatgaaccctctcccccacctcttccctgcccaaatctgtctcctagaatcttatgtgctgtgaataataggccttcactgcccctccagtttttatagacctgaggttccagtgtctcctggtaactggaacctctcctgagggggaatcctggtgctcaaattaccctccaaaagcaagtagccaaagccgttgccaaaccccacccataaatcaatgggccctttatttatgacgactttatttattctaatatgattttatagtatttatatatattgggtcgtctgcttcccttgtatttttcttcctttttttgtaatattgaaaacgacgatataattattataagtagactataatatatttagtaatatatattattaccttaaaagtctatttttgtgttttgggcatttttaaataaacaatctgagtgtaagctgg

SEQ ID NO: 2 - DNA, 1752 bp, Homo sapiens
agcctgacttcagcgctcccactctcggccgacacccctcatggccaaccgttacaccatggatctgactgccatctacgagagcctcctgtcgctgagccctgacgtgcccgtgccatccgaccatggagggactgagtccagcccaggctggggctcctcgggaccctggagcctgagcccctccgactccagcccgtctggggtcacctcccgcctgcctggccgctccaccagcctagtggagggccgcagctgtggctgggtgcccccaccccctggcttcgcaccgctggctccccgcctgggccctgagctgtcaccctcacccacttcgcccactgcaacctccaccaccccctcgcgctacaagactgagctatgtcggaccttctcagagagtgggcgctgccgctacggggccaagtgccagtttgcccatggcctgggcgagctgcgccaggccaatcgccaccccaaatacaagacggaactctgtcacaagttctacctccagggccgctgcccctacggctctcgctgccacttcatccacaaccctagcgaagacctggcggccccgggccaccctcctgtgcttcgccagagcatcagcttctccggcctgccctctggccgccggacctcaccaccaccaccaggcctggccggcccttccctgtcctccagctccttctcgccctccagctccccaccaccacctggggaccttccactgtcaccctctgccttctctgctgcccctggcacccccctggctcgaagagaccccaccccagtctgttgcccctcctgccgaagggccactcctatcagcgtctgggggcccttgggtggcctggttcggaccccctctgtacagtccctgggatccgaccctgatgaatatgccagcagcggcagcagcctggggggctctgactctcccgtcttcgaggcgggagtttttgcaccaccccagcccgtggcagccccccggcgactccccatcttcaatcgcatctctgtttctgagtgacaaagtgactgcccggtcagatcagctggatctcagcggggagccacgtctcttgcactgtggtctctgcatggaccccagggctgtggggacttgggggacagtaatcaagtaatccccttttccagaatgcattaacccactcccctgacctcacgctggggcaggtccccaagtgtgcaagctcagtattcatgatggtgggggatggagtgtcttccgaggttcttgggggaaaaaaaattgtagcatatttaagggaggcaatgaaccctctcccccacctcttccctgcccaaatctgtctcctagaatcttatgtgctgtgaataataggccttcactgcccctccagtttttatagacctgaggttccagtgtctcctggtaactggaacctctcctgagggggaatcctggtgctcaaattaccctccaaaagcaagtagccaaagccgttgccaaaccccacccataaatcaatgggccctttatttatgacgactttatttattctaatatgattttatagtatttatatatattgggtcgtctgcttcccttgtatttttcttcctttttttgtaatattgaaaacgacgatataattattataagtagactataatatatttagtaatatatattattaccttaaaagtctatttttgtgttttgggcatttttaaataaacaatctgagtgtaagctgg

SEQ ID NO: 3 - protein, 332 aa, Homo sapiens
MANRYTMDLTAIYESLLSLSPDVPVPSDHGGTESSPGWGSSGPWSLSPSDSSPSGVTSRLPGRSTSLVEGRSCGWVPPPPGFAPLAPRLGPELSPSPTSPTATSTTPSRYKTELCRTFSESGRCRYGAKCQFAHGLGELRQANRHPKYKTELCHKFYLQGRCPYGSRCHFIHNPSEDLAAPGHPPVLRQSISFSGLPSGRRTSPPPPGLAGPSLSSSSFSPSSSPPPPGDLPLSPSAFSAAPGTPLARRDPTPVCCPSCRRATPISVWGPLGGLVRTPSVQSLGSDPDEYASSGSSLGGSDSPVFEAGVFAPPQPVAAPRRLPIFNRISVSE

SEQ ID NO: 4 - DNA, 199051 bp, Homo sapiens
acacatacatatgccactcacatccgacgtgtgtggttgctcagtagggaaatgcttacagctgcctctagaagcaagtccgctcgctgcatggagagggaaacatgagcatgcagcaggactagctgtcacctcccgcccgcctgcccagagagggccagagcgtcggggaggcaagatgatccaccagcggttccatcctacacttgggtgagttctcagccacttgctgtggcctgtgggagaggagggactcattcaggctcctacttcctgagttggtgccagacatctggtggtgtttccccactgtgaacactcctcaactggggcagggaggacctccacatgccccagaagaggaatgagtgactcccggtctccaagttgacctggaggtgctggttttagtgcaacattcaaaccagcatgatttctacttatgaaattgttctgggtagatgcttcctggtgtgtaagtacatggcccctcccctcttcctactgtcgtcagagagcttacctgacagcaactaagcttttatttttcctgaattatttcagtacttcaaagtgtgggccgtcacttattctttatggtggattagaatcatttacgtccttttcagcctctttggacatgagtcctgactggcgagaaatggtgactgaggattggattctgtgcgtgtcctatccctgtagtcattaggatcatctccaaggggctgaggacaagtgacagcacactgtgttctccctgtccatagtgagccgcccaagagctccacccttacttttctctatgtttattctttcacttagcccattcattcatttcttccttcattcattcattcaattgcctttcttccaccaaggacttgaggcaaattttttatcttgctgaaattttttcaaaatgaagaccatctgtaatcataaaggggacaatcgttctgaaagggttatacataattctaagctatgcagagatcggccaccaatcttttccctttgcttgtgttgagaagtgagagtaggcgctctagtcatttaaactcctgcatggggagtccctccttcccctgcccagaagctggtttcccacccagcatggggtgtgaagagcaattgtccatgacagaatactgggaatctgccaaatagttttcttctttgtttctgttttcttccaagcttggttactttcgaggacattcctggttctaagaatgcggaaagtggagttggtggaaaagaaaggatgtgaaatcagtgtttagctagcgctccaccatttcttgttaatcggttagtttatttaacagctatttagtggctgtcactttgtacgtcaccacttaaacaagatagctgggcacggtggtgtatgcctatagtcccggctatgcaggaggctaaggcgggaggattgctggagcccaggaggtcgaggctgcagtgagctatgattgcaccactgcactgcagcttgggtgacagagtgagatcctgtctcaagaagaagaagaagaagaagaagaagacgatgactaggaagatataaaagcagaggtgtaggagaggacaggctgtaagggtcacatgatgtaattcccggtgcctcttcctctacacgtaaataaggggaaagagctatcttgaatggctgtggtaaggattagattgaatagcaaacatttaagcatctggcagagaaggggtatccgaagtagtcagtgtcctgcctccctcctccaggcctcactgtgactgagctggctgctgacaacctgagtctttatctcatgacctgagagctttctccaagccacacagggacaactgtaattgcccaaagggcagacgaaaattcccagaaatgaactcctcaaaggctgtaaatattccagctccctcagtcttgagtggaataatctacacggaatcaagctccagttgcccacagtggcggggcccttcatggcttctctccttccctggatactccttcactccccatcaatgcttcctgggatcatttcttaaactacatgtcctcgaactctgcattggggtctacttctgggggaacccaagctaagaccaccggccacctactactgtaggtacttaaagagtttagtcgtctgttttccaatgatcagctccatctccatttgaccttagactctgagttttgatttcccacatatccattcaagggttgtagtgggggaagatcctcctcctcctcttctggatttggcttggagaaagggcacaggcacagcatggagagcaccttaggcttgacatgtctccatgcaaacccgcacagcacgaagatgcgtcctactgcaaatgaccttcactttgtcctgcttatctgtcaccttcacaactcatttgatgaaaatttctgaagtgtggaacacaaataggagaattttatatagcacaagatacatagatagagcatgaaatcacattgaacctgatcttaaagctactctaactcttggctccttactgttttaacaagagaaagtcgatctgaggctaggagccatcaacaggcactggtagctagctacaaattaatagcatggctttattttcctgtatttgctttttatggttaccttatattaaaccacaacggcctgttttttttttaatttgtaggaatggtataaacatttcttttaaaatataaatctttaagttttaaaaaagtgaatttattattactattattatttttgagacaaagtctcactctgtcacccaggctagagtgcagtgtggctcactgcaacttctgcctcccaggttcaagtgattctcttgcctcagcctcccaagtagctgggattgcaggtgcccaccatcacacctggctaatttttgtgtttttagtagagatggggtttcaccatgttggccaagctggtctcgaactcctgacctcaggtgacccgcccaccttagcctcccaaagtgctgggattacaggcatgagccactgcgcccggcccaaaagtgagttaatttaaagaaaaaaacgttgctgacagtcctgacagcacacagaatatggcaaaccctggaaaatggggtttgattaagagaagactaggaaagccccactagaacgcaggctcctcaagggcatggctgcatctcccagtgccttccacccagggcctgcctggcctgtgccactgggctggaattgtatggattttggatatcccaggaagcaggggtccaagctgcccttgttagctacaggcttttttggtcttcaaaatatacaacttcactttgcccacagtggctcccaaacgtcccagcagtgatgcagggtagtatagacacctaaaaatgggtacaacacaagctccattgtatggtagttccaccctaagtaagaatccatgaggctccgatgtaactcagcaatgtgagctgaggggacgggtggaggtatttcttcatctgcattccttttcacttttgcttcagattagaagctctggttcgtgaaggtctgtaattcacttaactagaggtcaatgaatgataaatttttttgaacagctacaaaaccctctactttccaaggaaagtgatacatgagggtgaataatttagataaatttagcttgaaaaaatttttaaatattgtaacattttatactacaaaaaagtatatataaggtatccatatattctaaataatcataggaataaaaacataaatacacatccacctgttaccccactacccaaccctgaaagcctgctgtgtgcccctaaacaattgtatccttctctcccaatgcccactgggttggtctatgtttgtgtggctataaatacctgaggctgggtaatctgcaaagaaaaaaggtttaattggctcatggttctgcaggctgtataggaagcatggtgctggcatctgcttctggtgaggcctctggaagcttacagtcatggtgaaagatgaagggggagccagcatcacatggcaagagtgggagcaagaaagctgggaggtgccacactcttttaaacaatcagatcttttttttgagacagaatctcactctgtcacccaggctggagtgcagtggtgcaatcttggcttgccgcaacctccacttcctgggttcaagtgattctcctgcctcagcctcctgagtagctgggattacacgtgcatgccaccacacccagcaaaattttgtatttttagcagagatggagttttgtcatgttggccaggctggtcttgagctcctgacctcaggtgatccacccacctcagcctcccaaagtgctggggttacaggcatgagccactgcgcctggcctaaacaaccagatctcatgtaaactaattgaagaagaactcactcatcaccagatagatggtgttaattcattcataagggatccacccgcatgctccaatacctcccactagatcccacctccaaaattggggatcacatttcaacatgagacttggaggggacaaatgtttaaaccatatcattctgcccctggcttcccaaatctgatgtccttctcacattgcaaaatacaatcatcttctcccagtagtctcccgaagtctgaattgattccagcatcaagtacaaagtcgtgtctcatctaagactcaaatctgtccacctatgagactctaaagtcaaaacaagttagttacttccaaggtacaatgatggtacagatattgggcaaacattaccattccaaaagggagaaattggccaaaagaaagggtataggggccccacacaaatctgaaacctagcagggtagtcattaaatcttaaaggtccaaaatacaatctcctttgactccaagtcctacatttagggcacactgttataacagtggactcctaaggccttgagcagctctggccctgtggctttgcaggatgcagcccacatggctgctctcatgggtttaagttgagtgcttgttgcttttccagttaaagggtgcaagctgccagtgaatctgctattctgggttctagagggtggcagccccctttccgcagctccactaggtagtgccctggtggggactctgtgtaggagctccaaccccacatttcccctggcattttcctagtagagtttttctgtggggcctctgcctctgcagtaggcttctgcctgagcacccaggctttcccatacatcctctggaatctaggtggaagccaccaagccttcttcacacttgcgttctgagcatctgcagacttaaccccatgtggcaatcaccaaggcttatggcttgtgtcctccagaactgtggccagagctgtacctgggcccctttgagctgaggctgaagccagagtctgaagctcagcagggcagtagggccctgggcctggcccctgaaaccattcttttctcctaagcctctgggcctttgatgggaggggctgtcctcaagatttttgaaatgcctttggagggtttttgccttgtcttggatattggcttccttttagttatgctcatctctctagcaagtgaatgtttcacaacctgcttggattctttctctaccacagagccaggctgcaaattttacaaacttttacactctgtttcccttttaaatataaatttcaatgttaagtcacttctttgctcccatatctgatttaggttgctggaagtagccaagtcacctcttgaatgctttgctgcttagaaatttcctctactaggtagcctgggtcatcactcttaagttcaaacttccacagatccctagagcatacagtgcaaccaagttctttgttagggcataataagaatgaccccattccatttcccaaaaactttctcatttccatctgagacctcatcagccagaacttcactgtccatatctgtatcagtattttggtcacaaccatttaaccagtctctaagaagttccaaactttccctcatcttcctgtctttttctgagtcctttaaactcttccagcctctcccttaccccgttccaaagtcacttccacattttcagttatctttatagcaatgctccacttctcagtaccaattttcaattttctgtgttagtccgttttgcatcactataaagaaatacccaaggctgggtaatttataaagaaaaaaagtggggaccgggcacggtggctcacgccagtaatcccagcactttgggaggccgagacgggcggatcacgaggtcaggagatcgagaccaccctggctaacacagtgaaagcccgtctctactaaaaatacaaaaaattagctgggtgtggtgacgggcgcctgtagtcccagctactcaggaggctaaggcaggagaatggcatgaacccgggaggcggagcttgcagtgagccgagatcacgccactgcactccagcctgagtgatagagtgagactccgtctcaaaaaaaagaaagaaaaaagaaaaaagggttgattgacttatggttctgcagggtatacagaaagcatggtgctggcatctgcttcgggtgaggcctcaggaaggttacaatcatggcggaaggaggagccagcatatgacatggcaagagagagagaaaaggacagaagggagaggtcccagagtcctttaaacaaccagatcttgggtgcgttaactgagtgaaaactcactcaccatcaaagggacagcactaagccactcatgagggatctgcccccataatccaatacctcctactaggccccacctctaacactgtggatcacatttcagcgtgagatttggaggagacaaacatccaaattatatcacctaccacaaaaggaactattgtcttaaaattttgttagtcattcccttactttactttttgattggcctcctaggtctaagtgtatgcatagacatatatgcataggtatatatacaatttgcatatagtcaatttctgcctgtttgggaactgtaagtaaatataatcatacataagcattcttccaagacttgctctagggtcaacatgatatttctgagtgttatccatgttgatgccaagagatgttgataattcattttcacagctgtatagtatcctattgcatgaatgtatgacagtctatcatttctatcagttggcagtgctaagtcattgacaaaaatgatggttcagagttaggatttcaagaaggcacaattgccaccaaatttatccctgtttcatgcacaaactacttgagcagagaagtgaaaattttgcctcaagttagaagcaggttttagctaggggacatcaaaggagggaaggggtcttaaatgggagaggaagaaagggctaaagtgactccccaagattaaaaaataaaaacaaaaagaaaaaaaagaatcttcctggacagacaatttgtgactgggctagcccatgctgattgtgggcaaattaaggctttcactctcactgtcacttcccctccagataagcccttggggaaaagttctatatgaatacttaatttacaaaagtattgttccccagaccagcagattgggttccatgaaggtccatcactttgcttgatcctgaagagaaccaaatttcatatagtgctcatctataagcttcctattgatgtattttttatattcacctttttctatagcatatgcgactatgcagctaccacacagttatcaaatagtagtgtccatgaacctttagtaacctttgactagtttccatgactctgaaattccccacccacagcttcacttgtaaagagtggaaatatttagaggaagtgagactatcagcagctcagcctcaccatgggaagcattttctcctcaaagcacagtagtatgctggtgccttctgtcacactatcaggacatggctttagcaagtacagtgtcctctcagcacctgttcctcatgcaggtgctttgcatcatataatcgtcgaaacattaaggaagtaatgctctttgtcactccaccggagtggagaagttaaagtcaagagtgtacttcaggggttgtatcactggtttggctttagtagttgtgaggtcttgatgggtgagagtgatccctggcaaatgacatatattgattgattcattgagtgagcaaaggagtaaggtgggtgtattagggttctccagacaaacagaaccaatggaatgtgtgtgtgtatatatatacatatatatatagagagagagagagagagagagatttattttatgaagttggttcacacaattatggagactggcaagtccaaaatcagcaaggcaggctggcaagctggagatcagggaagaactgacattgctacttgagtccgaaggcactctgctagctgaattccttcttgctctgtggatgtcgctcttttttctattaaggccttcaactgattggaggcccacctacattatggaaggtcatttgttttgctcaaagcctactcatttaaatgttaatcttttaaagaagatagctttgcagtgacatccagaagaatgtttgatcaatatctaggtaccttggcttagccaagttaacacgtaaaattaaccatctcagatactgtatccatttcagaaaataatttagtagatattaatatttattgaacatctgttaaggactctgtatgggccaggcaccatattaggtgctggggattcagcaggaaagccagccagacaaaatccctattttcaagaagcttacatatggaagggtggaggtttgagtaattaaaacactcgcagtagttttcatgccttcaagaagcactgcagatacaactcaagtcaatcaaatccattctcccatatacatatggtattggggtatagtgaaaagaggaacagaggttctgacttcctggactttgtcttctactgaggacctcaggtctaaattatatgatgaccatagacacattttaacaattatatacaacatgttattcattatgtagctttcaaaagcacatataattcagttataaaggatgatgaaaattaacaaattgcatacaattgtattaaaaataaagtgacaaaggtattttgtacatgattatttcattttcttcatgagttttttttttttaatttttatggcaaaacagttcaaggaaccacttaacgaaggtgtttgatttcaaaagaattgatttgggaagacagaactgcttgatgatgtctgtttctttgttagctttaagtaactggtttactcaattggcctcttccttcattgtgttttggagtttttttgactgaagcaaagacaagcattaaaaataaagacattggtttatgttgtttagaactgagaatccatttaaaaaaaatgaattggagtatctatgccagattgctcttacatgatatatgtggccatgggcagaggagggttgcattcttaatttatgccctgaaagaatatcaggcttatttctcaaaaggaaaaatacaaatggcaagcaggtatatgaataggtgctcaacatcactgatcctcagagaaatgcaaatcaaaactacaatgagatatcatttcaccacagttaaaatggcttatatgcaaaagtcaggcaataacaaattctactgaggatgtgaagaaaagggaaccctcatatactgttagtgggaatgtaaattagtataaccactgtggagaacagtttggaggttcctcaaaaaactaaaaatagagctgtcatatgatccagcaatcccactcacatatacccaaaagaaaggaaatcaatatattaaagacatatctgcagtcctgtgtttattgcagcactcttcacaagtgccaagatttggaagaaacctaagtgtccatcaacaaataaatggataaaggaaatgtggtacatatacacaatggagtactattcacccataaaaaagaatgagatccagtcatttgcagcaacatggatggaactagtggtcattatgttaagtgaaataaaccaggcacagaaagacaaatttcacatgttctcacttacttgtgggagctaaaaattaaaataattgaactcataaagacagacaatagagggatggttaccaggggctgggaagggtagcgttgtgggtgggggggattatggggggcaggtaggggagatagataatgagtacaagtcatagaaagaatgagtaagacctagtatttgctagcacaacaggatgaccgtagtcgaaaataatttaattgtacattaaaaaataactaaaatattgtaattggattgtttgtaacacagaggataaatgcttgaggtgatggagaccccatgtaccctgatgtgattattacacattgcatgcctgtatcaaaacatctcatataacccataaatatatacacctactatgtatccactgaatttttttaaaaagaaaaaaaacagcctttaattagaatatttgcatgtcacaggctagggctaataatccaattaaagttttaggtaagggctggaggacacagggatgtgtagcacacgttgatgtacctcaaagaggggaattcttctaagaaagcgtcatcacgatttctcacctgttatctacaaccttcaacccattgctctaaaaaatcttacatttgagttgaagaaagaacaaatacgtttgtaaaacaaaaatcacatttaaaaaatagctaaatatgttgctaagtgaaagaagccaatctgaaaaagctgtatattgtatgattctaactagaacgttctggaaaagataaaactagggtaccagtaaaaagatcaggggttcccagggactgcaaggagggagggatgaataggtgaggcatggaagatttgagggcagtgaaagtcctctgcgtgatacgatagtggtagaagcgtgtcactgtgcatttgcccaatcccatagaatgtacaccaccaggtgcgaaccctactgtcaactatagacttggggtcataatgatgtgtcaatgcaggtttattgattgtagcaaatgtgccagtctgtggagggaggtcgacagtgggagagcctgtgtgcatgtgggagcaggaggtatatgggaaatctctgtacctttttctcaattttgctgtgaacccaaaagtgctctaaaaaatagtctttttttaaaaggagctaagtggcctctttgatgttcccccagaaggccaagaaagtgcccaacaccggacgtttgcactgacagtccctctgcctggaaggaccttctgggagatccctgccaggctccgtccccttcctcattcagctctgggccacaagtcacccaatccgccagccctccctcacatgccatgcaaaatggccacggggtcacctctgtcaccctccccgttgtcacctgtcctcaacaccacccgacgccgtgcagactgacgtactggcttatggtctgtttctgcctctgaaccgttggctccgtgggtgggtgaaggacgttattttgtcccctgctgtgttcttggcacatgggaggtgctggagggacatctgctgaaggaacgagtgagtgagccagtgagtggatcatccagtgagcgtgagggacgggtgctaccaggcagggaaagaagctctctgtaagcagggaagcctgctcagaagtgaagctggtatggcccttgcaaaacgggaaggacacagaaaagcatgaggagattgtgaggggaagaaaaggcggcttgaggagagccttgtgcacctagtgggtcggtgagggaaccatttggactggaatgcaggtcttgggaggacaggggtgggagccgtcctccagccgtgtgtgcgtgctgtaggcaaaggcagacttttcctcaggaaagcaaatttggatccgctccagcatttgaataacagcctgattgaaaaacaaagctctactctacatagcagagcaaagaatggttttggtcagagcatttttcaaagacaatgttcctcacttcttgcttcagcataggaaaacgtcagcagagcttcggtgcagcgttttactctaagcaggcctgtgattcaggggctggcctccttgggttcccacaagcatgatttagcagagagatgtgtctatttcatcattaaacgaaatgttccttagggaaaagactctttatatacctcagttgacatccctaatgatattccctgaatacccagttagagaagtgttagcctcttctatgtcatactttctatctgctgagtaatttctttcttaattgcacagaagagccacttggcccaacactccctatttgagttcgacctagcagagatttctttcttttgaggctatgtgaaatgcagttgagcatgatattgaaaacatgaacacaatccaaaagtccatcagtagggtccttattacaatttggcaatccacactttggaatactgtgctactggtgaaaaagaagaaagaggatatacacaaagatatgaaaagatgtgaatcaaatacaaagcaacaaatgcaaaagaacatacagtacaagcccatttttatctatctcattgtagaataaaagtctagcaaaatatagactcccaaatatttttaaatgttttgggattgggtttataagacaggttcactttctgcagtagacattgtctgtctttagatatttaaaaatgagtttacgttgctttgtgattgaaaactggctcaaattttaaaaactctgtgtgtgtacacgtgcacaatcactcatgcatgccaggttgtgtagtacacaggagcaatggttggagaaatggggagttcctaataaaatttaacagtaggaatgtgtttttaagattattttacttaaaaataataattcttctcccctcgtcaggcttatcttttgaccatttttgttttggcttgttttcttgttttgttaatttgttaataaataattgataaaaataaatggcaaagcaaaaaaaaagttctaagcaatgtaagaaagtcatggcatactctctaaggagattctttctctgcagcatgggaacattcacaaagcaactatcaagcaacataagttggggaaatgatcatcagggttcaggaaatggacagattcaagaaggttggagtgcttaagagagaaccaactgcctgagttcaaatccaacctgtaccacccacctgccatgtgctattgagcaaattactttacttttctgtttctctgtttctcatctgcacaaaggaggtaataagagccctacctcaccggtggttttgaaggttttatgagtcaatggatgattttgaatgttacatgagtcaacacacacacagcacctaaagtggtatctgacacattaagtgctcaatacatattagctagtgggaggaagaggaggagagggaatgagttttcataaaagagaagggatgtaaagaatgagtagggtttgacagaaaaaagaattccagaagatcaagaaaaaaacaaaacccaaaggcttataggatacatgaaatgatccagttaaattcaccccaacctctgtaaagaaagccgaaatgatatttcatgactagatgataaacataagcagatatgtacaagcactcaaatgaaatagaaggagggttttttaaagttagctttcctttattattctgtagacccttctgtgtgtcagtcatcagtcaacaaattcgtatggagctacgtggtggtgtagctcccaccagcatggaactttttccaagtgggtttaaagttggaaaaccatggcgatcatttgttttattgtgtgttgattagtagcgtatccaagagttgtggtagttacttcggtgtgactcattcaggaatagaagaaagattcattgtattactcttaaaatataaacaattcttaatttttctgtgctaatgaagaaccacaggaataaatatagttgatagattaaattatgtttattttattttatctgtaaattaagcaaatcttcattgttttgcctttttgaaacttttctccatctgtttgggtttctgggtaccccccagccctggtgtcttcttcccagcttgcaaacagccatcagggcccaagggcaaggggagaagccactgagggccagactgcgcacagtagcttccaagcaggccctgggtaattgagttgcttgaccttggcaagcacagaaccagcctcatccacgaaaacacgaaaaacacatgtgactaggtgctgagactgatgcttttgatcaccagccctgaccacactgaagagcccttttaagaaccaaggtccagtctcatacaatcccgagagttcagacaaaaaggccaaaattccatagctctgccggacttatttgcaaggggtgctgtgtagaaggtgccgaaatggctagtagctaggtttaagcaattacagtcactagttggttcaaagggatgccattcactcctggaatcctgctgtcaatgattgagctagggagtttggtctccagggaagagttaaacattagacaggaaccattacaaaactttccactaaaaataagttccttgtaagagaagttgagagacttgctaattgcagcttactctaaacctaatgacagtctgtatcatttgcaaagaaagcacaggatgtgtgaatgatggtgagggaagtggggagtcttggcagatagatctgactctgatagatgcagttggtcctctagactagtgatccattttggagtaaactgcattgggagactgatcaaatttcctttctccaggattcttaccaacagtaaagactgataaaacacatttgtgctgctgtgtttttcaaaagctcggccatataataactttaacagactccctaaatttcaaacatttccttgatgtaggatgatcacaatagaaaggaatgttattctcatccagccatcggtaagcttttgtcttccttaatcccagaaactaaatcactggctacctcagaggctctgacctaaatcttaattgatgcccactgcactttcagaccactgtgtgtgattttaaccagacaaaccaaggaggaaggattaatgaagaaagcctaatattttgaccaatcatagagtccactgcagtgccctttccattttaattgagctttatacggttctcctctcgaggtaaccctcctttcttaatgttcagtacagcaaaaactaatctaggttttctttttaatgtttgatttatctcttcaatcttggtgctaggtaacaacattggatcaaaatattaacagccaagatttagatattattttacaattaacacagcacattgactcatattatttcactttcacagtggtcctggggcatgtttattgtatctcccactctacagatagtgaaactgaggagatcacggtgggaaagatgacgtaactcacatgaagttgggcaactgatcagatgacacagctaggactgaagcctgggtcccctaagtcatttgcttagagctcattcaatgacgaggcaactccttgctgtgcatcctttcagcacacgttgttggtgtgaagacgctggttttcatcagactaaaatgcatcttacttcaagataggcagtttctgttttggtttccacctctcatacattgcttttaaagtgccaacctctaatggctatcccatgagaaaatctactgtaagtatgaagtgaccctttggtactaccagtttttcatcctaaatcccttttctttcttctttcttttcctttctctctttctttcttttttctttctttcttcctttctttttcttttttctttcttcttttatttctctctctctctgtcttgctccccctttctttctttcttcatttctttctttctttctctctgtctttctcctttctttctttctctttctttctttctttccttccttccttccttccttccttctttctcagactctcactctgtcacccacgcacaatctcggctcactgcaacctctgcctcccaggttcaagtgattctcctgcttcagcctgctgagtagctggggttacaggcacatgccaccacacccggttactttttgtagttttaatagagactgggtttcaccttgttggtcaggctggtctcaaactcctgacctcatgatctgcccaccttggcctcccaaagtgctgggattacaggtgtgagccaccacgcccagcctctttctttttttgactgtgtctcttgctctgtcactcaggctggagtgcagtagcacaatctcggctcacggcaacctctgcctcctgggctcaagtgattctccagcctcagccccccgagtagttgggtctacagatgcatgccatcacatccacctaatttttgtatttttagtagagacagggtttcaccatgttggccaggctagtcttgaattcctgagctcaaagtgatccgcccacctcggcctcccaaagtgctgggattacaggcgtgagccactgcgcccggccccattttattttctttcttctttttcttggcatttgttatgatcaagccttttttttaagtactgaatatccatggactccttccagttttacctcatcaaaatgtgcttgcagggaaggatttggtcttgttgatttcaattaatgtaactccaagccaccactcttctgctattcaccttttaatctatatttcttactatacataagaagctttgcttctctacttatttcaaggagtgtagggtgaagatgaggtttttaaatcacggtatctttcttcagtcctttcctccaaattctacacgtagatgtactgtgcttcagccaacttatctctaactaggacattcagatctactaactaagctatgacttattataggcaggcggtcagcaggaagagctgtttttttttgaaagtaggacaagaataggtctatggaatgttggggtcacttggtttcctcaatggaaagaaacgggatgtttctgcattaactagaacacttgaaaggtagggaggggtgagggtgattgagaaatgatttcaacaaacagaacattaagtactctgtttgtcagacagcgtgttcccatctggggggtgagtggcagaaaacatagtcgccatcatgagaagagctcccctaaatctgcccacccacctccaactcttgctccagtcagtttttctgaatgcccagcctgctacactgaccctcaccgctcttaccccggtgccagggtgagagaggccagggatcaggtaaggaaagaggagaggaaatgcagaggctccatttggcttataaaggaactgtaccataatagttattattgtttaaaaaaatagcatgacatccattctatttctctccctcttcttcaaagatatttcagcctcagggactttctgcttgttagtgggatggcgaaaaatgcatgatagatttctagttagtaggtagaagggacgggagattacatcctaatacagtagagtaactatgttttattgagcacttaatatgtactgagtgaacacacctgctttgattcacaaccacttaatgagggaactttggagcctccttaagggttacaagcaaaagctgtggagtcagcttgcctgggttcaaatcctagttgtgccatgtacctgctgtgtggccttggtatagttacttaacctctccatgaatcagcttcctcaccttaaaatggagataattataatgtcacacacctttggggggaattcccaaggccacccccaggttcaatgactcattaggaggacccacaggattcatcatagagacatgcccacagctaagttctattacctcaaagacaaatcagaatcagcaaaggggaaagcaacagaagaaaccagacatgagctaccaagagtcctctcctaggggagtcacacaggacatacttaactcctccagcaacgagttatgacaggtatgaaatgttgtctactagggaagctcagtagatacttagtgccagagttttgatttggagctggtcacttagacaccctctgtctggcatgtacacaaattccagactcccagaaggaaagcaggtgttcagcataaaccatgttgtttgcacacacagttaagtcacagtgagccactcatatcacggaccagcaggaacccctcacatgttcccagatgccagccaagggccagccttgcaagcaggattgagacagcagtctcagacctgctatgtgaactctttactgcttgctaccttttgattgttgtgagattacataaggtaatatatatatctgttgcttacaacagtgcctaatttgtgggaagccctacagatttttttagcccttactattatgcagaaaaaaaaatactcaggtttagaatgactacacagtcaaaatggaacaaactggaatctgaattcacatatccccaaaaaaggttcatgcatctattcacatcaccctaacatgagcaaagtagcatccttcttcaaaccgtaactggggatgttgttggtgggtccctcccttttcaggttcagagaagatggagcctttcattccagttgtgttctgaagacagagcttcttggagctataagcaccattaggttgcttctttctcaggttaaaccactcagagtgcatttatggtctggtacttaatgccccacatgagcatatttcagacttcccccccattccatgaggcttgctttgttgatgtccttcatttttcaggatacgtatccacaaatccataagaattttcttccataagatctagatagtgaatcatctcgccgtaattgaaatcatcccattgtaaaccatttttaggcttaaaaaaaatctgacaaagaaatttctcccacctacttctcccaatgcaaagtagttaatcaatctctttaatcatgggattacctctatcttatctttcaccaggttttctggtctttggttatgtcagtgggcagggcagcagagtgtccaatagctagctgtgaatgctaagcaactgtagtagatgccaaatcagttgcaccaccaaagtctatgcattgaaatgaagtcattgactgcaaccaatttagatatcttttagtattttttttttcaaagacggatttcaaaatgggaacagggctagaagaatcctttcaattttaagttaaaaattatgcatcatcaatgcagattgccatatggttgtagagtaagatgaaacagagtcttagagcaatagtttatttcagcattagcattgttagttgttagacatctgtcccttccaataaatgaagattttgtaaacttcttagtcatttctgtccccatagatccaagaatagaattcacacatggtgactgtttattaaaggtctgctccattaacactcaaatgctaatgcacttccacttaataaaagagcttcatctttgggtctggcagctcatgacatatcccaagtgagtaggtgactatttcctggatgactatagtcaacgcagtgccagattttgacacctacacaaatatctccctttggtgagaaaagcaagcaagagttatagtgaaagaatagtgtgactgcagttaataccataatttgaagaacaaataatggcatctataaaaaaataagatgtgaagctcatagaatataagaatcaaagtgctcatggtagccctggttgctactagctgagtctacacatgctaataaatggcagaagacatgaaaaggcaaagcaagaggcagaacacacagaagagagagaaagagagggatgaaaatggaattatgtcagtgtactcataagtttggactgctagaaccgagtactatagactaggcggcttgtaaacatcatatgtttatttcttacagttctggagactaacattctgaaatagggtgcctgttgaggccctcctctgggttgcagattgctgccttctcattgtattctcacatggcagcaaaagaggtagagagctctctgggatctctttcataacggcactacatccattcaggaggattcaccctcatgatgtaatcacctctcaaagccctcccctcctatcaccatcacattgcgggttgggacttcaacatataaatttgggggtgatacaagcattcagttcattgcaagcagcacagcacaattcatgaagacttttttcttctatgcaatctcccaaatattccttgaatatctgtacctctgcctttgctcagactaatttcttctttttctccatatgccaggctcagctcacataccacctacttcttgaacaccccagcccatctcagcccccaatgctttctccctcctacaaactcctagagcttccattgtgatgctgaatgttgttctttagggtcgcaattagattgtataggtgttcttcttgtactcctaagtttcttaaataaaaatgacatggtttttgttctctcatcagctataagcatttcctaaccatctgctgtgaatagggatgatatagtttaggtttttgtccccacccaaaaatctcatgttgaattgtaatctccagtgctgaaggtggggcctggtaggaggtgtttggatcatggtggtgcatccctcatggcttggtgctgtatttgtgatagtgaggtcttgtgagatctggttgtgtaaaagtgtatggtacctcccccctgccccttgacactctgtctgtctctcttgctcctgctttcaccatgtgacgtacctgctcctactctaccttccgccatgattgtaagcctcctgagacctccccagaagcagaagcctctgagctttctgtaaagcctgcagaaccgtgagccaatttaacccagtctcgggcatttccttatagcagtgcaagaatgccctaatacagaagataaagaggatatgatctagagtttggctggactttaaccagagcccccatccctacaactctgaccccctgacactgctgtctgagcacacagctgtcctttagcacctttagccttgttttcttatttccagaacaagctgcatatttctggagaccattcctccactatttcactttttgaataaagcttaagtgcaccaaaagtaaatggcaataagaaaaatgtaccatacatgcctcacacacatgtacgctcacagtcatacacacaaacaagctgatacattagttttactttggctcacctctagaatctgggtggacagtctgctctatgccttttctgttctttctcttccattgtccgcagaatatgaggaccaaagtgctcattgttgtttcttgaattctgcatgtaggcaaggagtggtagccttccctgatgtattagtcagttctcacactgctataaagaaatacctgagactgggtaatttataaagaaaagaggtttaattggcccacggttctgcaggctatacaggaagcatgatgctggcagctgctcagcttctggggaggcctcaggaaactttcaatcatagcagaaggtgaaaggggagaaagctcatcttccatgactggagcaggaggaagagagagagcagggaggtgctctctcaccaaccagatctcatgagaactcactcactatcaggagaacagcaaccagggaaaaatctgcccccatgatacaatcacctcccaccaggccccacctgcaacattgggaattacattttgacatgagatttgggtggggacacagaggaaaccatgtcacctggctaagtggtgaccacacagttctcacctgtgtgtgggttattcactttctgctcttccctaagactctccttaaattcctggcagactcttgctcatgctctcctttgggagttcttcttctgctctacaatgctttctgcatttgaaccctttcctcatatgtcacaccctcttcaccctaatgggggtttattttgcttgatcactctttaatccatctgtactttcccttttgagtggcacccaagactgagcctcgttccaatagcagtgccctggaaccacagatttgggagctgaataggactgtcatctctttgctgtgtcacacactagtgatggaagcctgcagaattctcccacagatggacagtttagttatgaatcccacaccaacttctgctcatcaaacatcctcctttcatgatataggcagaaatttcagaagattatttgataatgccttgttttatttttttgacacaactgtcaaccacgccacttcaagatgtggtttgtccctcatggcatgaaacaggtctcaaacgacttgctatctggcaacaaaatggtacaccaacacattaaactccttcaacaggagaacatcttcatgacaaagacagtggttcgcaggttggacaccaatcttataggatgggtttccttggagttcagggttaacaacatgtggcaacttgtttgggatattatgaaagagaaaagtattctattctgccttaaccatggcggaagcagcccttgaggagctgctgtcatgacttccagtcatccttctaaaggaagatgtctagaagaatgtggggcaaaagtgaagtttgtacagagaatgagaggaacttacagataactttgaactggcatatctgtagttatctctattaatgtgaatttacaaaaagttaactagtgaaatagggacagataggcatttgttctctgaagccatttgggtatgtcttcataatcccaggacattgggcagaggcttcctctatcctcttactcagagaaatccaaatatggcaaatgatccctgtagcttcctgggcaaaggcccatttgcttctgattctttcaagggtaaacaggaaggctttatagaaagcttcagcttgtttctccaagagtttcctaacacagagataaatacataccttcccctgacatctctccaccctgcccacgtgaaacccttgctggctctctgtctctgtaacccctctagcctttcctttctgggggacttgccagcttgctactccacctggagaacagaacaggatggagtagaacaggaattttcaattctctcctttatatacagaagctctctcaagtctctctaagcttttcagacttaacgtgtctcctacaaaatatttgttcctgactcaccactaagaagatgaactttaagaattgcacagtttgcctctcccccatgataatatgcatagctaagccacagcaaggctacctttctcattcttgctgcctgccgatggtgtgatcttagcccctctctcagtatttgaatttcctcggtctttatgaatggtaagagttgtttaagtctctccttgcaacactccgccacccaccattcatcccataatctttcacatggaagactgcatgtattttgtaaaaccagggggaaaagtcctgattctaaatcaagaggcaattattaagagtggcacgcaggtcatttttcttccttcctccaaccaccctgtcaaccaccacccgccatgttcacaaaagcctccaaggctacctacaagaaaatacccagctttcctctagggtgacttgactcttcaaactgcttctcagtggaaaactttttaaacgctccgttttatttattctctaacagttttcctgttaactaggtttggaggtgttttctgaaacatgaatgccattaatccaacaccaaaaagattccagaactttccagggcacacatggccaagccttccagaccagtttgcactggaggagcgttctgcactggcaggcgtttctgcagcttctgacatcagggaaaaggtgttattcctacagtgctgctgacgttatgtaacagcagagccattgctttttttttttttttttttttttttttgacggagtcttgctctgtcgccaggctgggagtgcagtggcgtgatctcagctcactgcaacctccgccttccggattcaagcgattcccctgcctcagcctcccgagtagctgggactacaggcatgcagcacgcacgcccggctaattttttgtattttagtagagacggggtttcaccatgttggccaggatgatctcgatctcctgacctcgtgatccgcccgccttggcctcccaaagtgctgagattacaggcgtgagccaccatgcggccccatagcttctttagttgaatggctgcctctggaggcgggacccacagggactgcctgggtggaagaaaggcagggaaggctgctttcactcatcaccgcagactcactgccattcagctaggccgatcttgtagaactgacgtagaaaagattacttctccataagtataggttctggtcagaaccaaactctctttccaaggactgcttcctgcctgtttgtgcacacatcttgttttcttagggtcattgggactgaatactaattaatcgaggtctgcatgatcagcaccgaagcaagcgcctgaaaagagagtgaatcttttttaaaagttactttattatttgtatttattttctgggtgttgtttctgattccaagtagttacataaaagttgcaaagccagttaaacaccctctgaatgttcctgcagaacttggactgggcgctccctatttagaggttaataatggtcagtggctttctcttcctttctaactttatttggggtgtgcctagccttgagatctgggttgtggccatgaataggtctctgtagtccaagaaacatttctcagactacggaagatgtgtggaaagacagtgccaagctgcctgccgctgtggcagcaccaacggagaagaaaaacaagccaaaggatgcgggtgtgatcagggcctgcgcaggggttggagtggtcatttggggcttccagagggataatgacaagtttatccacaggagtaaagggttagagcagccagaagacgcttgtgtaatgtcccagcaaatcaatttaaagacttaaatatgacaacatgctaaagaaagcctggaaggaattggtgggtgaaaaggaaatctgccggccttcaaaagtgaaaaacgaagcaaaatggagctccaaaaaatggtggctcaacgagaccccagtgggcttggctagaggctccggaacagaaggcctcagtcacctcattgtattcagcacagtctctaaagctgagagcaggaaatcctgttgccccacccatgtcctcagctgaggtcccatgagacaatattccttagataccagcagaaacttttcttacatgcgaaggggtgtaattcacaatattctttagaaagatggttgaaaggtcacgtcattcaggccataaaacatttatccacacatttattcatcaataatttactgagtgctataccagggggaggggaaagggtggggggggtgggttatgatgatgccaacgattaaagagaccagtcaagacactcaagtgagcctgtggtctaaaatgatgctactgaaggtggcagatgcccacctgggagtatcttaggaatgcaaattccagccccgcccagccttactgaaacagaaaccctgggggtggtgcccagccatctgtgttttaacaagctttcctgatgcacggaaaatttaagatgtatgggaacatggtgtctcaaacaatgatgtgtcctggccatttgcgagatgtgtggaaagtaatatattattaatgatagttagcataccgacatttgtgaataatttatatgtatgtcacctgcaaagattttgtaaaaatacagatccctggctccacccaattccaacggagtagaaatatccaggtgtggcaggcagtatttagttttaagacttcccaggtgactcttaggatccgtcaggtgtgggaaccagtggtctataagagccatttgccccataacaaagagaaaaaatcatggaattctagagggtggtccctcggagagcaggtttccccactcccctaacaaatgttaggcagatctcaattgaaacacatacaagagaaactccaactgcagcagaaatggagtggaggttgcttcatactttcctttctgcagtggctgttgcagctcttagtaaaaatctagagctctcggccgggcatggtggctcacgcctgcaatcccaggactttgggaggccaaggtgggcagatcacgaggtcaggagatcgagaccatcctggctaacacggtgaaaccccgtctctactaaaaaatacaaaaaattagccgggcgtggtggcgggtgcctgtagtcccagctactggggaggctgaggcaggagaatggtgtgaacacaggaggcggagcttgcagtgagcggagatcgcgccactgccctccagcctgggcgacagagcgagactctgtctcaaaaaaataattaaaaaaaaaaacctaaagctctcaaaaatatggtttgaaaagcatggatgtttctatcaccacctcctcctcctgccacatacgccccattcattgatgaagaaaccaaggctcagaaaagtaaaatgacctgaaaacatgtgactgaccattcaggtctgcccaagactaaaggcatcccagaaattagagcgttcagttttaaaacagggacagtcccagaccaaccaggatgaattcgtcaccctaggtcggagacttcacgacacccacagttcttgcgttttggctgatttattattgttgttgttgttgctattataccatattactgcaagaagaattcaaattactattggtttttaatttttttttaaatttttctagccccttgagaagttcttactaaattactatggtttccttttaaaaaccatatttgtttttattccctcattccagaaggatttaagggagtaatacccttattttatgtgttttgaaatacttgtaagtattctaaaatactctggactattcctgtgtccatgtctcctctatctgacttcagacccaccataccatatgcattttctctttggcttccatatatttgtgtgatgtttgctatggcacctactgtgccctactgagatctgtgtattagtcagaactctttagcttgccagtaaaagaaaacaaaaggatggagtatgtcagcttgggtagcagaaaagagcttcaggcacaagtggatacaggggctccacctcatcaggacatggtccctctttgaacccatagcaagatggtcacatgcagctccacacacccgcatcctcccagcaacccagctgacggcatcttgtccccagtagcttttgtaaaagtccctaggatgaactctgtttgggctgacttgtgctatgacccttccctaaaccagttgcagcccccaggacaatggaatactctgattgtccagactgtggccatgcacccacccctggcaccagggtctaagaagagagaaatgcaagtctcccaaaagaaagtcaaaagatggttcctagaagcagaggaggaacagatgctgggtaggtgaaaacagcaaatgtccatggtagtcttaaacagttcaagagggctgaccaactgattggctgatgcacgggcaacagcatgcagctccatgtcttcctctatccccactctgctgagatctaggtactattttcccctgaaacactaggttgcaagactccaaggtcaccattgtcagttctaattttgaagacacgcaccacatttagctgaagctagcagcagccccagaacccatgggactccatccgaaaaatgataagccctttgctgggctcccaaatatggagctcctgagagtgaggagctggtgactcatgttctctgtgctttggttgcccccacgttttccagctgggttggtgacgtgggactcagtactttcttcaatgcgtcctgtacacaaagaataaatagccccagagctctttctttttcttcctgcctttcttcctgtaattcattctcagcccaactcagctttgttcaaaccacagtatttcacattgcctggcaagttctgacacagctgcttgctttattctttcagtcttctgttaagccagaggtaaagttataccttgtggctaatttttagtctgtaaaccttatcccttgttcaagccgaaatcttagattaatcagcatgaaaatgccagctcccccaagaccgttgaattatggcccccatcactcttcctgccctgacattcatttgagtccctttcaacttttacaagttgttttctcttatccatgagcaaggtggtggcttgggcctttttaggcaattttcttttcttcttaatcacctgcccctattccatccaatctatttcaatttctatataatcatgtaatacatctctaatttgagtcaccaggttttccacgttaaaggtgggctttaggaatgtttattttacaaactaatagaacttccagtcctatggactctaactagtagtggggccactgtgtcagcttcccagagctgctgttacaaagtaccataaactgggtggcttcagatgacagaaatagattttcttacagttctggaggccagcagtctgaaatcaaggtgctggcagggccacgctctttctgaaccttcaaggggaggatccttccttgcctctttcagcttccagcagccccgggcattcctgggcttgtggcagcatctctcacacctgtgcctccatcttcacagggccgccttctccctctgcgtctctttcacacagagttctcttccccttttacaaaaacagcagtcatattgtatcagggctcaccttcatgacctcatcttaacttgatgaaatctgcaaagatcttatttccaaataaagtcacattcgcaggtgcaaggagataggactcccacataccctttcatggggaaggaagacacaattcaacccctagcagccaggaaagagaaaaacagggacagaaaaataactctttgatcttggtcaaccaaaaaggggatcctgatgttctcagaggatgttcacccagaaagagcctgggaccccgacaggaacatctggagatggaggcgaaagcctagcagcaaaggtgatcgctcaagagggcaggagaatccactggagggcaaaagccaaggacacatttgtgcttgaagagcctactgtgtgccacatgtgcttttatcccattgaatcctcaaataactctgccaaagagttgctattattcttttttaatacatggagaaactgaggctctgattaaataatgagacccagattataagtagaaaagcgagatcatgattgctattaccgctgtcacttctgtttttaataggcattggatctcttgtgctactatacaccaaggatgttacctgtattaactgagatcttcacagctcacaaagctagatattgatggccttatagagatgaagaaacagaagctcaaagagtttcaatcacttgcctgaagtcacacaagtattacataattcagccaaaatttaaactctggtctttctgactggcaggaccattccttaccatgatgccatgttgctggtggacattagggtatctaaactagggtagtcctagcttcagagaaagaagctgtataaagaaaccaaatgattatgcttgaggcttaaccaaagcaatataaaaagtgtatgttctcaggggaatgggcaaaacagaagagaaaaaggccggccaccgagcggctgtgggtgaatgagttaaccaaagagcaaatgtctgagttggatcatgaaacagcagatcaagtgggctcagtgtctgtaaacatctacactgcccatgaggacaagatctgtatgctccatctacacccagaggctgaaggaatgcctgtggtgtagacaactcacttttctagagaaatggagaagggattagacatgttaaccctgaagaaaaggaaacttggggtagggtaggctcagaaagtcttcagaggttgggaacgtggcccatgaaagagcagggagactggaaagggaccctgcctgtggaggcagctctgggccccacttgaacacacacgggtgaaccacttgacccaccttacagtgaaagaagctggcacctgtggaccactggagaaacctcagtagccatctggtgttccccaatgactgtgttgctcacaaccctcaagagtcctttgttgcttttggaattgtagggctggcaagatgtcttcacccactgctagattcatggctgaggcccctataatgaaggacagatgaacaagagaagaacatacaaacgcatagaatataagttttacatgacacagaagcctttgaggggaaatgaagaaccagagaaacagggaaacctgtgtatttgctatgctcgattggatgaagagtggacagtcatggagaggcatgaccgagcaaagcgggtgataacctggagggaatgtcaccacatctgttggctcagattctcctctgtgtccttgtgtcttcagaaaaaggatgttcctttcctctgagtatgcgggcatcactcacaccagggtccaatgtcctacttcaggggaaagtcaggaaatccttcctgggactgatgaccggcctcagagagaagggtagaacaagggaaggtgagagtggcctttctgcttttgctgttttctcaaatgccaattttctattttcaggggcaatatgtcctgaaccccatcaggatgaagccccagctccatgaagcccctcttgaactggtccatcctactgttccagtctcagctccctctgctccaggccttgaacttcacattccagcctggggactcctggcagttccctaaatatgcaaagagctcagctttctttcctggtcctggtcctggtcacttggccctctctgtctctcccttccttcttcccatctctcttcctttctggctcatgtccctcgcacatgctgtaaactcttcctggaacatctcccttccacctgtgaatctcttgccagctcacttcttttctccctttaagaatccacttctcaaaagaaaatggcaactctgtgaggtgatagaaatgctgattcgcttgatcattgtggcgtccacaatgtatatataaaacaagttgtacacattaccatgtataaatttgtgtttgtcgattatatgtcaagaaagacaaggaggtgtggaaagactgcacctctgtcaagacgcctttctgaccaccccccgaccctggttgacactccctgacatgagcccccgagtgtttacctacgctatgtgtatcagggcatcccgaccacttgctcactcacctgtctccccactgtgaggtcagcggcagggccttgttcagtgtcttagtcatatcccctccagcacccaccatgacctctggcactaagtaggggctcaataagccaatcattgtgttgatgtaccagtgacattgagggaagaccaagctcgccgacctctaagatcctgtccactctgagagtctgtgagtctgtatttctgctcccacagttagtcacggaggaagttgccaaagcagatgatgagacttctgtttggggttgcccaggtctgcctggcctttgcaatttgtaatcaggtcctttgaaagagaaactgaactgagagaaaaacacagtttggatgaggcaagagttgcaaaataatgagttatgtaatggtgatggtggcctgtggtagcatctttggccctgcccagatgatacaagactttgtatgtatacccttgagcatggccaaaaggacaattgtcaaaaccacggcttaagtgttcaaaagcctcttttcccataagatgttgcctcttgaggtcagactgaaatcctgtacctgtaataatttcctccttaggactggatgtacatgaaaagattggagatatatatgtaccttttttatatgccatgtaaatggtataacccttgcactctttggccattaacagccaattgtcaattagtttattgtgtattagatcaaactgtattgcccaggccagctcctgaagaactgtgaactatgaacatctcagcctagaaggataatgtgaccttcaatttgcacaccatccattgtctctttcaaactaagagcctctctaagctagataggccaaggattatttttttaacttttattttaggttcaggggtacatatacaggtttgttacataggtaacctcatgtcatgagggattttgtatagattatttggtgacccaggtactaaacctagtacccattagttgttttttctgctcctctccctcctctcaccctccaccctcagttagttcccagtgtgtgttgtttccccacatctatccatgtgttcttattatttagctcccacttataagtaagaacatgcagtgtttggttttctgttcccgattagtatgctgaggataatggcttccaattccatccatgtttctgcaaagaacatgctctcattctttaatatggctgcatagcgttccatggtgtgtatgtaccacattttctttatccagtctatcattgatggccattgtggttgattccatgtcttggctattgtgaatagtgctacaataaacataacatgtgcatgtgtctttatgatggaatgatttctatttctttgggtatatacccagtaatggaattgctgggtcaaagggtatgtctgtctttaggcctttgagaaatcaccacgctgctttccacaatggttgaactaatttacactcccaccaatggtatataagcattcccttttctccacaatcttgcaagcatctgttatttttttattttttgttaatagccattctgactggtgtgagatagtatctcattgtagttttgatgtgcctttctctaatgattagtggcattaagcttttttcatatgcttgttggtcacatgtatgtcttcttttgaaaagtgtctttttatgtcctttgccaaatttttaatggcgttgttttttcttgtaaatttgttaaagtttcttatgggttctggatattagacagatgtaagatgcatagtttgcaaatattttctcccattctgtaggtcgtctgttccctatggtgatagtttcttttgctgtgcagaagctcattagtttaattagatcccatttgtcaatttttgcttttgttgagattgcttttggcatctttgtcatgaaatctttgccagttcctaagcccagaatggtattgcctaggttgtctttcagggtttttatagttttgggttttacatttaactcttcagtccatcttgagttgatttttgtatatagtataaggaagggatccagtttcaatcttctgtaaatgcctagccagttattccagcaccattattgaacaggactcctttccctgttgcttgtttttgtcaactttatcaaagatcagatgattgtaggtgcacagctttatttctgagctctctattctgttccattggcctgcgtgtctgtttttgtaccatgctgttttggttactgtagccctgtagtatagtttgaagttgggtagtgtgttacctcccgctttgttcttttaacttaggattgctttggcaattcagactctttttttggttccatactaatttttaaatagttttttctaattctgtgaagaatgtcattggtagtttgataggaatagcattgaatctgtaaattgctttgggcagtatgtccattttaatgatgttgattctttctatctatgagtatggaatatttttctatttgtttgtgtcatctctgatttctttgagcagtgttttgtagttctcattgcagagatctttcacctccgtggttagctgtttcctaggtattttattctctttgtagcagttgttaatgggattgtgttctgctctcagcttgactgttgttggtgtataggaatgctcgtaatttttgtacatcaattttgtatcctgaaactttgatgaagttgcttatcagctcaaggagtgtttgggcagagactatggggttttctagctataggatcatgtcatctgcaaacagagatagacttcctctcttcctatttggatgccctttatttcttctcttgcctgattgccctggccagagcttccaatactatgttgcataggagtggtgagagagggcatccttgtcttgctccagttttcaaggggaatgcttccagcttttgcccattcagtgatgtgctggctgtgagtttgtcacagatggctcttattattttgaggtatgtttcttcagtacctagtttgttgagagtttttaacatgaagggatgttgaattttattgaaagctttttcttcatctattgagatgatcacgtgggtcttgtctttagttctatttgacccatcacatttattgatttgcacatgttgaacaagccttgagtcccagggataaagcctacttgattgtggttgattagctttttgatggctgctggaaaggtttgctagtattttgctgagggcttatgcatcaatgttcatcaaggatattggcctgaagtggttatttttgtttgtttgttttgttttgtttttcttgttgtgtctctgccaggttttggtatcaggatgatgcaggcttcatagaatgagttgggaaggagtccctcctcctcaatttttgggaacagtttcagtaccagctcttctttgtacatctggtagaatttggttgtgaatccatctggtccttggctttttttggtttgtaggaggctggggatttttatcccagatttataaataaagaaattgagtctcagagagaagtgacttgcccaaagttgcagctcatgaaaataaaaagaagtggccagacatccgatctttgtaccccagtgctcctctccactttgtaccccagtgctcctctccaccctgcacctcttgggcttgctcttctggtggaaacacaaggacctgaggtgaagctggagagtggaggggatggtggagagggctgaggagagcaggctggtgagttgtgctttggggcctcttagcccatggagatacatgaaggatgaggggaaggggttggagcatagaaatggagtttggggagcaggtaacaggagaagctggctgacctttcacaacacaaatttcaggccagtcctgactaagatgctctgggctgaagccaactgagcatgagctcccacagagaaaagaggtttgcacatcctctccacatgggtgcccatgagccagccccctactaagcacaaattcagggttgctgccctaagcagctactggctgagtgatcaaagcaagtcaagagccttgaaaagttgaaagtggctgctcaaccagcagtcagtccagatcctatctataactccagtcctccccagccccctccttccccgatgagagtccagaccagcctcaaacagaaactatggagatgaatcaaagacagagccaagacatctttgcctgggaattctagtgtatccatcataattgggtttattttacccagtaaagagagggctttccactcacctcgggggggggggcctccgagccttcttataacagtacaacgaaagtgaaccacagacatttgttcccttaattaacagcgttgctcttttgggtgggtcttgaactgttagcactggtctcccacattctttagtcagttaagggctgccaccatcatgacatggaatagtaggactgggagaatgtactgaatcagtacctagtgcagaacaaaacccttccatggaacataaaaggtacaaatattacattcacagccatgtttgttcattcaaagagcatcttctgaagactttctgtgtgccagacactgtccccagtgctggagaaaatagacaagatccctgttatcatggagcttatatgctaatggtggagacacaaaaaagccaaataaataaataaacacgctagaccatgtcagagagtggcaagtgccatgaagaacctgaaaatgagacatggtgttgtaggagatgccttagatagggaggtcctgggggcagagtacctggaggtctgagatcagagcttttacgcaaacagagcaggtgcagaagttgtgttcgaggaacaaccaggaggccagttggcctgcaaggcatgagccagggaatggtggtacaagataaacttggaaattgtttatgctctgtctctcacactgacttggccttcgatctcagctaaaatgctgctttacttcctactgtattggtgtttgcaaccaatgcatgatgtgtcatgtactttctactcagagaaaagtcctctaccagtgttgatgagggtgaaaagatcattcctactccaggaagtctctttggaaacttggtggcggaagacaggagagctaagagcagttcccatcttgtatgatctaaggttcccctggaagtgaagccacgatcccctgtagctatcacagcatagggatgtgcggagatcctggctccacatatagttggcaggaggtgagtctcctttaaggtgttcaaatgtagcacacacacacacacactctctctctctcacctgctgtcttgctcgatgctccatctcttctattgctgtcctgagaaccaagacagctccatgtacaagtaactcaaaaccctgacactccctcacactgcccaaaacaagacactgtcaaaataagtcacagatgtcacagttccttgtcactcagttttcttggcttagatttaaagcattaaatcagctcatcttcatctctcattccctagccccagctcttccctgctgagttatctttgatattcccttgggtggatttcttctccctccttcttctctaagaatctgtaagtttattttctctcttactctcactccccttctcatcctgcctcaccccggtccctctttctaagccctcttctccaccgccctattctagacaagatcttacaaaaatacctttcttccataatatcttctctacttccacaagaattcccccagattcctttcctttttgttgaaagggctgactcctggcatttataattttaaccagcagaagggcttgaaatgagaagtatgagtacttcgactcttttccacacctgttcccaatctccacttttttttgaatactgactctgtaatgggtggagagtaggggaaaagaaagagagatgggaaaacaagaaatgaaagggatttttagtaataaaagcaaatgaggagataaggtaactgtgttctgaacatcagggctggagaggctgatgctcatgatggacacaggaggagaggcgcagtgctggctaacaacctggacacagcaccaagcagattgtagtcacatgctaaagcatgtgctatgccatctaggtgcagtagagatcagccataggctggagtttgccccgaaggaggtggcattgaggtcacacactgcagagtcatccacatgactttgtagattggaatcttattttatcaactgcttacctgaaataaacatgccccacctgaaacttaaatgcagcttgatcttttctttggaagagtgtgatgcttacgacaggaatgtgttgccatgggatgctgctgatattttgtccacactcctatcttagcctttcgccactttgaaggtgccctctttctccaggataaacatcttcaacaacggggactttccaacagagtggaccaggtgaatttttttaactctctggaatttgatgttatgtgagatttctaactgtggaattgcgctcacattcatgttagaatattatgtctatcacatattcttatcagcacatttttgtagccagagatgtatgcaacccaagtgtcatgagcccactacacctaagagtttagacttactaattcactgaaaacttaaaagaggccaggatgtagtagattgcttggtgatagatagcagcctactcaccctgtctcttgagaaataacttcacttctctcccccttatcctaattctctaaaacagtcctatcttccaatggataaagtacagacagatatctggttacctttattgtaaacatctatagttcacccaagagcctagatgaagcacctcacatagcatgccaactgctggcccgtgtatttagtctatgtttaatacccttttacttaggtttcttgccctgtaaattggaattagactaaaatctggtgtcttgagtttcacagcatattgagtttcacagtatgattttagcctgtctactcatcttatatctgatagcagtaaagaaggtaaattcattcattcatatattcctttattcattcattcatgtaaatttattgagcatgcattttgtgctaggcactgttcttggtatggtccacagctctgaacataacaggcaaaagttcttgcccaaatggaagttacattctaggaggtaatataaagcaagacaaaaatatccagtgtgttagacagagatatgtgctagggagtagtggagtagtggggtgcagttttaaatagggtactcagggaaagcctcattgagaaggtacttttttttttttttgagacagagccaccttctgttgcccaggctagagtgcagtggcgccatctccactcactgcaacctctgcctcccagattcaagcaattctcctgcctcagcctcctgagtagctgggattacaggcgcatgacaccacacccagctaattttttgtacttttagtagaaacggggtttcaccatgttagtcaggctggtctcgaactcctgacctcatgatccacccgcctcagcctcccaaagtgctgggattacagacgtgagccacggcactgggccgaagttaccttttttaaggttttttttttcagccaatgttaccatggtgtaatttatcttctgtaaaattcccacattttaagtgtacagatgagtggcttttgactaatgtatacatccactaccctaatcaagctacagaaaatttccatttccttgaaacgtccctctttctttttcatatttagtctcctactcccactcaagctaccacagatactatttacatcattataggttagtttttcctgtcctagaatttaatatgcaactatgcatgttaagtcttttgaatgtggcttcctttggttagttgaagccatgttactgcatttatcagtcattatttttttattactgagtctattgtatgaatgttttataatttgtttactcagttacttattgtttctattactcttcattctttgtgtggtttcttcctggtactattctctttatactgaagaacatcctttagcattgcctgtagttcagatctgcttgtgatgaatcttctcagattttgcttatctgaaaatgtcttcatttcaccttcaattttgaagactatttttattcaatttatatagaattctgtgtgaataggatttttacatctccaaagatgttgtttcattgtcttctagcctctactgtttctgatgagcactagtaataattcttaactttgttcctctgtatgtgtctttttctttggctgcttttaacattctactttatcttcagtgttcagtcatttgactgatgtacttaggtggggcttcctttatcttcatcttacttgggcttcgtggatttttaagtcattttttaaaattttgggaagctcttggccactatttcttcagatattttttctgctctctctctctctctcctccttctgggacaccaaatagacgtaagttagactgtctgatattgttccataggtctttgaccctttgttcattttttccttaatattttttatttctgttcttcagatttgatattttctactgctgtgtctccaacttcactttttcttctatcatctccaacctgctggcaagctcttccgatgaatgattcacttcaggcattgcacaattctagaatttccatttgtttctttttagggttcccatttatctactaaaaattcctcatttactcacaacttagggccatttgtctctaattaattaatatattttttgaatatatattgtaaaacatatatgttttaatgtctttattttctaaatccaacatttggtccatcttagaatagttcctttgctttcattttttactatggattacactacccttgtatggtttttgttggtttttatgtctagtgatttatcattgaatactgggcattgtgaatgttacattgtagaagctctagctcagcactcttcaatagtacctgcaatgaagaaagtgttctgtgtctgcaccatccaataggacagctgctggccacatgtggctattgaacacttcaatgtgactagtgtgactgaggaactcaattttaattttaatctaaatgttcgcatatttacacccagaacttctcaacctctgttatactgtttcagtctcaacctcatagcagctgacatctggcaagcctctgatggttttccctgcacatatacagtcaagccctcagccgtggactgagggaggggcttcccatacgcatgcaaggacttctagggctttgtctttgcacagattccagctatttcagttgcctcagattctgatccctgcctcttcagcccagcaagagtcctgtgctctgctcaaactcaagtctccaggcagacagctggactactgtggggctcacctcacactcccctctccccatttttgcagtctggtgttgtttattttccattgtctgaaaactatcttgcttcacataccttgtcctgttttctaattgtttacaggagacgaaatagtctgaaactagtcattccatcacagtcagtagcctgagaagtgtcccttcaggtcataatccaaagaagattgtgggataactaactaggggaagagagtttcaaacagggggacgtcaatggaaagggtgggaggcagaagcatgcctgcctgacttagaacggtagggaggcaacatggctgagcacgagagctaaggacagagagagtaggacagtaggtcagagaggcatggtggtgggaaagacactgtttggcttcataggccattatctgcactctagcttttactctagtgagatgaaaagtcattggaaagtttggggccaagaactgatttaggttttaacagaatcacactagctcttggaaacacctccaggacaaaagcagggtgctgaattagaaggccattgagagaatctattgactaaacttgcaaatctaattaaaattctgaattattcaaggtcgatggctgagtttttattcatttcctagagtttggggctcacgaggagacaggtaccttagtgtggaagatcacatcatctgaagtctgattggctgtgtgactttaggcaagtgacttcaactgtctttctttatttctatacaatggaaataataagaatacctattacataaaagatattatgacgattaaatgagataattcctgtcaaattctctaaattatacctggtgcatataattcctgtcaaattctctaaattatacctggtgcatatgaagtaagcgttctacaaatgttaactattactatctgagaggctgaatgtctgatgattattactgtaccctgtggacattgacattgatctactctgtgaataaagggtaccacactcaattctgattctcaagagatatgtgcaactggcatagaaaaaatatctcaaaaacaagactgaaggaaattagagccaagtagaggtccatgctgtcagctcttgcataaggagggaaggctgaggcgttattcattcaggctgaggagatctttgaagactattgagaggcaatgagttagggtttgaagaatggattagatacagagactgtggaaagggaagggaattctgaaggtcacctgaacttgcggccatcactaatgtttaaagagcttcttaaattcaaagtgaaaaattatgagttcaacatggttattatccccttaagctcacatttggaatcaaccataagaagtaggatatcattaccgtacagctgaatggctttattaacttatttttggaaattagatgacaaatgcaagcacagtcttgtttaacaagaagcatttcccagttgtttctatgagaatttaagaaaggttctagaaatgcaaatagagagaacccagtcaagtcctgaaatctcagtgcagcagaattgagaaagtgaataatggcccacaggtcacaggaaggcaatgaatacgctaatcaaaggttgtgattaatgaatgttgtctcacatttcatctggcataacatgtgtccaattgatcatttttagcatagctcatcagaggagaaaaacttggtgaaatatgatctggtggggcaggatgcaccagttgcacaacagacataagctgctccactttggccacacctgtataaaacatgagaaaagtaggttttcatagaggttgaggcatatctaactacctcaagtagaaaaagagtatccatttatttaatgagggagagagcagtggaaaggctcagcctcatccaggctgagaagtgattaccttggaaatgctgtttgttttgattgagaaagtcagctgagaatgtattttaaataggcagaaaatatatctatcaaagaaatactatgcagtcatcaaaaagaatgaggcatgtttggtattttaatagttatctccaatgtttataataaagtgataaatgcaatatatagataattatatagtgtatgacaattatgagaaaaatgaaatgtacatctgcacatacataaggttgcacacacaaaggatgcctctgggggagggaaattgggtagctgggactgaaaataaagataaacaggagacttatgtttcagtctatatcttttgaatttatttgtatatgcacctagatccagatagttttatttctcggttgaaaaaattaaaaaagaataggaaaaaagaaaataacaaccatagtttaattttttttttttttttttgagacagagtctcgctctgtcgccaggctggagtacagtggcacaatctctgctcactgcaacttctgcctcccaggttcaagcaattctcctgcctcagcctcccaagtagctgggattacaggcacacaccactacacccagctaatttttgtatttttagtagatatggggtttcaccatgttggccaggatggtctcgatctcttgaccttgtgatctgcctgccttggcctcccaaagtgctgggattacaggtgtgagccactgcgctcagcctaatttaatttttaaaagagctggaatgcgtccattcctttcccatttgcaaagggctccagaatcatcccagatgatggctttcaaaatgatagttcaataagggagatttaggataaagtgcttctttctgatgcttcacttaagggtccctgagagtattagtttgctagggctgttgttaaaaaacaaaaacacaaactgagtgacttaaacagcaaacatttattgtctcccagttctggagactaaaaggctgagatcaagggtgtcaggaggattggctcctttcgagggctgcaagggagaacctgtggctctctcctaacttctggtgtttgctggccgtctttggcattccttggcttgtagaggcatcaccctaatctctgctttcatgttcatgtgtcactgtccttgtgtgcatgtgtgtttatgtccaaattttccacttttataaggacaccagtcattggattaggggtgtgctctagtgacttcaggttaaccaatgacatctgcaacaaccctatttccagataagatgacattctgaggcactggggcttaggacttcagcataagaatttggaggggacagcactcaactcatgacaccaagggacacttacccagagttaaactgcttactgaggggaggtttttgctatgtgtctatgaagcacagatagtaacatgcatctcctcatgcccgagatgtataaagtgaatacacgctggtatgattgaaaaccttaatattttttaacgcactaccatcctctgaggaaagaagagagcttaaacttgcttaactaagaacaacagcttgttggagcgataaatccatgaaacaaaactcagatcccctgctcttccctccccatccatgccagctaaaggcatgtgcacacagcaatgtttattaaacacctactgatgcccgatactgcactgagagccagggacggagttggacagaacatcctcctgcccttcaggtggagaaaagacacataaaataatgcaggcatgcactaagtgactatgcttcagtcaacaacagaccgtatataggaccgtggtcccgcaagactatgatgaagctgaaaatttcctatcacctagtggcattgtagccatcctaacatcacataataatgcattgctcacatgtttgtggtgatgctggtgtcaacaaaactactgcattgccacaacatataattgtgtacagtctataatatttgatgatagtgaattactattttactagtttgtttttactatagtatacttttaatcattattttagagtgtacaatttctccttatttttaaaaattaactttaaaacagtctcaggcaagtccttcaggaagtattccagaagaaggcattgttttgtttttgtttttgtttttgagacagaatctcactctgtcacccaggctggagtgcagtggcatgatctgggctcactgcaacctccgcctcctgggttcaagagattcctctgcctcagcctcctgagtagctgggaccacaggcatgctccaccacgtccagataatttttgtatttttagtagagacagggtttcaactattggccatgctggtctcgtactcctgacctcatgatccgcctgcctcagcctcccaaagtgctgagattacaggtgtgagccaccgcgcccagccaagaaggcattctaggagatggcaggtccctgtatgtcattgcccctgaagatcctccagcagggcaagatgtggaggtggaagacagcaatactgctgatcctgaccccatgtagggctaggctaatacgtgttctagtgtctttctttttaattacaaaagagtaaagaagttttaatttttcttaagtttataaagtagaagaagttatagtaagctaagggtaatttattattggagtaagaaaaattgtttgataaatgtagtgtagcctaaatgtacagtatttataaagtctacagtagtgtacggtaatgtccgaggccttcacattcactcactgactcacccagagcaatttccagtcctgcaagcaccattcatggtagctgctctatacagatgtgccactttttaccttttatatccatattcatactgaacattttctatgtttaggtaggaagtatttacatacacaaatacttaccattgtgttgccattgactacaatattcagtacagtgacatgctgtctacttttgtagcctaggagcaataggctagaccaaataacctgggtaagtagtaggctctaccatctgggtttgtgtgagtacactctatgcactttgtacaattacaaaatcatctaacaatgcatttctcagaacacgtccccatcgtcaagtggcacatggctataattatatcactatagtatagtaaatgtagagccatgaccaaggcagaaagaaaaccgttaactccacttggcgatgccaaggaaggtggcctatgagaagtgtcataagagatgactgtgaaaggctgactctgagggaggtgagggcaggaggaggtgactagggaaaagggagtcctggggcatgtcgtgtctcaagcgggggagcccagacagactcctggttaccaggaatggagacaggagttggaagtaaatctcaagtgcagacgagcttctgaaggagcttatcttcagcctgaggatttgggacttctttatcctccaggaaaccctggaagatttagaggagccacttggtcagatttccttctttgaaatatattagattggtgcaaaaggaattgtggtttgggactgtgaattttagatccttataactagactcaaacacatctttattaattcaaataggaacaattactatcaacacatttttgccaatgagaaataagtttgtttattcctgtagcataaaggtctgtgctttgggattcaatgaacacttggaaagcattttctgcacactgctggttgtggaagcaaaaagttgttgagatgcttgaagaagtggtagtcggttggcgagaggtcaggtgaatatggtgggtgaggcaaaactttgtagcccaattcgctcaacttttgaagcattggttgtatgacgtgcagtcgggtgttgttgtggagaagaatttgtccctttttgttgaccaatgccagctgcagccactgcagttttcagtgcatctcattgatttgctgagcagacttctcagatgtagtgatttcgccaggattcagaaagctgtagtggatcagactggcagcagactaccaaacagtgaccatgaccatattttggtgcaagtttggctttggaaagtgctttggagcttcttctcggtccaaccactcacctggtcgtcactcgttgttgtataaaatccacttttcattgcatgtcacaatccgatcaagaaatggttcattgttgttgtgtggaataagaaaagacaacaccaccaaatggtgatttttttttactttcagtcaactcatgaggcacccacttaccgagctttttcaccctttgaatttgcttcaaatgccaaagaacagtagaacagtcgatgttaagttcttcggcaacttctcgtgtagttgtaagaggatcagctttaatgattgctctcaattggtcattgtcaacttccaacagctggccgccacactcctcatctttaaggctctcgtcctctttgcaaaacttcttgaaccaccactgcactgtacatttgttagtggttcctgggccgaatgtgttgttgatgttgccagttgtctctgctgctttacaactcattttgaacttgaattaaaaaattgcttgaatttgctttttgtttaacatcatttccatagtctaaaataaacataaaataaacagcaagtagtaagtcattagcaaaaaaacataaagcgagaaatgcccattaaaatgatgtataacataaccacatttatttaagaatgtattccaatatcaaacagcaaattccaacaatgcaaaaatgcaattaacgtttgctccaacctaatattttcagagagaatgaataatggggaaagaaactgaagagaaagtaacaggcaaggagatatttgcaggtgagaaaaaaattatgaccaatagtctaaacagtggtagcggtggcatgaatagagaaaacaggggcacccttatcttgcccgatttgtacaaattcagttaattctattttaacttatttatttgtgttatttttcagatgacaaaagataatacatactcactgtaaaaaattttggattaaaacatttaaaatgtataaggaatacaacaaaatcgccccttaattactcagaaataagcattcttattaatgtttgtgtatcctattaagttcttttcaaaatcatatctatgtacatatatagtcatttactcagacttttataaacagctttttccactttatatatttccctattagtaactttatagaacttgatttttgattgatgtgctatatttatttagctaatctagaggacagatttgaaaactgttaaggaattataaattgcagtaggaggtgattaattagctgatggggtatgagggaaaggaaaaaaactgagcaaccccaacttttgggctaaagcccttctttttacagctttcttcttgttttggccagaactggagggtccatcttgtgaaaaggaggtggcagaaggatctgtgaatatatgttacattcaacctcaacgatggtgaacataagcactgttcagggcatgcagacacagccccaggttcacaagctgccagaacattcattaaagtggataaaatggcctgcaatgaaatcctcaaaggatgtggtagataaagcaaatgccctcctaaacacagctgcaggctgccaaaacccccagccacacctggtgagcattctcagagaggagcaagtagagacagccttccctgccaggagggagtccctctccaggctgtgtggccctggctgtggtctctgcacctgccgcttgcctgatggctttcttgcattctgggagggcatgcctgtccgagcacttcctctgctcagtctttccatagcgagaggaggaagagcaagaggagtcaatacctgtgaggcacaataaatccaactgaggtgaataataaagcgtattcatttccaaaaacttagaagacaatgttagggcagatattgggaaagaaactgactaattgacccaggctttcatttcaggctcagtttggtttccattgcctaacacaactctcctacgctcctgtgcctcttcagaaatggcttctgattgaaacacaacctgtgtcttttgattgattgggaactgaaagatgttcctcttttaatctcatggatggaacccaatatatttcactttcttctttgtgctgatagacaaagcctcggaaaaaaatgctatttaaataatagctttcactgacagtagactcatgggaaaattgtccttccttccttccctccctccctccctccctccctcccttccttccttccttccttttttccttccttcctttttctgaagtgtatggaccattattgcttttactttgtcttatttggcttatgggaaaccgtgggactcctcatatatctatgtgctgagctgacataagggggactattaaccgcttctatgcagcatttattttgctgaagagaaaacatggagtgtggctttgttgaaaagctccccatcattcacagttcactgaaactcatccattcaatcatcaagcacagatctacctctgctccacttgtgcctgggatggtgctagatgctgagaacgtgccattgcccacatgttctcagcatctagcagaagaatcagttccagagcacactcacccagcttctggaatctcacaggttagttgggaggtcacttaaatagaacacgacgtgtgctgtaaacaagttaagcacagagtgcaaaggagcatctaattcaagagctgcttaggatggttttgtagagaaggcatgtatgattctaaaatgaaggcatggcacgtgcaaggctgtggtgttacaagagaacttggagcatttggagaagcggacgtagcgcaatgtgaggcgagagatgagagtggtacatcctagcaaggaaactcccagtcttggaggtaatggagaaccattgatgaattttaaggattttaagaataggcataatgtagtcaaattcacactcagtgaagtagtccttgaaccattgttcactgcaccacatggtcacagtcttattaagctgacagttgaaagtttcattggaaaacaaacctggcagttcttgaaatggaaacatgaaggtaatgcagggcctacaactctaggttgcaaaaagatcaaggacatttcatagatcttgccttacttttcctcttagggcaaaacacacattacaaagaccctcaaatgatgctcactgttaccaacatttttttctaatcttacatctttcatcctaaatgctcatgaaagacatgttgcttctggttcaaacttgggccaatgacaatgcttttcatgtttgttgacccaataatcagccattgcactcaaagacttagagcggatcagtttaaaaacagctattactgcatttgaactacagctcccctccagccctctgtatgtctgggcttgctgctgccacaggaaagctcctagttctacccagggagggattgtgtttctcagcctgtttcagcaccaacccgtaaaagctgcttatgtcaaatgtcagttaattgcaaacttacccgtgaggtttaattgaccttattccacaacaagtgtggccatatgaaataaacccaaagattcatgatcaggcaggtctaagtgttgcattttggagaatggcaaggggtcgtttttggaaggagatggagcacctcctatgctaatctcatgagattagctttaaacatcttcagtttcctccagtcaataatttgttatggaactgtcattttacatttaaacattttttgaacccttttatttttgcaccctttagcgttgggataaaaaattcttaagtcatatctcctccccactcccaccaccgccacactgttttatataatacttccttttactattttactgttttaaatttatctaccttcctgtccacaccccccacccccgcctcaccctgttgcttcagaaaaactcatgatttgtggaggagtaaatgctcacaactatctattctctcagccctacatctctctcaacttgcgtctctctggacagaacaatttttatctttttagcaattcttataccgcagttccccttcactgccataattctggtgaactcactgtttgagatcagtctccactgttccccatggagatcaccaaagccgatactaccagaagctcacatttgagccctgcagaacattgaggaaaagagcattttgggtttggtttgatttgtttcagctattttttcccctctctagaaacatgggtaggtggagcttaccaggtgaggttgctgactttcttctctagagtctgtagagtagagtatctacacaatattccatttgtgaaaatttgcacaatagactagataaacaacggattacggagaaaacagccctaatactcagaccctaaagcagtgctaggttaacaacaaggtgcttacttgcttggggtgccagccaaagtcagaacaatgaggctttcatggacttatccagaattttataactgataaaaagaaatcattttatgttttgtggtttagtattgctttaatctgggtttatatatgggaggaggcaccaaaatatttcagtgcttggggacttagactaaaagccacaaggaggaagagaaaaagcaggaaacaggctgccctttgtcacggaccttgtctttcctggcactctttggctctggttttcacagacatgagtctgatgagaatgctgagtgattggcttccagtctcagcagagtgtatatgaggaaagaaagcactggttgcctttgctacgtctagcctatgtctccacctcccccagtgtatcctagttagcccctccccaagcttaccccctggtcattctcacggggtcctgttttttaccctaggcctcttagtgctctctgttcccgccaaaatatctttcagatccgttagtcatattaaattagcaacagctctttacaagttaaaggtcttctccctcccacagataatgtcataccaacacgggttaaagtcttagctaaagaaggagtgtctaactttggattctcagtcataaaccagtggaaaggacatctgactagggggcaggtgatctcagtgcatctaagctcccgctgtatggactcgtgctgcctaacagagtagctaccagttgcatgggacgattacaatttaattaattaaaattacataaaataaaaaactcactacctcagtcacactggccacgtttgacccactcaataaccacatgtggctggtagctcccacatcggacagcacagatactgatcatttctggtctcacaggaagctccccattggatggtgcaaatctaagtaatttccttcttggcttatgcaaaggcaaggccctccccagtgcagggttgctcaggcttagcactattgccatcttggactggattcttctttgttgggggtggggatgtcctgtgcattataggatgtttagaagcctccctggtctctatcccctacatgccagtaacagccaccgccccccccacccagttgtggcagtcaaaaaacatctcgagacattgctaaatgtcccctaggggacccctacactgaagttggctggagctctggggatcagggaggacatctgcaagcgtgcttatgagttgtaagctctaagaggggagggacattgcacagggcaggtcaggcacattgtaagtgctcttaaaacattacagttgagaagaatttcagagtaacatttatagccaagaaagatattcttcccccaacttgggcattcccttgatgttaaattgtcctgtgcgtcaaaaccctaaagaactgcagggaagcctataaccccaaaggaaggcagagaaaggtcctgggggacaggttgtggggtgagttaacttattccagccaaggtgaaggagttgccccgggcttcactctgagacttggagcctagtgtgctaagctcccagttcccaaagtgaccattcccacgctgaatgtcattactgcctcatcagcagcttgtcagctgtaatttctaatcccaagccgggtctctcttcccaggaccaaagtcataaagatgtttgcccttgcacgggtgtttgacatgtgctaggccatatttgtgcatttgtcttagggccctcttgagggcttagcacttctctctgacccaggcaagactttatgtgctgtgcattcctcctgaacatgatgtcatgcttgtgcctcaccatggaattctgcagccaggcactggggctcaagtccaaagacgggaagacttaaaaggctcaaacaagcaaatgtttgtcattatttaagattttaagacaactgaattctgaaatgtttatggtcctggcctcctttgtgggtcatcaatgacctcttcccttttaggaggtatctcatggagagggcgtcttggcctgctcccctctggggccactaactcacaccagagctgactcaaccattccaggggaagattggtaagaagtttattcaccagacatgtctagctgaaatgaatgaaatcaaactcagcagaagtcaacacttagcacggaaggcaaagtagagacaaagggtcacccggctgctgcacaccggcctttagctttagctcaagttgttctgctttaaaggacaatgccaatcatctcataagtaaatgaagacaatgattcaacagtgctgtcaagtttgagagaaaagagaagccatccctacacccaacacttaatatattgttaggcttggggtgggttgcccagtgccttctgggatgacctgtgctcttttcttttatccaggagcaattagaatcaatctgcttcatctggaagttctgcccaagggtctggcaccataggaagttgtccaggattattttaaccctgttacaggatccaagtaattcctgatatgtatgaatgtaaagcccattcttgtattcagcgtttctcagtggagatacttttgacattttgggtgggatgaatcttccttatgggagtgtctccagcacacaacagggcacagaatgcaagtggtgtcctcctctggtcattgtcacaaccatccacccaccaatgcacgcactcccaggcaccacgtggtgggtggcactgcccccactgagcacattgcaagcttattgccacagaaactagaatgctagtactacccatgggagcaggcagcaggcctgttctttatttatttcactctttgattctgcagacctcagatttacccactgttattgatctgtggaaggcttttgactgtccattttccccctagggtgagctcatataagtggaagagaagcaaagagatagctgttgcacagctgttccattcctgctccctgttgatctcctaatgttgtgaatacaccctaagaattctcccaggtgtggattaagacgacttaagccaggaggaaatttgccccaaggcaaagcatcctcttttccctctgcagaaactttgtccaggcaccctagcatgagggattgcctccccatctaacatcttcacacaggccctcttgctggacccacattaatggacggcagcttctgacttccagcaggccctctttcactttccatcgtctttctctgtctgtgttttatagcatgaggcactgaagttatcaggtgatcagagaagactagaactggatataaaccaacagatcatcgagtaacgtggctttcaacctccagacttcgaggtctattgactgtgaagatactggaggggactcaaaagctattatcattttctaaaatggtgtcagaactgttcgatgtactttaaataggactcacaggtgtattaaaatgtcaagttttcttttgcctaaaactgtatgaacgcggtgcaataactggttatttcaatgctgacaaaagttctgattgacagaacttgcactcattatatatcactcagtacctaattgatatgataattttgaaatcaggaagactgtggagagagattagtaagaggtccttagtggtaaaaggactaaggaaattgtagtccgattgtctctttcttcaaaagttgaggcccagagatgttaagtgacttgctgacagttggatgattaatgccctagaactatggtggccatgccacaccagtacagtccctatgtgctcctgttgtcccagcatcatcaccagtaggaatccctgtcgctctcaaaagaaatccagtttgattaataagttacatggtcactctacctaaaacccaagtctccaactgccaattcatcccttttctcaccacacaactctacctctttctctctttttcctggttctcaaaattgtttctcctatctgaatgcatctcttatgttttcacaagtaagtcatcctcaaagtttgggcgactataaatgacagctccaaatccagatggcctgaaccgtgggaccttttgttcctgagtggagggggaaggaagatggtacggggcaggggcagctgggccccaggcaagcccagggccttgcccaagcctcagacagccacccatgtgctcctgtgttctcagtgacaaaggccaggaggggcagagggaagctggtgaatttttatgatttaaaaaatatgaatccacactggatagaaaaaaatacaatgtaaaacaccacccatgccgctctgaaagtctagaatgtccaggtgactccagaatggtgttcatagactttggcaatactttgaaaacctctgtgaacaataaaagttaagcatgagaaagaaaatatttcccataagaaaatgtaaacccttttccttgtctgccacatggggccaaacataccagtgtgtttaattggtagatcagtaccactctcaagaatttcttagatgccataaacacagaatgcaattttggtggagtcccacagcaagctataatcatgagcagggaggacctgggttcagcagctgtgctttattcctgtgttgctttgaactcacagcagagctaaatacccggctcataagaccttctgataacaaagtccagcggacttgggagaaacttggggttttttttgttttgtttttccttttttttttttttttgagatgaggtttttgctctgttgcccaggctagagtacagtggtaagatctcggttcactgcaacctccgcctccagggttcaagagattctcctgcctcaacctcccaagtatctgggattacaggcatgtgccacgacacctgtctaatttctgtatttttagtagagacggggtttcgccatgttggccagactgatctcgaactcctggcctcaggtgatccgcccgcctcggcctcccaaagtgctgggattacaggcgttgagcctctgcacccagccaagaaacttgttaaaatgaaaattgggtctatgtagactgggagattaaaaatgactcctttttaatgtaaggaactttgctttactgtttcattaaaaggtttgccagtgcaaaccgaaaatgtaggagccctttttcaaaagcaggaacaaaaacaacctctgctgtgaaaggtactaaaataaaagccgctttttttcttctgcagtctctcttttgacttgtcacaaggcttttaaaatcattcttattcgctatttaatgccactctaagtaaaggaaaattaaaattttaaattgttagcatgaatcttaccattcatctttatattgtgcaaagccagctttaaacgaaaatataagagcatttaatttgtatgctaaattgttccaaatgatgcaatttgcatatttcattcttaccagaacagtggaaaatgctgcacaaaactaattcaatgcttttatttcgcttctcaataatgcacattctttttttttttttttgagacagagtccctctctgtcacccaggctggagtgcagtggcatgatctcagttcactgcaacctctgcctcctgggttcaaatgattctcatgcttcagcctcccgagtagctgggattacaggcacccggcaccacaccctgctaatttttgtatttttagtagagacagggttttgccatgttggccaggctagtctcaaactcctgacctcaggtgatccaccacctcggcctcccaaagtgctgggattacaggcgtaatccaccgtgcccggcctgatacatgcacgttctatcaatgctctctacctttggcttactgacaagtaaggaagaatttaaaaaaggcctatgggttgccttatctttctatttctttctgtgtcttcattttcagtttaagttgtttgcaaatgcaaagaagtaacatgagtaagaaaggtcaaaccaagtttccttggtcatatgtgtttcttagaataccactgctgcctttgtgtttgaagcaagttttggttttcaaatggaaagtgtggcctctcagggctgtcagtgtccctccccctccccagctaactcatcatagacaaaacacacttgggagtcacttagaagcttcatgaactcccacacattgtgaatacaccagaattctgagttcatggcgaatgctccatgtgaatagggtgacaagaaaggacaggcacacgtatctcctgtgtttctgctcattccatgctgtctcatcagaagtcacttacaaaatacaagtttcaagaggaaattattacaattttaatacggtggccgcagagcatgaaacccatcaagaagtccttctgagcaccaagtcctatgcaagcacacaggtgacgtgccatgaagctggccctgcacgtggggtggcaccatgcatgaaaatggtgaagagatcccaggggatcgggcggtgcactgagaaggaacaccaggcatccagacctgcacacagggcagtgtgcacagcaggagtccagggcagccagagattcactaccagaggtacagcccgagagcacatgccatgccaggaaagaggagacaggcagagacaggaagatcaaagtggagggagaaaagccagattactggttaactaagacactcagccggcagtgtcaggagagagccacaaaatgaaggcaagggaatcacggaagccagatactagcaaaggggcatcggaaaccagtggccacgtggctctgatcccaagcactgagtgccctccccggcatccttgtggggctgtgaggttcgtttcatgtgtctggacgtggctcctcagcgtggtcttccagctcctctcatccctctaccctcttggtaaaaacaagacatcttctaggagtgaggcaacctccccgctgccctgtagagagccacacttctgcttttctagtgttctaagaatgcttttcctgatttatcatcgttaagaatgggtgggaaactagctatgttgaacatgtgacgtgcaaggtggttaatggtgatccaccaatgagcaggacgccaggaccttgtgcaactgggagactttgcaacaccacagcggaaggctgtccctcagaggtttgtagccacctaggggcctccttctatcacccatgactaagtcttctgcattagcttagagcagtgtttttcagccttgaaaccatgaacatttggggccagacagttttctgttgtggaagactgtccagtgtaccgtaggatgtttagcagcctctctggcctctgttcactgcatgctagtagcaaccccctttccctaccctgtgacaaaaatgtctccagacgttgctagatgctccctgtgggaaatcatcacccttggtgagaacctgtgactttgagcccatgagccctgcagaggatcatgtctgagaggacgccactcccaccacatgctcttccagctggaatggttgtctttgcagtgcctgcttttctgaaagtgtctctttattgctttggcttccttctagcactatattccccactcctgggcaagttagtaaggcctgggggtatagtaaagtcactcagtgggcaagtctccttgctctgtgttcatccaaagagagttagatcagccttgaaagtcactgcaaaatatatatatcctgaggcctacaaagatttttgtgagctcaccgtccctttgctaactctctagggcactgtgtactactatgtagcaagagctcaatgtttgccagccttgtcatatgttttgtctcttttaatcttcaaagagaaaaaaataactcctataacataacagcgtatctcctataacttataaaaaattcctataaagtagtattgactcccatgccgggaattaataagtaacttgcccaagaccacccaggtagtaaatggatttgaacttgggttttttggctgctggtctaagaccttttctatcaatgcttccctggcttcgtgcatgtaagaatcacctgtgggtgtttgcaaacaatgcaggtccccaggcctcgcccctagagccttggtaggcaggtttagagcaggccccaagaatcgggatttgaaacatctgatgaaacacgtcattccggtaatgactgtgcaggtgactgccccttgagtaacactgaactccattattctgtgcttcctggcaaaccatcagggaaggagggaaggagaaaagagaaaagagaggagaagggttgagagagattgaaagcactcaggctgatgcagggttgagaggagctggtttcctccttcctctctcatccttgcaggcttagccacatgtctgacaatggcaataccgtgtccaaaactccacacccacgagatgccccttgacctctcctgcctctgtgtgtttgggcagcctgggtgtgggttcccccagctcagtcctcaggtgccaggaccaaagctcccatcagtgaacctgactaattcacaaagcatttctttttttttttaagttctgggatacatgtgcagaatgtgcaggtttgttacacaggtatacgtgtgccatggtggtttgctgcacctatcaacccgtcatctaggttttaagccccgcatgcattagatatttgtcctaatgctctcccttcccttgcccccggcccaccaacaggccctgctatgtgatgtttccctccctgtgttcacgtgttcttattgttcagctcccacttatgagtgagaacatgtggtgtttggttttctgttcctgggttaattggctgaggatgatgatttccagcttcatccatgtccctgtaaaggacatgaacttgttcatttttacggctacatagtattccatggcgtatatgtgccacattttctttatccagtctctcgttgatgggcatcaattcacaaagcacttgcatcagcttcatttgattatggaaattagcccactaacattgcatttctttgttcacagatactttctaaaatccttggccttcgctagagactttcctggaaggtttgtctcccctggctagatcatgaaaaacctggatcagccttaagttggatatctggtcacttttgcttttaaatagtctggcaaagcaagaggtacaacacatcctggtttgatgtactttccagcaaaaagtattagcaaaacaataataatattcagagggctcagttcccagtagaattcagcacatactccagatctcctgaggttcaggtctagttgaagggaaaggaatgactgagatgagtttgagtttcagacttgagtttctcccagctcccttgagaggcaaagaaaatctgccgataaacacgaaacaaagctcattgtcctgctacttgtttgcaagcaattgtatgtctgtcctgcagacctcactgggctcacggcattttgaatagctttctgtgatgtaacgcacacaggttttcactcacactatgcgcagggaattcagctctcggagtcatgactacgtcatccttcacctctcaaaccatcgctgctggtggccttcgcttttatttgttaagctgtagcttcaggaaagagccaattccctccctccctcccttccttcctccctccttccttctttccctccctccttccttctttccctccctccttccttctttccctccctccttccttctgtccctcccttcttccttccttcctttctttgcccctccatttccctccctctttttctttcattccctatctccctcccttcattctctctctctctgtcatggttaacaacacatgcttcaacaggttttttttttaacctcttaagaggtatatggttaaaaagtctctttgctattcctgtcttgtacctaagccacctacccccaccccacccctgccatacacacattcatacacacaagtaaaccattggtactgatttgatgtttttccttccaaagtgctttcaatatatatgaaagcacatttgaatagatgttgtcagcccccaaatgacagcctgtaaaacacagtgctctgcatcttacacttttcactcaccattatatcttagagatctttccaaacgtaaagaccttgtacattcttttttatggcatcatagtactccagttgtatagattagcatcatttatgtagccaatcctctattaacaaaaattcaggttgcttccaatatgttgctgtcaccaacaatgttgtagcacgtagccctgcactatgtcttcctgcacatgtgccagtctgtgtgcagcataaactcctgaggatggcatttgaggatgagtggctgtatgcacctgcagtctggatagatacgaacaaatcgcttatcgtaggcaccgtgtggacctctcttccaccaatagtgcaacgggacctggcagtccctattgcaacaagttcctgaggctttcctgggataagaaaaaggcgagagagtatagaaggttatttaattagaagaccaggttccccctctcacttcccaagccacaaccatcaaaattctcaaacctgattctttatgatacaacccaagaaagatatatttttatttttaaaatcgtaacctaatgaattaggatttttttgactgtgagtaacaaaatacagttcaactcagcttggcagtggactgggggagaaagagcggcagggcgtggtcactgtaagaagaaggacacatctcatggtacagtaggcaggagtgcagccgtgctcccaggagggacagcatccaggagctgggagaccacaggacagccaaggatacagggcctgtcacccattgctgcttctatttggatcttctttcttgaaatatttttttcctctcttctattcaatcctcacaacaggtaaaggtggaagctcatagtgaccaaattcacagttggagacagactttgtgtgcatgtgtgcatgttagtgtgtatgagtgtgtgagtgtgcatgagtgcgtgagtgtatttgcttgttagtgcaagtgtgcaccagtgtgtgagtgtgcatgttagtgtgcgtgagtgtgcatgttagtgtgcatgttagtgtgtgtgtgcatgttagtgtgtgagtgtgcatgtttgtgtgtgcatgtttgtgtgagtgtccatgtttgtgtatgtgtgcatgttagtgtgtggcatgtgtgagtgtgcatgttagtgtgtgtgtgtgtgagtgtgagtgtgcatggttagtgtgtgcgttagtgtgagtgcatattagtgtgtgtgtccgcatgttagtgtgtgtccgcatgttagtgtgagtgtgcatgttagtgtgtgtgtgcatgagtgtgtgattatttgcttgttagtgtgagtgtgtaccagtgtgtgtgtacatgttagtgtgtgagtgtgcatgtgtgactgtatgtgagggtgcatgagtgtgtgtgagtgtgagacttgtgtgtatgttagtgtgcatgtgagtgtgcatgtgagtgtgtgggtgtgtgagagtgtgagtgcacaggatgcttttctgctttgattccccattcccagaaaagggcgttggccctgaacttggggccaggcacccagcctgggccaggcagctgtgaacagcagagcttggtcatgttgtccaagctgaaatgtgggtcccgctgttctgagtgggcagaagagccaggggaatcttttcaagccgagcagatattccacatggcatctgcacaaccacaaataaagttgtttatctttgtcactttaatattataacaaaagcattataaaaacaaggcagaaacataatgaactctaaggcccaataaatctcttggttaaatggccctcgtggtttctgaagttatcccagaatgggataatggcagaaatgaattaggtataaactggacaaattctcacctctcctgttgtttcttttcagccaatagtttcctaaaaactgggttatcagagacgctcttttagagtaaaacaattttttttttttacatttttaaaaacagagcttctctccaatgaatgtccagaaagaccatacatttcagggctggcctacaggacatatttcaaagtgatgtgtaatgtcattttagaagagtgagctgttttctgttgtttttttttaacttaaagacaaaatggccagggaaaaagctgccaagtctctgagtaatcttattgagggttcagctttctaagtatgaccttatgctagcaacagcccctgagtaacaagaaaacaagccaagctaggaagccttgtttctatgagacgaaatggtaagacagcaaagtctgaaggtgaattctaattatgtaacatgagtgagtcatcaacgccgtcagcgatcacagacaatgatgcagtgacccgccgtctccccacacttgcaaagcacagaggctgtgtttctcatcccccgctccacaccttcctctcacccctccttccttccttcttttctatttttctcttttcttttccattttgtgctgcattactcagggttctcagaaccaataagatacacatatatatttagaaagtgatttcttgtaagaacttggctcatgtgatcatggaggcaggcaggtcccaagatctgcagaatgagttggcaaactggggacccaagagagctgatggtgtggttcctgtctgcgtctgaggctctggaacccaggagagcggatcacatagctctagcacaaaggccagcaggtttgagacccaggaagatctgatatctccatttaagtccaaaggtgagaaaaagccaatgttctagttcaaagacgaccaagcaggaggatttctctcttgctcaggggaaggtccacctttttgttctattcaggccttcaactgattgaacaaggcccacctgcatcgggagggccacctgctttactcaatttactgatttacacgttaatctcatttcaaaacaccctcagaacacccagaataatgtttgcccaaatgtctggacatcctgtggcctagtcaggtggacgcatagaattaactatcacgtgtgccttcctgttctcgggtgcactggccacgcatgctgtcacccatttcccgtttatcatcttttctttacagccaagtttctagaaagagaagtctagactgtctgcagtttctcatctctcattcacaagtcaacccagcggcagttggcgcctgtccccatcattttcttgaaactgatctcaagaatctgcataatctaattgtcaagttctttcctctgttctttgtgtaataacgcaccatcctgaatctctccttcaggcctctcttctctgtgcggccctctaggagtgatagtccccaggatcctaccatcttcctatctatcttttttttttttaatttatttttttgagacggagcctcaccctatagcccaggctggagtactcactgctacctccacctcccagtttcaagcaattctccttcctcagcctcccgagtagctgggatcacaggcccgcacccccatacccagctaatttttgtatttttagtagagacggggtttcaccatgttggccaggctggtctcaaactcctgacctgaggtgatctgcccgcctcggcctctcagagtgctgggattacaagtgtgagtcaccgtgcctggccccctatctcatttaacaagctctgtctggcagatgttataagctctcttgctttaactgccagctctaggctcatgactataaaatctctgtcttcaacattctctctctctgaatctcagacttgggatatataactgcttacagattctctccccattggatagtctccacatgaaactggaacttaacatgccgcattcaaattcaccatttcccccgtagacttaattcttaatttcttctttctcagaatgatactagcatccatgcagtctccagaggttttatccaggagacatttattaccaacggctccgtctcccaccttgtaattcaaatcagttactatgctctttcggttctccttgctaaatatccatttcctctcctcttcactgtccctgtctccagcttaatccgaaccttccttataattctcaactggagtatagctttataatggatttctctccacctccatttcaactgccccttcaatgaattagtgactattttcagtgtgattcttatgcaagaaaatgtgatcgagttaattcccactgaaagcatttccaagcctaccccattgcctttaggatacaatatgaagacaattgcaacagtccaggagagagactgtgagctaagacagaggcaactgagatggagacacaggacagaatgaagggagctgggagatcctacaagctagaaatgccaagaccccattacccatgagacgatcagacgtgggagtgagagtaaagggagatgaaggaaatcctctccatcctgactttgatgataaagtgagtcatagtcttgttctctgagctggggaactctagatcctgactttcctcaaagcaaacagcaagtgaacttacttgggtggggcaccctgtctggggaagcaaagccttcaggaaactcaaaggtctgcgtagagatgaatcagagactcaataacgaagaaataaaaattaataccagatgggtgaaggaggcagttgaaagtccttgtaaatagtcagcatccaagagtgctgcagaagtggaaggtgccacaaacaatgctcttctgccaggagattcctaaaaatctgctggcaaagaccagagaaagaatcagagccacgtgcccagcaagacattacctaagctcaaaagggtttaaaggacttataaccctgccttttaccctcaattatttcatgatcaccaccatgccctttttcctggtcaggtggttggcagtagtttggaataccttgctgtttgtagaacatgttaaagcatgaattatttgttgctatgccttctgggtgcatatttggatgccctaacagatgaactaatagctcttttcatctcactctctttattgagtcttgcccatttacaacaaaggagagacttgttttgtagatctttaaaacacacctgaggattttgaattcatttataagccaatcccctccagtgatcattcagtaagaaccaaagtcatttgcaaagctatacaccaacaacatttaaactggttaaattgagccaaaccacccaatttggctgttcagccaaattcaagtatgtccaatgcattgggatattaaatccccaacaaattcttctttggcatggcctgacaagatcactggtatttattggttgcttttatacaaatggaaagaaatatatcataaccaaaaagttttcacaggcaacctcattagaatcttgcatgggacccaagagtgggctgaagaacacagtctttcctgccaaagagcagccttttgctctgcaagcaggtggctgatgggctgttttatgaagggtttaatgatctctgtctgccttagttacctaccaaaataaactgtgtgaatcccaacgtggtagaaggactccctcattaactgtcaagcaaaatcttggtagggctccacagcctgaggaaataaagttgctaaggaagacaagtcagtgattctgtagtttctacagacctctgcttcagatactgttagcagcccaggaagtagttctgttggctgcattgatcctgggcccagaattaccctaaggcagaaccatcagggagacagagctagatcagtctccattcccctaggacactactcatttggcgacaagctaaccagagagcttcactcaatttataatattcataactgataaaggccttttctggtatcccactaattatatatccaggttataacctaaataagatacaaaactgaggatgcatttttgtctgatctctttatttgatgcctgaggaaactgagactcaggaatggctgaactgcctgaagttgcacacctgagagtcgagcccaggtctcctgacttgcaggccacagttcttcctgctgtgaataccatcatgtgctgccagctgcacatggttgaatgggagttacagaagtttggaaaacctgggtcagatatcagactagagaaacatccaaagagagataagaaaaaacatagactggatggtccacaagcctcagtgtaggaaatgaagtggattagccaggaaatcaggaacctaggctgttttgagggggcataaaagctgccttgctcaatcatgcttatttcaatctatagagagaaacaccctacaggcagaagacctgccatttttacccatgcttggtccaagagtacgccttccttcatccatatttctagctttctccccacccactcctttctttggaaggaagttattttcctttcctatcactgaaaattctaacagagccccactgagagtcttcttcatcctacgtcctcatttaaagccaaattttactgagcacttactatgcaccaggtgctgagctggggtaacaaagatggagcagccacagttataatccacaaggatctcctcatccaaaggtcctgtttatgtagagtgcttgcttgcaccatgtggacagtgagcatacttctaaaccccaaatctcaacatatggtccaagaaaagcctgcttttctaatttgcgaatgttttataagggtgtctttaaaaggcttacaaattgaattgtgttagtaagtcctataacaagttcctttactagaaaaaaataaattttattaaatcaggatttttgagaaaaatctgtgctgtgtgttctccaaatccatatgttttaacttgtaaaacctccctataatcacagtctattgcagttgggaaggatctgaaatgtcacctaatccagaagatgtaaattttttattttttaacaatgaaacaatttttaaaaacaaatattaccgtgacttccaaaataataaaagaattaaaattggcacctttctcctaaaaaatgagcttgtttactcttcccgtcgcaaatgaggaaactgagatccaaagagagtgagaggtcaaaggtctcaaagaaagttacttgcagagtgagggtaggaacataggatcctttcctattctctttccacccatccatccatccactcatccatccatccatccttccattcacccacccacccatccatctattcatctatccacccatctatccatccatccacccattcacctatccatccacccatccatctattcattcatctgccatccatccatctatctacccactcatatatccatccatccatcattccattcatccacccacccacccatccatctattcatctatccatccatccaccccttcacctatccatccacccatccaccatccatctactcagccatccatccactatctatccacccatccatccgttcattaatccacccatccattcaacaatccacccaattttctattcatccatccatccatccacccaccatctatctattcatttatccatccatccatccatcatatatctacccattgatccatccacccatctagatattcatctatctacccatccaccaaccatccatctattcatccatccattcatctacccatccattcatctacccatccatctatctacccactaatccatctatccatccatccacttcacaaaccttcaataagtcctaggggtcctgcacttgaaaaacaggtagacagaggccagaccatgcatggccttatgagtcaccttaagaattttggacattgtcttaagaacaataagaaagacattgcagtactttttgttttgcttgggtttagggattttcttttaaaaacattttattgtagaatgtttcaaaagtagaaagagtagtatcaattacctagcttcaataattctcagcacatggaaaaccttgttttacgtctccccactttccccaccccactgggttattggcctgcaaatactcagtatgaatcttcaaaagacaaagactctttaaaaatatatatatatatatataatatatataatataaaattataataccattatcaaacttaaaacatttccatagtaattccataatattaaaatttcattagctgactaaaaagtttagagattgggaactcacatgacacagttgacattttagagacatcagctctggctacagcatgaagaaagggttatagagagatgagccaagtctcaagggccaatgcagtaatccagatgagaatggaagtggcctgaacatgacagcagtagggacagagaggaatggagaggtacaagagcactgcaggaggcatcgtcgagaggacatcttgaaagccatggggaagatagacaatggaaaccattaggatgaggccatggggaagatggacaatggaaaccattaggatgaggcccagcatctagtgtgggtggtggtgccattcactgagaggagaccaaagctgaaaatatccatttggattaacagatggggtgtgtcttttggagaggtggagcacagggtgggagaggggcatcacggggagctgtccagggccagctggagagaatgcttgggctggagagacaggttcaggagtcctgaagctgtaggtggaaactgaagttgtggctgcaggtggtgaaagtagaggaggctgaggacagaactggaggctcagtgccatgatgggaggtgaagagaaacacccagacagactagcaccaaggaaagagcatcatttaaaaggggaaacgtggtcaatggtgtgaaatcttgcagagatgtcaagtaaagtcagactcaaagtgggccactgggtttaggaaaaaggatttagagcaagggatgttgggaagagcccggttggtgagggagagaaagcaagcaccagactgtcaccagtgaaaacggaggaactggaatttcttctgcgcccgacccaaagtgctaggattacaggcgtgagccactgcacccgacccagtctgtaatattttattatggcagctctagcaaactaatacagccaggcactgtgattaacatgttacttccttctttttatttaatattcacaaacatctcatgaggtaagtgctcctgtatctccttttcttgatgaagagattgaagcttagagagggaaacaaactaacttgcataagatggaaaagtcagtaagcagaattctaatgcagtttcccagggatgctgtcacaaagcaccacagactgcagggcttaaacagaaatcgatcgtttcacagctcgggaggctgggagagaccaacgggtcggtagggttggtggcttgagagggctgtaaggaaagaatctgcccatgtttcttcatatcagctttcctctccgtattgctcctctttataaggacatcagtccagttggatgaggggcccaccctgctctagtaggacctcatcttaactaattacatctgcaatgactttatttccaaataaggtcccattctgagatactgggggttaggaatttaacatatgaatttgggggtacacaattcaatcctcctgccctgcctggatgaaggccgtgtgagctgaaggactcagtcagctaggggaaaacctgacttcagggtcttaaaggaaaggggtgactgctgggagcaagtcaggagagaggtcatatatggagaaaagtcccatagaaggcaagacaggatggcattcagtggcaggtgacaggtggagggattcacttgggcatgagaggacacattttccttattgttacaaggatgagggaaggaaaaagggatgagttgaaatgtgaagtcaatctgcagatgtggaggagggaagttgaggaagttcatttcagagggcgcctgctttctttgtggagcaggtggggagactgcctactgaggttaacagcagggtttaagattggggctcagaagaaagacagcaaataaaaccagagacattgaaaaacatggggaaagtttgaaacatccgctgtgtataaactgcaacagcctgctgtttctagactaggccccattcaatgtagcattgcagaagataatctactctcattttaattagaaaaataggagaagaggagggtgagctggccagggaactacagaaggctgcctgacagtaacaagggtctagatggcattggtggccctgaggttgcagtggcaccatctgcagggtgtgtggttttgccagccatgctcaatagctgggcgattgatgcagagtaagtaaacagttgagttcatccaaagctgggctttggccagggcaatgcattaaaaggacaaacggcaaggaggttgagcatattggcaagaggagggtgaagtagggaagctcaggggtttcagtgggcagagagggaagtgggcatgtgaggaggctgtggctatttctgctgaagaggcctgctcatgccccttgctttcggagcgcatggctgttgctgcttcctggaggaacagatgctgccagatgtgccatactaatgagctgcaggctgacaggctccccagatggtctccctcctctgcagtggtcctgactggtcccagctgggcaattcagcaatttgtgctcagtgctgccacaacgctcagagcatgctctggggacacacacccctgtgaaaggatgaggttggtaccagctgccctcctagtggcgtgtcgatgtatcccctggatcagtcagctcatttctctgttactttaaaatgcagtatggagtgactctgtttacatcttggattttattgctgtaatcttctaagactaccaatcttcccttagctgccatatttcaaataaaaactatggatattattataaatattattgatattactattctatacctctactgatgttattagcagtcaacttgaaactccaagttaccatattcacttcagtatcttcatatacaaataaaggagaagaaaaacccataaatgttttagaggggtggtgacacactaatgttattcctagtacaaaatggtcaacatttaaaaaaaatactaaacattgtcagaagcaatgggagctattataccttgttgatgagaatatcgattgatacgaccactttggaaacagtttggtattttctgttaaagctgaaaacaaagcaggcaaggttctgtgagcctgtagtcccagctactcaggaggctgaggcaagagaatcccttgaggcagcctgggcaacacaaagaaacaaggaaggcaggaaggcagggagggatggagggaaacctatcatccagcaattccacataaacacaacagaaacagataaagatctacgtagcattattattcataatgggctagtactggaaacaacacaattgtctgtgaacattattaataggatggaaaaatgttggcatatccatacagtggaataccatacagcaatgcaaattacaaactacagctacaggcaataacacagatgcattgctcaaacctaatgctgagtgggagaagctgacacaaaagatcatatgctgtgatccatttatccaaagtttaaaaacaggggaagtcactttattgtataggagtgccaagtgacatagtaaagcacagagaaaactaaggagggaatgacgagaacagtccaggtagtcacctgtaggcaggcccaccgttaacagacaactggcacattcagtaattgaggacacataagtatactttagacgctgctttgcttatatacaaataaaaatctgcaatatatatcatatggaattattcttttcctttgacatcacttcaaaatgtatattatctgattcttatcatgagtttaaaacaaaggatcaatgcctgatattctcccaaataataaattatcaggattccttggagcatgacaaaaaacaattttttgtggggcttaaggtagaagtacagatggagaactgcatattatgggtctaaatattgtaaaattataaattaaactaacaagctgttaaataaaagatgtcccggccgggcgcggtggctcacgcctgtaatcccagcactttgggaggctgaggtgggcggatcacgaggtaaggagattaagaccatcctggctaacacgatgaaaccccgtctctactaaaaatacaaaaaattagcccagcgtagtggcgggcgcctgtagtcccagctactcgggaggctgaggcaggagaatggcgtgaacctgggaggcggagcttgcagtgagccgagattgcgccactgcactccagcctgggtgacagagccagacttcgtatcaaaaaaaaaaaaaaaaaaaaaaaaaagatgtcccatcctcctacttggacaaatgtctcttcatagtgacctgagaaaccacgttggaccttagaattcttggactgcttgggtcttcctgctgtaacatgtgccacaggaagaagccacccctagacccagccatctacccttatgccccagccctgctccatcccataacccaagggccttggtgctcatatgtatcactcttgagccctcaagtctaccttcacccatggccttttacgaatatctgcttccaggccccccgtcaggaataaggacttaaggaagagcccacaaagaccaggaagtaggtttggaatcgtctgaacaggaagtcccaatgtcctggtccttggcacggggtctagaaagggagacatggatctcgggtgggcatggtctcttggccccacagacctctttccccttgagaaagttcatggctggaggacagccagaagcccaaaagcacaaggcccaacacagagaccccggtgcatggggtaagggtagtaccaccttaatgggaaagagaggggttgcactggaaagggctcttggaaagcttctggagtcctggcagtactctatgtcttgacctgggtggcagttaaatttataacaatttattaagctatacatttattttatacagttttctatatgtgtgttatatttcccagtaaagaattaatgacatgtgtgtgtgtatatatatatatataatttctggtactgtagtttatggtatccccatagacaaatcagctctgagaggttgtcttataagcacagacaccttgggcagttaaaatgcctcaaggtgtgagtacctaaagaagcaatagacagacagggcgctggaaacgcagtaaatctcccttttgtttctccatcctgtgtggggccaagacactggggtaaccacacatgggttcaggcagagcaaatgagtcatgggcctgtgtccccttgcctagccactgcaagtgcctcagaggaaaattcctttttcccccctcttagccaagactataaatactgcgtttatcaaactgaaattacaggaggctgttcccatcctggtagaagtgaaaggagaccaactcccaattatcctgtttggaaaggagttctaggaggacttctcttcctcctaagggcagctgcataggttcattaatttttttgctgagcttctattatgtgccagacactcttcttatttttctgcttccccttttaaaacaacctcttacttattcttgataggaaaacactgtccttttacaaagattcacattaccaattctcaaaaagatattcacgtgccccgtgtggtttaaatatcagggtttttctaaggatatataccccaactatagcctacaaatacatacacatacatacacacacaccatctcaaaacagccttacagctgcaagatattgaaagagagtgaaaaattggccagtactaactcaccgaaagcccagtccatgtttttcccaaaaaatcaaattctgggctttgcatctaagctatttaaaagccacatttccaaaacactagtttttctccttttctggaaacaagaaaagcatatggctccagtgaccttcacaagctgctggtaagaggtagagtcaggcacatcttgtggcttcaaaatgataaaagtggtaacatattaagttggtataaagggggatggtggggcctcagggatgggagagtagaaaacaatcaatgaaatcaatgacaagactaaaactgtaggttataggcaaggaaatttcactctcacctctactatccatacaaaacatctggcaaacgtctacccatctctcaagactccacccaagattgaccttcctttgtgccctcaccagacccactgcacatttgacccgaaatgatgtaacattttattgtgctgtatttttgtttgttcagtgagactgtgggatccttgaggacaggactatattttatgtgtctttgaagttccaactaaagcatagtaagaaccccataaatgctttctttgattgcatgaatgaatggatgatggattccattcacaagactatggatttggcttttccagctgctatgatgcaacccttaaatgatgaaaagcatctcaatttttttcagatcttaccaacctttccatctctatctcctgttttcagattcagtaagctgtgaggtccgtaatgtcagacactggcaaacatcatatgttcttcaagtagagttatgaaaacgaagaaactggtcagaagagtaaaacgccggaattgtcctttccaacatccagagctgcatcattccttggggcaaaatgtggacaagggtgagtactgatagaaaaaaacagacaatttgtgattcccctttttccagtttgctcagcctaaattctctgcaataataatacaaatcatgtttttttgtcatacgggcctgcaactaacatttggggaaaatactgttaagtttagactgccagattttgctgttaggtgaattttttacatggatgcactgatgcccacagggcatcctattccatccagaaatctctggggaagcagtcttctgggatgcagatagattattccacttaacataatggtgcccgagcaagcctggaagttacactcactgaactattcattcagaagctgattgcccacgtttggaaatagccagttcttggtgccttgtttctctgtttgccagtcaccttcaaccattcaacttccattcggccattcctcaagaaaatcaagttggcctggagtagagtgtaggatgaaaataatcaatttttctatctaaccaaggcttcctaaaggttttatgaaaattcagtagaagaaatgatatgtaattttacctattagttggcctctaaaagaggcaggcatcatcgcatggcatagtggcattgagggtcacaaagatctgaattttggtccttgcttttctgtttagtagtagagttgacctggagccagtgacctgacccttttgaatctctgtttctgtgtttataaaatggtgacaggaagattgttcagaggatgaaatgagaaaatgcacatagagtaactcatgctcaaaatgaaaaaaggtaaattcccttatctattgagatcgatcaactgttttctgtatctcagagaatcaaccatcaactgcacacaaataaaaaagctctgggcaccgtatcaagccaagaacagcccaatctcctttctgggcaaacgttccaaggtaaatataataagaaatgctttctttaaataatttgataagtaacaaaaggatttccctggaaggcattaaaaacaagtttgattgtcatatcactgtgggtttttttaattatattttaagttctagggtacatgtgcaaaacgtgcaggtttgttacataggtatacatgtgccatgtgggtttgctgcacccatcaattcatcatttacattaggtatttctcctaatgctatatctcccccaggcccccacccactgacaggccccggtgtgtgaggttccccaccctgtgtccatgtgttctcattgttcaactcccacctatgagtgagaacatgcaatgtttggttttctgtccttgtgatagtttgcttagaatgatggtttccagctttatccatgtccctacaaaggacatgaactcatccttttttatgactgcatagtattccatggtgtatatgtgccacattttctcaatccagtctatcattgatggatatttgggttggttccaagtctttgctattgtgaatagtgccccaataaacatacgtgtgcatgtgtccttatagtagcatgatttataatcctttgggtatatacccagtaatgggatggctgggtcaaatggtatttctagttctagatccttgaggaaccgccacattgtcttccacaatggttgaaccagtttacactcccaccaacagtgtaaaacccttcctatttctccacatcctctccagcatctgttgtttcctgactttttaatgatggccattctaactggtgtgagatagtatctctttgtggttttgatatgcatttctctgatgacaagtgatgagcattttttcatatgtctgttggctgcataaatgtcttcttttgagaagtgtctgttcatatcctttgcccactttttgatggggttgtttgtttatttcttgtaaatttgtttaagttctttgtagattctgaatattagccctttttcagatgggtagactgcaaagattttctcccattctgtaggctgcctgttcactctgatggtagtttcttttgctgtgcagaagctctttagtttaattagatcccatttgtctattttggcttttgttgccattgcttttggtattttagtcatgaagtccttgcccatgtctatgtcctgaatggtattgcctaggttttcttttaggatttttacagtgttaggtcttacatttaagtatttaatgcttctagttaatttttatatacggtgtaaagaagggatccagtttcagctttctacatatggctagccagttttcccagcaccatttattagatagggaaccctttcaatattgcttgtttttttcaggtttgccaaagttcagatggttgtagatgtgtgatgttatttctgaggcctctgttctgttccattgatctatatatctgttttggtaccagtaccatgctgttttggttactctagcttgtagtatagtttgaagtcaggtagcgggatgcctccagctttgttcttttaagtagttttttccaattacgtaaagaaagtcaggtagcttgatggcgatgacactgaatctataaattaccttggaaagtatggacgttttcataatattgattcttcctatccatgaacatggaatgttcttccatttgtttgtgtcctcttttatttcattgagcagtggtttgtagttctccttgaagagttccttcacgtcccttgtaagttggattcccaggtattttattctttttgtagtaattgtgaatgggagttcactaatgatttggctctctgtttgtctattattggtgtataggaatgcttgtgatttttgcacattgattttgtatcctgaaactttgctgaagttgcttattagcttaaggagattttgggctgagacaatggggttttctaaatatacaatcatgtcatctgcaagcagggacaatttgacttcctcctttcctaattgaataccctttatttctttctcttacctgatttccctagccagaacttccaacactatgttgaataggagtggtgagagagggcatccctgtcttgtgccggttttcaaagggaatgcttccagcttttgtccattcagtatgatattggctgtgggtttgtcataaatagctcttattattttgagatacgttccaccaatacctattttattgagagtttttagcatgaagcgctgttgaattttatcgaaggccttttctgcatctattgagatgatcatgtggtttttgtcattggttctgtttatgtgatggattacatttacagatttgtgtatgttgaaccagccttgcatcccagggatgtagccaatgtgatcgtggtggataagctttttgatgtgctgctggattcggtttgccagtattttattgaggatttttgcatcaatgttcatcagggatatggcctaaaattatctttttttgttgtgtctctaccaggctttggtatcaggatgattctagcctcataaaatgagttagggaggattccccttttttctattgattgaaatagtttcagaaggaatggtaccagctcctctttgtacctctggtagaattcagctgtgaatctgtctggtcctggactttttttggttggtaggctattaattattgcctcaatttcagagcctgttattggtcaatccagagattcaatttcttcctggtttagtcttgagagagtgtatgtgtccaggaatttatccatttcttctagattttctagtttatttgcatagaggtgtttatagtattctctgatggtagtttgcatttctgtgggatcagtggtgatatcccctttatcattttttattgcatctatttgattcttctctcttttcttttttattggtcttgctagcagtctatctattttgttgatctttttaaaaaaacagctcctggattcattgattttttgaagggttttttgtgtctctctctccttcagttctgctctgatctttgttatttcttgccttctgctagctgttgaatttgtttgctcttgcttctctagttcttttaattgtgatgttagagtgtcgattttagatctttcctgctttctcttgtatgcatttagtgctataaatttccctctacacactgctctaaatgtatcccagagattctggtgtgttgcatcttttttctcattggtttcaaagaacatctttatttctgccttcatttcgttacttacccagtagtcattcaggagcatgttgttcagtttccatgtagttgtgtggttttgagtgggtttattaatcctgagttctaatttgattgcactgtagtcagggagagtttgttgtggtttctgttcttttacatttgctgaggagtgctttacttccaactaagtggtcaattttagaataagtgcaatgtggtgctgagaagaatgtatattctgttgatttggggtggagagttctgtagatgtctattaggtctacttggtgcagagctgagttcaagccctcgatatccttgttaaccttctgtctcattgatctgtctaatactgacagtggggttttaaagtctcccattattattgtgtgggagtctaagtctctttgtagatctctaaggacttgctttatgaatctggttgctcctgtattgggtgcatatatatttaggatagttagctcttcttggtgaattgatccccttaccattatgtggtggccttctttgtctcttttgatctttgttggtttaaagtctgttttatcagagactaggattgtaacccctgcttttttttgctttccatttgtttggtagatcttcctccatccctttattttgagcctatgtgcgtctttgcacatgaaatgggtctcctgaatacagcacacccatgggtcttgactctttatccaatttgccagtccgtgacttttaactggggcatttagcccattttcacttaagattaatattgttatgtgtgaatttgatcctgtcattttgatgttagctcattattttgcctgttaattgatgcagtttcttcatagcatcaatggtctttacaatttggcatgtttttgcagtggctagtaccagttattcctttccatgcttagtgcttccttcaggagctcttcttataaggcaggcctggtagtgacaaaatctctcagcatttgcttgtctataaaggattttatttctccttcacttatgaagcttagtttggctggatatgagattctgggttgaaaattcttttctttaagaatgttgaatattggcccccactctcttctggcttgtagggtttctgccaacagatccgctgttagtctgatgggcttccctttgtgggtaacccgacctttctctctggctgcccttaacattttttctttcatttcaaccttggtgaatctgacaattatgtgtcttggggttactcttcttgaggagtatctttgtggtgttctctgtatttcctgaatttgaatgttggcctgccttgctaggttgaggaagttttccaggataatatcctgaagagtgttttccaacttgattccattcttcccgtcactttcaggtacaccaatcaaacgtagatttggtcttttcttatagtcttatatttcctggaggctttgttcatttccttttactctttttttctctaaacttctcttcttgctttatttcattaatttgatcttcaatcactgatatcctttcttccacttgatcgaataggctattgaatcttgtgcatgagtcatgaagttctcatgccgtggttttcagctccatcaggtcatttaaggtcttctctacactgtttattctagttagccattcatctaatcttttttcaaggtttttagcttccttgcaatgggttagaacatgctcctttagctcagagaagtttgttatcacagaccttctgaagccaacttctgtcaactcatcaaactcattctctgtcccgttttgttcctttgctggtgaggggctgcaatcctttggaggagaagaggcactctgtttttttggaattttcagcttttctgctctggtttctccccatctttgtggttttatctacctttggactttgacattggtgacctacagatggagtttcggtgtggatgtcctttttgttgatgttgatgctattcctttccgtttgttagttttccttcttacagacccctcagcttcaggtctgttggagtttgctggaggtctaatccagaccctgtttgcctgggtatcaccagcggaggctgcagaacagcaaatattgctgcctgatccttcctctggaagcttcgtcccaggggggcactcacctgtttgaggtgtctgttggcccctactgggaagtgtttcccagtcaggctacacaggggtcaaggacccacttgaggaggcagtctgtccgttcttggagctcaaatgccatgctgagagaaccgctgctctcttcagagttgtcagacagggacgtttaagtctgcagaagctgtctgctgccttttgttctcctatgccctgaccccagaggtggaatctgtagaagtagtaggccttactgagctgtggtgggctctgcccagtttgtacttcctggcctctttgttttcactgtgacactttgtttactcaagcctcagcaatggcagatgcccctccccccctcaagctgcagcgttgcaggtcgatctcagactgcagcgctagcagtgagcaaggctctgtgggcgtgggacccactgagccggcacaggagggtatcttcttgtctgctggttgctaagactgtgggaaaagcacagtatttggtcaggagtgtactgtttctccaggtacagtctgtcatggcttcccttggctaggaaagggaaataccccaaccccttgcatttccctgatgaggcaatgccccaccctgcttcagctcaccctccatgggctgcatccactgtccaaccggtcccagtgagatgaatcaggtgcctcagttggaaatgcagaaatcacccatcttctgcatcaatcttgctgggagctgcagactggagctgttcctattcgtccatcttggacaatagcccgcttactgtgatgttttaaggtcaaggtaatgacctcttaacaatcctcgctagtactagattctatggcaaaagtctgtcacagaactggatacttcagaggcttccaccaaaccaaattagtaatccaaactggaacaaactatatttatttgtgaattctcaatccattcaatataaataccaatttctctatgaatagtgaaacaaaaaatgtctctcttctcattttttatacctactcagccaacattactaaactgagacaaaaacagagagatacagggagataaaacattccctgaagcaagtcagtatttcattccagctgtaactctgcaattaacattagttctatggtatttccaatacatgctgattctcaacttttggaattctaaacctaaaaaccatataatttcaccacctcaattttttaatttgctttagaattatctatgttgagtcaaaagggcctttgaggtctttaatttcatgacttctgggtgattttttcccccattattaaactttattttaacttttcatacacacagatacacacactcacacacacacatcacttcacactacgcatacatatattcctactgctctttttcaggtaggatgctggttaaaaatatggactggggctgggtgcagtggctcatgcctgtaatcccagcactttgggaggtcaaggcgggcagataagttgaggtcaggagttcgagagcagcctgaccaacagagtgaaaccccatctctactaaaaatagaaaaattagctgggtgtagtggtgcgcacctatagtaacagctattcagaaggctgaggcatgagaattgcttgaaccccagaggcagaggttgcagtgagctgtgattgcaccactgcactccaacctaggcgacaaagcgagactctgtctccaaaaaaaaaaaaagaaaagaaaaaaaaatacggactagaagccatactgcctagtttgaatcccagtcttgcctctattgagtaatagggccttgaacaagttattaaccctctttgtgcctcagtttcttcatctacaatatgagaatgagaatagtaccgacctcaaagggtttgtgatgattaaacatgcatgttgcttagaattgtgtttggcacgtactaagccctcaaaagaagcttcctgagttttatagcacataaaaagtcaagtcagtgcagctaaaagaaatcattgaagggagaagatgagagacacagagcataatgaaaggcctggtgggagaatgagccttgggaatctggatggggctagacttggtcactcacctgaacttccttaagctgtgatttttctggttccagaggtgacaatgaagacaccatgagtgaaggcatggacagaaaaattcactggggaagcctgtgctaaactcataaatactcttaaaagtaaaccccttacaagaagcctcagcaaataaaagcaagccctgagggaactgcactaatatcagtgtgaggaggaaggcggagaggtctcctcacacctggagagctgtccctggctgcagagaggctggcaccctgcagcattcttttcccaggatggttctgttttatttcattttcaaagagctggtagttaaacatttaccattgctccactgaagacaataaagaataaaggggctggctcagaaaaaaatgaaaaccaaaaaaaaaaaaaaacaaaacaaattaaactgcaaagctttttcacctttgcattagggcaggaagcctgcagccaggcatggcatgttatagtttatctaaagaaaaaaagccaaatcggctgggcgtggtggctcacgcctataataccagcactttgggaggccgaggtgggtggaccgcctgaggtcaggagttcaagactagcctgggcaagatggcgaaaccatgtctctactaaaaatacaaaaattagccgggcatggtgatgtgcacctgtaatcccagctactccggaggctgaggcaggagaattgcttgaacccaggaggtgaaggttgcagtgagctcagatcacgctactgcactccagcatgggtgatagagcaagactttgtctcaaaaaagagaaagaaagaaaagaaaggaaggaaggaaggaaggaaggaaggaaggaaggaaggaagggaaaggaaaggaaaggaaaggaaaggaaggaaggaaaggaaggaaggaaggaagaaagaaaggaaggaaggaaattttgccattctttcccactaaatgcaagttcactgcagttccaaggtacttatccacaccgtgtatttacatctgcctcaggtttgtagtaaatgctgtaaacagagagatgtgatgaagagaggtaatgcatattctttatcacctctctaaaaacatgattatcctgacctattgtagggaatatgaaaacactatgtagtgagaattaccatcctgcttcattatacttaaaagagaatttaacctgttcagatttctgagttgttccttaagtataaaagtgaaagaatcaggatcaaaacgaagaacctctaaatccgcctattgtatctgcttgggctgccatgacaaggtatcacagagtgggggcttaaacaacagaaatttattctctcacagttctggaggctggaagtccaagataaggtgtctgcagggttgatttctcctgaagcctctctccttgacttgtagaccttcatcttctccctgtgtggtcttccctctgtgggtggctgtgtcctcatctcctcttcttataaggactcctgtcatattggattagggcccacccatgtgacctcattttaacttaattacttctgtgaagaccctatctctaaacacagtcacatttggagttccttggtgttaaagtttcaacatgaatttggggtgggggtcacaattcagtccatcacacacctaacgtgggtgtaatgtgtctacaggaacagtttgattgagcaacaccacaggttgcattcccagagaagcaaattttgagatggagattggcatgctggaagtttgtggagagtgctcctgggaaactgtcaaggcaagagaggaagcaggattaggcagaggaggaagctgaaatcaggataaagaccccagcaagtcacagaggccctccaaagctgggatgtccttccatgttgtctgaactgaggcaaggtagttggaagtttatgccccttcctagacagtcactgtaaacaggccacccgagggaggaggtgtgctgtgcctcagctggggacaatctcaagaggggactctgaagcaagctgctaggtgccaacccttccatagctgacagaatgattgactaagcctgaagtggggtgtcaggtcatggaccccagtgtccactacaaatctgaaatttactttcctcaagtgagtggaaggacttaccattatcttcttaagaaatatctcgcaccctacagaatgggagaaaatatttgcaaaccatccatctgataatgggttaacagtcagaaaaataaaacgcactcatacaataataacaataaaacataatctggctaaataaatgggcagagaacctgaaaagacatttgtcaaaagaagacatacaaatggccaagaggtacatacaaaggtgtgcaatatcactaattgtattagtctgttctcacactgctaataaagacctacccaagactgggtaatttatatagaaaaagaggtttaatggactcaccattccacatggccggggaggcctcacagtcaatgcagaaggcaaaggaggagcaaaggcacgtctttcatggcagcaggcaagagagcttgtgtagtggaactgccctttacaaaaccatcagatcttgtgagacttactcactgccataagaacagcacgggaaagacccgtccccatgattcaattacctcccaccagattcctctcacaacatgtgggaattatgggagatacaattcaagatgaggtttgggtggggacacagccaaaccgtatcactaatcatcagggatatacagatcaaaaccataatgagatatcatcttaccccagttggctatcatcaaaaacactaataagtgttgtgaggatatgggaaaagggaacccacgtatactgttggtaggaatgtaaactgatatattagttcgttcttacattgctataaagaactacctaagactgggtaatttataaagaaaagaggtttgatgggctcacagttctgcaggcggtacaggaaacatggctgcagaggcctcaggaaacttagaatcatggcagaagacaaaagggaagccagcacatcctatatggctggaacaggagagggagagagcaaagggggaagtgctacacactctcaaacaaccagatctcatgagaacttactcactatcacgagaacagcaaaagggaaatccacccccatgatccaacatttcccaccagacccctcccccaacactgaagatcacaattcaacatgagatttgggtagagacatagagccaaaccatattagctggtatagtcgttatggaacacagcatgcaggttcctcaaaatttaaaaatacaattatcatatgtagcagtaactccacttctgggtatatatccaaaggaaatgaaatcagtacctcaaagagttctatgcacctccatgttcattacaacattattcacaatagccaggatatagaatcaacctaagtgttgattctactaatacatgagcagataaagaaaatgtgatacacacacacacatacacacatacacacacacacacacttacacaatggaattctattcagccttgaagaagaaggaagtcctgtcatttgtgacaatgtggatgaacctggaggacattatgctgagtgaaataagccaggcacagaaagacaaatactacatgatctcactttatatatggcatctaaaaaagacagactcatagaagcagaaagtagaactgtgcttaccaggggttgggggactgggaggattggaaagatgttggtcaaagagtacacattttcagttacaagatgaacaagttttgggaatctaataaataacatggtgacatggttaaaaatactgtatttaatatatacttgaaacttgctaccacagtagatcttaaatattctcaacacgcacacacacacacatagacggtcatggtgtgaggtgacagatatttcaattagcttggttgtggtaattatttcacaatgtatatgtatatcaaagcatcatgttgtacactgtaactatatacaatttttatttgtcaaatatgcttcgataaagctgagagggggggatagaaaacaaagaaatttctcacaatgtctctcagtagatctaagggtaacatattaaaaactcgaaaatatttggcccaatcctgggctgctaacatgggttagtggaaaagtgcactgtggcgccagaaaggtctgggttcaaatctctatcttgctgtttgctaatatttcttaacctctctgaacctccaatttctcctgtgcaaaatgaatataataatacccatcttattggactgttgcaagatttaaacaaaaaaaaaaacatagacttagattgtctagcaacaatgcttgacacaaagaaggcatttaaaaagcatttgttcccttcccctttttacagcaaatagttcattggcagtgaatgattacaaactacaagtgtttctcaacttggagtggtttctcaagtatgtgactggaaccacctgtagagattgttaaactacagatccctggaccccaccccattcttaatgaatctagttcatgggttctagggtggagcccaggaatgtataattttagcaagttccatggatgtttctgatacccagaaaatcatgaagccctctgcttgaggctgagctcagtaagaatattctttgtattagaacccagggaggtctgtgcttagaggatgcctgaggacatttgcacctccctccttgtcatgagttctgtggatgtacatctgcacatcacatcacagagacctctctccattgcataaattctgtgtattccaaaactaaaacatgcataaatcacatcagttatagactcaaaccaattctcctttttgagatgtcattttattgagttataaatcaccactaaaaggcaattttgtgcagacagaaattttactggaggatgcagatcccctgagcttgtctggaaaatgagaagcctattcaaagacgaagtgtcctgctggtggaagagtcattgggcctgcaaagaggcatgtctggatggaggtttaactttttcatttcaaccaaacaaaatggagcccctcacccagatgggattgctgaaggctttctgggtttgattatgggtcacaaagtccagctgcattgcagaaattacactgtcaagaagacgctgaccaaggtccagaaaataaacaggagctgagatgcagaaagtgacctcgaagcttaaacaggctttcccatgcctaccagacgcttttcttgatttaacaccgggtcatgtggtttttcagtgtcttctgtggctttcttttcccatagatgggcctcacttattctaaaatataaagctttgggggtttcttgaaaatggcactttcactcagtaaaaataagtccagatgaaaaccttatctgtgggaatccattctgaagaaggattaaagtaagtctattttccccaaatgatcaataaccacccagacctaatcactatctctgattacatgatgaaaaagattctggaagcagcacagcaaaaatatgacaatgacagagaactcaaaggtgaccctgtactcaccatctccatgcagacatcacaagtgcagggatgagtaagccctttagttggagatctatgttgctaataacaagacattctgagttttcttcttcttagtgagagagccttccatgaccattttcccatagtttgcctttattcgtttctaagaaactatttttccagttttgaccatggtgctgtaacccacagaggcaccgttacactgaaactatgcaaccctatctgttaagtattatccaacgcccacttgggttttcactggctcatttagagaagcacctttgagtacaatatccaattaaacagtaggtttacatggagtgcttcctgctcgtgttaaaaatctcattctggccgggcgcggtggctcacgcctgtaatcccagcactttgggagcccgaggcaggttgatcacgaggtcaggagatcaagaccatcctggctactacggtgaaaccccgtctctactaaaaatacaaaaaattagctgggcttggtggcaggtgcctgtagtcccagctactggggaggctgaggcaggagaatggcgtgaacccgggaggcggagcttgcagtgagcagagattgtgccactgcactccagcctgggcgacagagcgagactccgtctcaaaaaaaaaaaaaaaaaaaaaaaaacctcattctatttctgccctgtgctctgccattccctagatacacagaattttggacccagtagagcaccttcacgaggatagtgctgcagtgaaccgcagtagcaaggaaatcgtacaagctcagtggctcagcacaacacactgttctcactcgtggtccagtcagggactctcctggacagctgtcctcggggatctgggtctcttccatcatgggctccagtatctcggggcctttcacttccagcatgtgaaacactccgtcttcttcaagagggagtgtgtgggacatgttagggagcaggctagaaagcagagtacatcacttccactggcactctaccgtctagcactcaatcgcatcatcaacctaaatccgaagaaagcagggagatgtagagatgagcacagctgctgacagtgcctgcctcggagagatgttagctgcccctttctttcaatccctttttaaggttttgcagttgaggcgactgagactcggaagacatgttacccacagctagtcagtgacagcccagcgcagtgttcacccaggggcctcttgcccacccttattaattccaattaatggataaaagggctcatttggtctcgaggtacagctggagctttgtttcctgctcttctacgcaggactccacggtgaggaggaggacgaccactctgctgcaaaacccgcagttccagggcaatgcctcttggtctgggagctgcacagatgaatacctcaaggagcaagtgccagtagccaaccgtaattatgggaaatgcttcttggctcctaagggatataaaattactttggggaaagtcaaggaaaatagaaacagaataccccataatgctttatttggaggccagaagtcacatactaaggcttgtgttttgtgtttgattctgtcaagagagcttaaaaggtggagacagcctttggggggaatgaaggtctggatggtatcagcctggcttgcaagcgtcgctgtggctcatgaaaacatatgtcttgaaaggttgtcctgctcatagttccgagcaaatgtgagaaacaacagaggcttccaacaaatacctgctaaagaatgaggaaatggacacaggcaaataggcaaatggagtctccttaacggaatcgtaaggctgtctggaggtaatacgagtggaaagaactcctgtgtgaaaatctgcatgcatctttgcccccgtggaaccgtctacacaagtgctaatggaacagttagttacatacctatttttttaaactctgactttaccattacagaggttatatatctataggattttttgcctgaatttttagattttcacctggagatctggtatggaataattaaatgctgcatattgtttctcttattcttaaggatcttggagaaattatttaacagtctgagatctccttctctccttccctaccctccccacccctgacctataacagctagggagagaaaataaatacaaataatatctgctggccaggcacagtggctcacgcctgtaatcccagcactttgggaagctgaggcaggcagatcatgaggtcaggagatcaagaccatcctgtgtaacatggtgaaacctcgtctctactaaaaatacaaaaattagccaggcgtggtggcaggtgcctgtagtcccagctactcgggaggctgaggcaggagaatggcgtgaacccgggaggtgggggttgaggtgagccaagatcgcgccactgcattccagcctgggcgaaatagcgagactccatctcaaaaataaataaataaaataaaataaaatatctgccatttggctgcaaagtatggtgctgatttaacctgaatattaccacataaaatcaaataacaataataatagaaaataggtttatagcagtaccagaattatattacttaatttagctgccttttcccaaaatataatcacacttcctagattttacaggtcagatataaaagagtacagtggaagaattcaatcacatgtgccttcattgttcactttttcatctcaagctcttcttttcatgctagctgttccagctcttcaaaaaatgtttgttcttgtgagtcagaaatattgtatccattttattaacagcctgtttgaagccaataagatgaatgcgtttgctgagcataggttagtttatggcaaagtctggactcaaatcaatggcaggagaggagaggcaagctagttagatacctccaaaggacttggacataaggaagatttcagagttaaattagcaaaatgcatacattcaatacatacacactagtaaaacaaaatggctgcaattagtcaattatggaagtaaaccaagaaaacatccatctgtctgtaaaatagaagagtgtgggaacttcttaaacttcagtcctgctgatctggggtatagtaatgaggaagatgaatatatggttgtaagtcagtgagcagaatgccaagtggctgcattgtgcctgattggatgaaatgttatccatgttatctgattggatgaaaggtatgtgaacagaaggggctggtcagccaaagaagcaagaaagaaggagaatcagagggtctgaaagcccctctagatggcaaagcccttggacatggaagcatctaagaaaaacatagtcttggcagtgttgaccaaaagtatggttccctttatgagacgttccctgttgtgagcaagagtgcctcaagccattgacagcagcattctaagatccattaagagcacttgttctgatcctgtggacaccaagcaaccttgtgataatttggctcctcacatagtgagactattggcagctctgcctcaacacattctggtctacttgtcagttgtatagacgaatttaattatatctgacgtggtgtgctgactccaccctaagcacgccaacaaaatcacttttatgagcctaacagaccttagaccagggtgtactctttaaggtaaacaccaccctcggcatgcagctggacaggcagtaatgttgcccagcaacaccccaggccacacgccatacgccacttgaactgcagctgaaccagcctgcgtaattttgactgagccacatataaagtcaagatcaggatgttctaacaacatgaccacctctagtgatctgaccaaacaattgccatatcacaagccaggagcagtctgcagagtggaggaatggaaagaacctaaaccattttaacaggccatgtgccaattttcaactgtacccgggaccccaccatagacagcttcatcaaagatatcaatgctgttgacagagtaatgttttccaggttttatcccaccctactcagttgcagtaattgttaggtgataaagacagtgacagctcattacaaaattcaacttccagaagctggaaggttaagtgacacctcttacctgctgggtgatgggttagcgtcttaaccttatccttttgctactctctgccccaaactccaaccccatctggaagcttgtgcacttgaggcagtagatttcacatgaaaccaagtcagaaggctttacaacagaccattaagtaggaatgtgtaggaaaagtacgtagaggagaatggatgaaggggatgaagaatattgcctaaaaactcaagaccgttatctgtagcccttataacactttttatttatgtgttctgtgtgtgtgtgtgtgtgtgtgtgtggatttgtgcactactgtaccttcataccagcttgtcacacacgtataaacctatgtccacagacattaactacttggtttttgttttgttttgttttgagatggagtctcgctctgccacccagactggcatacagtgacaccatttcagctaactccaacctccacctaccaggttcaagcaattctcctgcctcagcctcctgagcgtctgggattacaggcacctgccaccatgcctggctgatttttgtatttttagtagagatggggttttgccatgttggccaggctggtctcgaactcctgatatcaagtggatccgcctgcctgggcctcccaaagtgctgagactaaaagcgtgagccaccgcgcccagcctacttggcttctttaaacagctttattgaggcataactgacatacgataaactacacatactgaaaatataaattattttaatctgtaattacacctttattttttaaaaaattgtgtgagcccaaccagataaccatgaaaagttccatattaatgatgattgtactgagtagagaagcctccaattaaagtaaattttgataacattgacatatatatatgcactggtggaaccatcgccaaaaccaagataacaaacacatccatcacctccagaagttttctcatgcccctttgtaatcccacctctgctgcttcctacccccagccccattcctaggcaaccgttaatctgctttctgtcactatacatcagtttggatattccagaaaattatataaatgatacatatcttatataccctttttctggcttcttatactcagaatagttactttgatttgtatctatgttgtaatatgtatcaatagttcatttattttcattatggctgagtgttattcttcatacggatggaccacagtgtgtttatccattcacctttgatagatatttggtttgttcccagttgggggcaattagaaataaaattctaaaaacatttatgtaaaagggtgtgcatggcataggctttcttttctcttggataaaaatctaggaatcaatgactagattatatgatcagtgtattcctaacttcctaagaaactgcctaactatgttcccatcaccagtgtttgagagttccagttcctcctcacccttgccaacacattttatggtcagattttccttctaattcttgctattctaataggtatgtagtggtaccttctagtggctttaatttgcatttctctaatgactaatgatgttgagcatcttttcatatgcttatttgtcatctgtgtgtgtcctcattaataaaatgtctggtcaaatattttgtccattttctatttggtttgttttcttattattcagtaatgagagtttcttatctattctggctacaattactttatcagatttatatattgtaaacattttccgccagtgtctggcttgtcttcttagtctaataacaatgtctttagaagagcaggtgtttttaatttttatgaagtcctatttattaattttttcttttatggattgtgcttttggtgtggtaactaagaaatccttgcctacccaaagtcacaaacattttctcttatatttttatagttttaggttttatatttatttctgatccactttgaattaatattcatataatgaaagatatgaactgaagtgcactattttgaatactgatatccaagtgtactagcaccatttgttgaaagaactatgtttctccactaaagtttctttgcacctttgtcaaaagtcagttgtccatataggtgtgtaggcctctttctattccacttatctatttgtcagtctttaagccaatatcacattgtcttgattagtatagttttgcaattcttgaaatccggcagtattaatcctccaagtttgttcttcttttataaagatttttgtttttgaggatttttgttttgctttttgtttgtgctgttctaggtcctttgtgtttctatatgaagttcagaatcgatttgttcatttctacaaaaaaaagcctactgggcttttgattggggtgatatcaaatctataaatcaatttaggaagaactgacatcttaccgatataagtctttggattcatgaacacattatatctctccatttatttatatcttctttaatttttctcaacagttgttttatggtttttggtgtacagagaactgtacaccaaaatatcatttctcagtatcaaagtattcaaagtacatcacttctcagtatcagactgtcaggaaaatgatcaatttccccttcaagactgacaagctaaaggcaccagaggcttaggcttcttacagcaacacaatgcagggactataaaaagcaaacgatagcacctatttcctaaagtcacgaatgttaagtgagtttaacatttatgcagtttaacgtaacaccggttgtgaaggtaaactgcctgggttcaaatcccagctgcaccacttataactgaatcaccttgggaaattcacagtctctctagaactcagttttctgatcagcttaatgcagaaaatactagcacctccctcataagggtcttcataagaataaaataagctcactaaagacttagaactattcttgtcatataagaactaataaatattagttatattaatatataaatcttagcaagttttatattatatttattatattaatatataaatattagcaatcattgttgattttattattagtagcacttaacatagtatttggaacaaatgagtatccaataaagggtagatattattggcttatgtagcaaactagtggttaacaccttcaggtatgcttctcaactgttttgaataaccgaagctgaactgaatttgctagaagtaggtctgtttgttctttattttttattttttatttttttgagacagagtcttgctctgtcgctcaggctggagtgcagtggcgcgatcttatctcattgcaacatccacctcccgggttcacgccattctcctgcctcagcctccctagtagctgggactacaggcgcccaccaccatgcccagctactttttttttttttttttttttttttagtagagacggggtttcaccgtgttagccaggatggtcttgatctcctgacctcgtgatctgcctgcctcggcctcccaaagtgctgggattacaggcgtgagccactgacactgcgcccagccagtaggtttgctcttaaaaggcctgaccctgaacaggaacattccattctttggatgctgtatttaagatgctatgtcagacatctctatgcaggatctcaccatgataggcaaatctccaccacaattagctttactactggcttccttaatctctctctggcctatcttgaggtctaaaaccctggaggagattgtatgaattatatttcctcattgctcctgcaatccttagagagatgacattttcataaggatgcatctacactaactctggccctttctctagagtaaagaagtgaccagatcacctttcatacatactagactggttttatattgtgatatgatttccaaacccaggaaggctctgtgtgcctctcatcactcaccactactaccatccacccttgcacacacacacgtgaaccctccctcctggcttgctgacacaatctgtctaattggaaatccatttctgtgcttgatgactttgttccctataaaaatacgaattatctttgaaggaaaagcaatcattaacctttgtgtgtaggagacagtattaaagtaatagaaagagaaaagcactcaagattcaagaaagaggcattcaagattattagatcccaaatctttcctctcttgcaagaagagtttgccatggtcattaaagccatggcactgggtgaggtcatcatccatgtggtgactattgctagagaggaaaactctggaatctaatggtctcaaatgcctttttccctcctctgtaaccaagattctactcaagttccctgatctacaataacaggatggcatttgagccattcattcattcattcatgcattcagcaaatcctgaccaccctctcaccatggtcaggtattgttttaagagcaggggacacagtagtgaacaaaacaaaatccctactcccacaaagcttatatccaagccaaagagacaggtaatcagcaaataaacacaaaggttgtaataggttgtcaaggagtaagggatttcaagaataaaaataaaatagggtaaagagatggagaatgccaggaatgctagtttagatagagtatttaaggatgttctttctgaggctgcaatggttgaatagagacttgaaaacagtgagtgaggcgacagctgggcagctagtagaacattccaggtacgggactggcaaatgccaaggtcataaggtagaagtttgctcaaagtgtttgaggaaaataaaagaagcctgtatggttgcaataaagagatcgctggagaggcatccaaaggccaaaccatatagggcattgtaggtgatcataacgacttttctgtatattccaagcgagatatgaaaccactggagagttccagaaggaaagtgacaagatctgaccttatttagaaaaatcacttgggccgatatacctagaacagatcaccagggagccagagggaaagcaggacagccagcgaggagctgttgccgtagctcaggagagagatattggtggcttagatgaacaaggaaggtagtagtcaaagaggcaagaaacagatatgtgatatatgttgaaggatgggatgtagggtttaggttccatgccatgaaaaaagtaaaaaatgactctaaaattggttatagcaaaggagaatgccatttactgagatgtagaaccatggagaaggttggaggagggacagcaagtctgttctggacatgtgaagttggcattgtctatgagatatccagggttcatgttgagcaggcagttgtatacacacagctgggcttcagaggaagagtcaaggttagagagacttccgtttgtggtcatcactgtctgcatggccattaaagccatggcactggcaccatgtggtgacttgctagaaaagagaagaggagcatccaagaaaagacagtgagagggaacagccagggttgtcggaggagtatctggaaagcatggtaacatgtaagccaaactgtaaaattgctccaaggagggagtgagcaaaagtcgctgagaggttcagatggcgtttttaatctctactatttattactgaattaaaggagatgaacacctgaaaccatgtattaaagtaccttgtgctacaggtcaagtaccagaaatcttgaccaaaaatagcttaagcaataaaagcattcatgatgtcacataatataattctctgagaagagtaattctgagggccgggcacagtggctcatccctgtaatcccagcactttaggaggccgaggcaggtggatcacttgaggccaggagatctagacaagcctggccaatatggcaaaaccctatctatacaaaaattagctggttggggtggtgtgtgcctgtaatcccagctacccaggatgctgaggcacaagaattgtttgaacccaggagtttgcagtcagccgagatcacatcacagcaccccagcctgggtgacagagcgagagtctgtctcaagataaaaataaaaataaaaatatataaaaaaagagtaatcctgaggttggttatctcattggctcaaacatatcaaggaccaagatttcttcatctttgggctctgccaccctgttggccaggtgtggtggctcatgcctgtaatcccagcactttgggaagccaaggcaggaggatcccttgagtgcaggagtttgagaccagcctgggcaacacagggagaccctgtctctaaaaagataaaaacaaaagaaaaaacggggggactgctgtagctccagatatcacatcttctcacaccaatgtccagaggtggaataaagggaatagcctttcattgtgtctctttctaagagtgaagaaactttaccagcaacctcctgcataattatcttttcaacgaacccagaactgtaccatgcacccatgtctacgacaatcctggaaggcagaatgatagaaatcgatatcacactttagggctggggaagagcccagggcctctcaaaggacatggctgctctgaggaaggtggaagaagtcagggttctgtaagcaagaaagaagacttaaaagggtagttcttggttcaacaactgataccatctgcaacacaagcatttgggcattctaaacatgcctatctttcttccacagcaatgatacaaatataggaagttatgaataaatattcattatctctcagccaagaggacaaggttttccttttcaggctagtgtttgagcaaccattgaatgcttatgcatgtcgtagaatctgtgggttcaaagaggccttgaaggtccatgtatcctcaatataaaatccccatgacttcttgtattagaaaagatcccagcaagacatacaggacacactcagattatcctaatgtaacaggaactcagaggatttgatgccaggactagctacaagtgaggccagggcttggcaaacaccaagggcaatgcagtggccagggctagtgtcagggaaacctccctcaccatgcctaggaggcagaagagggctccaagcgtggggcccccaacaggagtcaagaccattggttgagggacatagccaagccacagtggccttgtacggatgggagaggcaggggaaaatgtccagactttacttccttctccactcaactggaagccaaagggcagaggagccgcccagtggaataactgcaggtcagactctggggtgcagagcaggggagaagagggtggagatggcaccggaggagcaaatggaagacacccagtcctccccatggtgggggccagccactcctcaggctgctcatttcccctggccagttctgactgctggaaagttcccagtcaatccagggtccatgcaaaacaggtctaactcttcacttacatgaaaatactttagatagaggacaacagcccacacacctcacagccaagtggtggagtgaacaaccttgagatgttagtttagttccttggccccagggtacccagtgtctgatggaattggaaagctaaggtctccatacatcttccccttggcatgttgtttctcagctggaggtaattgcatcccccacaagacactggcaatgaatagagacatttttcactgtcaaaaatggtggaaggcatgcaactgacatctagagggtagagaccagggatgatgcaaaacatcctataatgcacaaggcagcccccaccatgaagaatgatctggccccaaatgtcaataggccaaggatgagaatcctgcccaggcaggagctgagcctggacaaggctgtagctgcaagacctttcccgggagccacccacgatgtttctctgggacatctttgttttcaaggtgagctaatgctgaaatctgtgttttcaaggtaagataacgcaaaacagtgctagagtccttgaagaactggagggaaggaataagcagcaatggagtttcaggggtgcggggagcgggaggagatgagagctgtttgtttgcagtgggaatggcaattgttgaatttccccttgcctggccccggcttctcaactaatgcaagggggagccctgagccacccttgatatcctgcgagccatcctcacatcacaacatcagctttcgcaggcaagcatgtaaacaagaagaccagccacgagaaacataagaaagaaataaaagttgtttggtcttctgtcaggaacagattgttggaatattccaaccccagtccaaaaagaacaaccaacaataacaaccgggagaccgcagcccacgctgagacacacgaagccttcgcttttcccggtgccgcggaccgtttccaggagaacgcgccgctggcatcgtcctctgtttttgccatggcctggggagctctagtgtttgtccaagcacccgcattagggccaagaaatatgaaaatgtcatctgtgagcatgaatcaggagcaagtgaacttctcatctgctgaaagtcagcaggtgtgagtattctgacaaacatctgcagtcctgcagcaattcctcatttatttggcatcaacagatcagctggaaatatcatattttaagtgaatcttccagatagctcaagttcaccctattaaagaatatccttaatgatgtagccttttagggtgaagacaactttccaaaaggtatctattgcctttacttcaatcaagtatattgacaatatttctattttttaactggctcagaataatgagtataatgtaataataaaaataataagatgtctgcagacctaggggtagtttgcccagacattaaatgaacccagatcagaacctttttccccctgctttttttttttaactctttatcctccctttgtgtagctgtcagctgctactctttacttacatctcccgacctgtccatctgtaatccctgccttctagtaattgccgctgtgggctaggacagtggttctgaatgttggcagcatgctgaaatctcctgggtcccatctccagaattgtgttttcactggcctaggcaagaggacagtttgcaactccccaggtgactgtgttgagtagccaaggctgagaaccactgagatgggaaatccagtatcttatctgttagaattgtgcacaaaataagagttaatatgatctgagagattttcctacaaataagctttagtgtataaacctttggcatgtattttgagctcttcgaatctgcaactttctcattcttagctgtacctcagcaatgtgacctcaagctaggagagaggtagaaaggaccagtggttaagtgtttggggtctagagctcaattacctaggttcaaacctcaactctgtggcctcgagcaagtatcttaacctttttgaacaccagcctcatctataagtgttggaaggactcagtgagtcagtgcacagagagggctggggacagggtctggcacgtcacaacactcagcacagtcagcgttacaggcagggtctggcagggtacagaattcgcttcagatgaacaaggaggagaggcagaggtgcgaactgggaaaagagcgcaattcaaggctactgtggttcccagaggctggcgagtgagaagcttgactagcctggacaggaagcgggaggggaagaagatgtgttatgagatcccagggaaagctgaggctgtggagagaagcagggaggcagcagagaggaagcacccgactcccattctccctccagcctccgacctcttgcaggagcctccctcccgctggctggatccagtgagaagccagggagtggaaaagaagtggccctcaggctcagcttctcaagaggcaaggcaaggcaaaggaagaaagagaatgaatctgggtgggtgggaggcaggcaaatggagaagaaccagccgagttagctattactaatcattccgtagctgggaagtcaccaaagaaagtccctattgccctagagtgggtgaacgctacacaacatccgctgtagaatcagaaagagaattgcccctcaagttcccacatgctggaagaaatgtgcctccaccacagacctttagcaccaaactgagatggttcaacactgctatgggcaaaagtccaattttttaagatgtcctagcctccttgagaatctcagggctgagggcaacgtgcctcatccctgtggactagttcgcgctgctctctgagccttttctcaccagctggcctctgtctcttttccaccccctgcccatgcctgtcagaactcagacctcctagctcacttcctttgctaattgaaacacattcctgagccccatttgtaacatgctttggaatttcttcctccaccacttccccacccccaaacgccacctctctcttctcactcatgaatgttgaccttttgtctaataaaagcttcattcttccaacctcccactattgacttaagtagccattcttggctgtgtttacatttgctctccaaaaccatagtctcactacctatcaagtactcagtggtgtaagtagaggcagaaacccttttcttccagcagcttccattttaagtgtaaggacaagagacattgctcagagtggctggtggctttcccagtggatgtctttgcagcgtgatagttccgccccatgctttgccactgcaccatattacaaatgaaaattagtcacttccagatgcaccccccgggcatcagagccctcttgtactgtgctggtacacttgcttcgctgccttggaaactctgcagtgactctattttcatttccatcactagtttgtttgtttgtttgtttgtttgtttccagatcctgtaaccaaagagctattcctttgccaggatctaattgaactattcatccttgttcctccattatgttccttccaaattcctttgaatccctctttcccatcacatatgcattatgctataataatggccactatttggctctgttttcccttggaagcctggcacatgttactactgtgctctcctgagtaaagagagaaggtggaaccaatcctgttcccctctggtactcagatgcccttctgcaaaagcatcagaatcagggaaccaggacctccagaaagagctgggtttgaagttaaaaaaaatcctaatgaggtttgacttggcagaattttaagcactgatttgggttcaggtgggccaaaagcgtgagtagcagcaacagcagcaccctctgtgtacccactccctgcaaacccctgttctaggccctaggaattccatcaatccctaccctcaaggaacttacattttagataaggagagaagactcagcatgtgtgcgcgtgcgcacacacacgtgcacacacacatgcacgcacacacacacgtgcacaggtgcacacacacgcatgcacacatacatgcacacacacacagagccaataatgcaggctagcatagaatgaatgccaattaagtagtagctaaataataataattaacttgcatttaaaaatctgtaacacaggcatttctcttaatcaagactcattttctcccaggtaatttccattttaattggtattggtggaggttttaattagatttcttaatctatctctgtttctgtttgcacaactgaaagatgtctcccacttccaaatctagcgtattgtttgaaattttgaatttatgacatctccacaaatttactatagattgatccatcagtatctaatgatgtcttgagatgatttcttatgattaaaacactttaaagtagtgattatctaaagtagaatctaacttcccgtttgaggaggttgaaacatgtgcttcctatcttcggttctcattttttttaatgtgggtgctgctttagcaaagccaataactacaagaacatcctcccccagtttgagtagatgtgtcaccagaaaagcaaaagtccaatgctgagtgatttgagtggcttggaagaatttcccagcttgcagcttatactgaacgagcattaatacaagtaaaccattaactcatcagtcacacctgctctgtttgctctgtgcttgtttctatcctagcacccttgacaaagtgctgagcttgctgcctgtgggcatgtcggcctccttgctagaccattcactagctgagaacatgcaggaggtcttttaaaaaaaattttgtatatatatatatgtgtgtgtgtgtgtgtgtgtatgtatgtattttaattgacaaataagaaatgcgtatattttatgatgtacagcatgatcttttgaatgtttgtgcaatggctaaatcaagctaattaacatatgcattagctgacatatatcatttttttagggtaaaaatatttaaaatccactctcttagcaattttcgagtatgcaatactttactattaactatagtcaccatgacacacaatagattctctgaacttactcctcctaactgaaattttgtatccttttactaacatttcctcaatccctgtacctcctctccccaaccttagcctctcataaccacctttctactctctacttctatgagttccacttttttacagcctgcaagtaagtgagatcgtgttgtatttgtctttctgtgtctggtttattcccctgagcaaaatgtcctccaggttcacccatgttgtcacaaatgccaagatggccttttttgaggatatgtagtattctactatctatatgtcctgcgttttctttattcatctacatttattcatttatccattggacacttaggttgattccataacttggctcttgtcaatgctgctacaatgaatatgggggtgcagagagctctttgacacactgatttcatttctttagatttgtacctagaagtgtgtatatatctagaccagaatggaattgctgggtcatatggtagtcctatttttaattttttgaggaatttccctactgtttttcataaggactgtactagtgtacattttccccagccgtgtgtaagggttcttttattcacatcttcaccaacacacatcattggttttttcatgctttattttttggtaatagcaattctaacaggtctgaggtcatatattattgtgatgcagtaggtattattcagcttggtacagtgagtacagcagagagtacagttcccaacagagagtacagtgctctgtgcccagcaggcccagaagtggattaacgagttgattgaataactgattagtgggaaataaggaaagcattaatactcccagagagcaaggatagacctaggggtgcttgtgagaaaccaaggttgatctacagcattcacagcctggtgaaaggggcccagagtgtggcaccagctgtagccctgtctgcactgagggccaggtgagtgagatgtgactgggtaccccttccaggtccagggaagaatctgaagagtggggcccacatcacccttcagaacataagacatggacactccctgatcacagggacagcccaggtcatttagccctatcccatacccctttataacaaaatactctattattacttccgtaaaacttggaaattgagatatgtgcaaatgagggtatgttccaaaaagctcctaacaaatactaactccaattctcatctggttcttgggcttgacatagagagggagagagagtggaaaaaggatttggtctcaaaacaacttttggattttgcctggaaacagtatctcgtagcatgttcattgcagcctttggctgaattctttcattagaaagaggaaaagcacatttggatgttgacgtgacattcaggtaggcaacatttctttgctcgacttgggaaaatgctaatgaagaagaaaccaatcctataaaaagaggtcagagtacgtcaaagtacctgtccacccccatagtcgttttccttaatcttgacatctgaatcacttgctgtcgggtgaacacaggaattttccagggaacaatctcatattgagtgaggctctactcacggttgccctacatgtcatgggtgtccatttcggccttccattgtatgaacaatgcccagggtaattcggatcttgataacattgactcacaacctcaaataaatgaagtcatatcaagccactggcaagacggaatctgccggccggaaagggagtagaaggctagaccacaggcggggactgtgtggagggcaacacaggtgaacgcacacagataggcgcagtccccggccgttcgcacctcagcatcggtggcacttgtcatgattcaggttgcccttgctttcagcaaattcaacccttttgaatgcttgtttttatagaaactaaattagagagggattattcatttacaaacaaattgttcattttaaccagagtcttaagtaactgatacctctgtgctagttataatttttttaatctcaacttggatacacattttcaagaatatatctattaggtaaagtacactcacataaggaaaagtagatggttaattgcctggctatttaattcccaatatcataatcttggacactcctttcaataaaccttcacctagccaattcccaagaaatcacttcctcaagtgagttaaactgggcaacggttaagcaataggagtgtctttttttcagatgccagcacagagccacttgtccctgttaatcacgaagactggaaaacaagcagagctatgtgacggatatattcaccagaccctatctctgtgggaggcggtgttttggcacagacaggctgatgatttcagggtcaagagggaagtgattaatcaaactgggaagaagacagaggaaaatccagcaaacagctatgaagaacatataaaaacaacaaccacccaatatctgtatgggtaaacaacgctccgtttgcacactggagaatgcaatgaagtgtgaccaggatgaagccgaaaacaaagaaatgatgcttccaactgcggctcccaggcatggcttttctttctgcaccttggagactcctctgcagctccattctcatcccacacctccagggtctgtgcacaccaaggcaggtggaaggggaggcaaggaactgagcaatctgaggttaggtgggggaaaggaaacacaccttctactattagtgcaaaacgagaattttcccagttaccgatcttgaaataaattcatcagatgatagcgttctccttcttcttttgccccttcttttgctcacacatcctaccttaatttgaaacattgcaatgaaagagaaatgtaaaaagcaaatctagaccaagctgcgttcaaatgtgcatgtagccagaaaccttaaaagtagaaggtgatcattttgttttgtttgaattttttaaaaagtataacatctgtcaggtactgactgtgaattctacatcttgtactgagtcgcccctctcttctatggaacattagaaagcaagaggaactaccatttgtgatagacgaagacagatttgcaggtggagggagtgacaagacctgatttgttttctgcacataatgagtaatccttcagacacagagatcctcatctgcagcacgagagaaaaggtaaaccaagtccccaggctcagcacccatggaaaggagcagagggagagagtcctctgagttggcacacgagttctgcaccgggctgtcctttgatatgacagctctcttctgtggtggggccacctaagaagtgcttgggaaaatatcttgataggagaactagacggaaacatgctttcagagaagggatgtgtcttgttgcttattgtggtttttcaatacatgagcctagtttacatagcaggggcccaaatgcagctctgtataatattgtcatacttcagctatgtgcgtgtttatcatttctttaccaacaacagctggagaaaatggctgagattggagaggagggagcagaggtagagaggaagtcaaaaccttggaatggatgacataccacttccccaatgaatgaagctgcagattcagccacatgtagttgatgtcgccatgtcaagactgcatttttccttccaaacacagaagtatggggtaaacttaatgcaggactatgaagatgaagccattgaggcccaagactttatcttgatttcttcaattccttggatatgtttactccctccccacactgggcccttgtagctgcttagactgaacctactggcccttctcttgctggaaagttgccctccaagaagtgcaagagctcagattgcacctgctaactgttaagaccagacttggccaggctaccagatctttctgcaacaaggccagcttcacactgcctgagcagacctttctgttctgccaaaggcagctgaagcagggaaaatggatcagcaaagggatctgggccaggcgcagtggctcatttctctaacctcagcactttgagaggccaaggtgggaggatcacttgaggccaggagttcaagaccagcctgggcaacaaaatgagaccgcatttctacaaaacaataaggttaaaaaaaattaatcaggtgtggtggcaactgtggtgccaactcttgagacactaaatcgggaggatcacttgagcccaggagatggaggctggagtgagctatgatagcaccactgtattccagcctggaagatagagtgagaccctgtctcaaaaaaagtaaataaaggaatctgaacttgaagaatgggccaaaaaagagtgatacttgactgcggttcctctttgcctgtgccgtcacctgggattggaattctgcatttcccacccccaattcccttctccagtcatctaactcctctgcttcctccaatactcagctaaggcattacctcctcctagaagccttccctgaaatcctcaagcagttctctttctttgacttccctctttggagcctcaactgtctctttgggtttgtctgtcctgctagactgaacgtaaataactaatgagggtatctgcatggaaagaaacagacccttctaagtgctgtgttaagtaacttcactgaaccagatgagagcattagagcagctgctttctagggttttgccagctcctgtatgcggacgtgaggctgctggggatgttgctattagtgataaagttaagggtccaagaggttctttgcttcacgactacgtcattggaggctgataagccatggccaagtgtgttcaaggtctccagctgtcataaaagtgtctgcttgtttattttaggtagataagtgttgctattattcctgggatggtaggaaaagccgggggcaagaaatcactctgtgaagatatattgagatccctggaacatttaaaaaaaaaaaaaaaaaaggttgaggggagggagagaaaccacatagcctgcatttggtgatactgtaattctagctccctttaattacagttaatcactacttactattttgtaatctaaggtaatgaacactgtagctttgcttgctaattgaagttgacagaatgcgagaaagcgccctatggcaaacccctttcatcaggagagtgttttatctttgtttatcaacaagagagtggattttttgtttgtttattttaaggagtcacactctgttgcccagactggagtgcagtgatgcgatctcggctcactgcaacctctgcctcctgggttcaagcaattcttctgcctcagcctccagaatagctgagagattataggcacgcaccaccacacccggctaatttttgtacttttagcagagtcagggtttctccatgttggccaggctgtgctacaactcctgacctcaggtgatccacccgccttggccttccaaagtgctaggattcaggcatgagccaccgcatccgcccaagagtgtttgtttgtttgtttgtttgtttgttttttaatggtttactctaggtttaattcagaggaagtaagagattattctgcagaacacccttgggtatttaacctggcacaactcaattaataagtgatccattttactattacaaactaaatttatctttggaaataatgacagaccgaaacaacccagaaactacatatatctattttgtatgaattaaaaaggaaagaaatcaccagaaagaaaaaaaaagagttatttaattgagtgcatggccccataagggcaattggaaacctgtatttaagtttgtatgcaattttgtgtatgcattttctggaaagaaaagtcatactttattcagatacccaaggaggtctgtgatatcccctctgccaatctcaacttagatattagtgtttagtgaatgaaatagtccataaactagattgactataaatctggtaataatgttgtaaaataaaggttttccacgctctacaaaagaaaaccaaaacaaatagcatagctatagttctctcaatcctcatccccaaattctctgcagctccctaaatagcctaagacaccagagaaagtcagaaatttattgtcacagcagctagaatgacctgtcacctaaccagacaaagtccagagcagaactgaaggagcagaagttcttagaaggtttaccttgcactgccatcactcacttccagcccaaaacctttaacaggtactttgtttgtagtgaatggcttaacttcactgaattgcagttaacctcaaacgtttgggttttttgttaaatgttttaagacgagaggaaaatagcacttttacgtaataagaaatttcagatacttgacctctctaagttcacaaattcccattttaattttcatttttactgaaatttcttacagagaagtaaaatccctcttcctaatttcaagctgatttaaatacctctgaaaccaggttaaaacctaggatatgatatagttctcccatttgggccagttgaaataaatataaatttagccctttttccccaaatattggttgtgtgtgtgtgtgtgtgtgtgtgtctgtgtgtgtgtgtgtgtgtgatggagcttcgttcttgttgcccaggctggagtgcagtggcccaatctcggctcactgcaacctccgcctcctgggttcaagtgattctcctgcctcagcctcccaagtagctgggattacaggtgcctgccatcacgccaggctaatttttgtatttttagtagagacagggtttcaccatggtggccaggctggtctcaaactcctgacctcaggtgatctgcccgcttcggcctcccaaagtgctgggattacaggcacgagccactgcacccagctggtaaattctttattatcattaaaagccaacaattttgactcagtcttattctatatatctgttctttcattcttcttgtatttcaatgaatgcttctataagtatactgacttcagccaggagtggtggctcccgcctgtaatcccagcactttgggaggccaagacaagatcacttgagcccaggaatttgagaccagcctaggtaacatggcgaaaccccgactctattaaaaagcaatacaaaagttatgcagtctcggtggcgcatgcctgtagtcccagctactagggagagtaaggagggagaatcgcctgagcctgggcagttgaggctgcagcaagccgagatcgcgccactgcactccagcctgggcgacagagtggggccctgtctgaaacaaaataaaagtatattatagatgccgtttttaccttgactcactgacatccagtttcagagccagcaaagctgaggcccaactctgctgtggtctaaatctgttgtagggtgaagcctgagggtcagtttggtgcccccttttacttttctctacttaaattcaatctattcttacggcataatacttagaaataaactttctattataagccttagatataatattcaaaggtaattagtttattggagaactggagaaaggccattttttaaacagtttattggagaactggagaaaggccatttttctcccccagacaagacccgtatctccacaggcattgacaatagcttcctaatttttttttcttactagctgattagtgctatgtctaatgaattgcccatacccttgttccctaggattgttgttgaaaatatatgcagcaatcagcatatgtatttagttgaaaaccaatgtctccaacagccttaaaagcccagctttctcttctaatatcaaaatattctattttactaataaaccatttcttaagccatgtaaaataaagtctaagtacaaatcttaaggcattatgaaaagatacttgggaactacatccctgcagccaaggaagtggtggtttttttttttttttcaaagacatctgaccttatcaaagcttcagaccaagaattcagttcatcagttcatctgctatctaataagcacaagagccatttgtccttcacatgataaggtcatggtacattacaagccacttgcaggttttgttttcttgaaaggacacatttgcagggagcactgccagagagaaacgactggctgaaatcaaatagtcgacatcaagggatacctatttcagaaaaagcgattgaaggcagcagccagaaatgctgagattttcatatgagggatgtttgtaatcataagccagcaggtaattccagcatgtgcagattctctttgacatggtgctataaaaactcttgggctaaaagcaaaatctctacctgacagaagcaatcctcactcccatctattgatactttgctcctgattcacagcaataaatggtccttaaagtgaatgagaggagggtaattcattccctacacacacaccaagatgagcccagtcttcttgcattaacttcttgctgaatgcaattgatccggaccattggctggttttccagagacttcaaatagcctgacttggcttgttcagccagtagggttgagatcagagacccctacatcaaggtcactgaaggtaccattggaaactacaactatcctggcttagactcagaccactggttacaacttcccattcctaggtgacaaatataaacccatacagtagttgaagactaaggaccaataaaaagcagaaaagttttttttaataataataaatacacctggctaaaaattccagtggccagaaggaataaatttagcatcttagctttcgttgctaaaataggatctgcttccaggctcactcttgtaagggaattgtgtatataatggcttctttttccagagtttggggcagggtttctcagcatcagcactattaacacctggggacaaataattatttattgtggagttgccctgtgcattgtaatacgtttggcagcatccccagatgctactagatgccaatagcactatgtctccccctcccccgaatccacccaagtttgacaatccaaaatgtctccagatatggaaaaatgttccctggagtaagtgaggggggaggggtgcaaaatcacccacaggtgagaaccactgctttagggcattatttgtttattaattgtataaatgtatggggtccaagagcaaatttgttacatgcatagattgcactgaggacaagtcagggctttagcctatccatcacttgaataatatacattgtacccattaagtaatttctcttggtcccctcccttcccaccccctctcccttccaagtctccattgtcaatcattctactctctatgtccatgcatacatggtttttttagctcccacttatgagtgagaacatgtggtatttgactctctgtgtctggcttgtttcacttaagataatggcctcagttccatccattttgctgcaaaagacatgattttattcttttttatggctgaagagtattccattgcatttatataccacattttctttacctaatcctccattgatagacacttaagtttatcacatatccttcttattgtgaatagtgctgtgataaacatgtaaatacagttatctttagggcattatttaataaacacatttcatctgtaccaatgacacctctcccctgattccttgctctccaaaagtacttccttccaaaagaattgcctccaaaagaattgccttttcttctgtaaaaaggtgaccagtcttagtttgaacaatttttctgccaatattactagtcataaggacaatacattaattgatccaattgttctttcaggatagagaaaagtgcttccatccatacatgctggaaaactttaagcatagatttattgaaagaacaaaataagttaaagtccagaaaatactgtagcaatattcaagtcatcgagaaaaccagaaaaaaatgaaaatttaaaactcatctgaaatcttcacctgaaaccacacagaaataaccattgctgatatttggtgagcgtttttccacttatctctccttgtccatataacagatataaagcctggtagacacaaagaagttcttctgtgaaataacccaggattcattatcccgtagtttcatattgacatttagaataatgagaggatactcatgcaattttaaacttgaagtatttgatttaattttccttgaattaacagattaaaaaatctgaaaactgaagaatctgatgaactttggacatttcttcactgctagagatattagttcttaaaaggtccctataatttaagaaaatgtgcaaaacctatagagctggctgggagcagtggcttacgcctgtaaccccagcactttgggaaggcaaggctagaggatcacttgagcctaggagtttgagaccagcctgggcaatacagtaagacccccatctcttaaaaaagaaacaaacaaacaaacagaaaaacttaaaagagctgaagttattgttatttttaaactgtgcttttcactgttgactccttgacaggaaagatgaggaagtcagttaacatatttttttcaacctcttttcttctcttaccagtatgattagttatattaaaatacttacttgtgacctttaaattctttttttcagccttactccccaaattgtttggtctcagttctgttttaaacgaatccacagcctctcagtttctgagttctttattttgattcattttttatttggctggattggttttcaagacacactttttatttgcaaaaagaacccatggatgctgtgttccttgaggtttgattcgttcctaaatatctgcctcctgctttcttactcaaggaacaactgggctagagattgaattcttggggaccccttctcttgctcaatctttatagacaccactccactatccctggtggttccccaagcagtgacctatgagcgcgggatgctggggcatgtggttcctcacagagccctgattcttcctctgggggcgccatctcactcagactgcagcctgggcatgctcctgtcacctcgaggaggtgatgggagtccagcttttgttgggccccctctcgccactgcccagcccctgggctcaatctgcatttccagtggggaggtagccggttgcaaagccccttctccatctacaagaatggcagcagaggctgaccctccttccttgccccagacctgccttccacatccggggaactctgatggttgccgtttcccttcttccatgaaggaggctctaccactgtccctattttaaagatgaggacactgagacatagaggaattaaggaatatgcccgtgttcagatagctaataagctcaagtctagacttgaacctaagaagactaagagatgctctgatatctacatggattattgtgagagaaatggtctctatcttgactaaggtttgcaaggatgtaggcttacagaagcatacattaaaatttgggttaggactaagaacaaacttcctttcttgagagcaacagggctcagtctaccaaaagaggttataagtaccctgtgtaaatgtcccagacaaaaatggcacctatgcacatgtgacctcatggcacctatccacgtgtgacacccttccagccaaccaaacaatgacctcatgatgtcaaaggccaggaatgtgaattgggaaggcgaaaataacagcttgctttcactttccaagcacaagccagccagcccaagacgtttctctctgccatgtgctccctgcagttcaagagggccatccatgcgccagacagattaaacactaaaggaattctagacgatcactcctgggagggtttttttccactactttctaatccaatgaagcctgggctggcaaaggcagttgaattgagagtggctaaatatgcagagtccttggaggttagaatacagtctgtctaccaagagaaggcattttgccttcagtctgtctggatttctaatatctactgcagactattaatcatgaaggccagactcttgaacctctttgagttgtttcacatttaatcagaatcctcccccttacacacacaaaaaagctacaaaatcctgcctggttatctgatttaaatgaattttaacattcaaacaatggtttatctggaacatatcccctgcatcgaacgtatatttaatagctttgaaataaagtcaaacaaaaccaaaaatgcaattactatgcatgtcatgaaatcatcagaattaaaaattagccaaggtcatattgttcatttcctttagatttcctgttaaaacactggttaccccagattttcaccatcaggaaatgggaaaaaaattgaataactcattttctataagacaatttccatcaaattgtattgggtgagaatttggcccagaatttacactttaatgtatgattttgcattttaaatgtcatctgattttatttgtgattttcacattaagcagatgtcataatttacctgaattccatgaatagctctgttcatccacatacccattttccatgtatttaactgagctttaacttattttattcttttaatgaatgtatactgtgtttaactcagacttttctattttggctttctgagatgtgaggatggaaatgcttttctctaagaaccctattctgggatagggaagccaaattggaaatgtggagccacactgatatacagcttccagaatagtcatatttccccgttccaaccacacataaattcctaaacttgcttcacacagagaatctgggaagtgaacaaagcctatgttttccctcttctactctccaaagtgtgggttgtgtgttggcaccttaggacaggaagggaatttagaccgcatgctcttgattgcacagtctgggagggtatggggtggtaaggagagcaaatgttcagctaggccagtagaatgttgccaccaatctgtcactaacgcagctgccaaaattttcacattgccgagaaagtaagtctttaaagcaaaggctctttgtgccttctttttggaagtttcttgctaatttcctcctctgcttccctggcgatctgagagctagagcttttgtaccatcaactctcagcaaatagaagctgggccagcaggctgcaaagcaaagggtctcattaaaccacagccctttgcaagtcaggtccgggcacatgtttggcatcaattttctacactggggcatattccaaaatacataaggctctcaatttttctgtttctttaaaagaaattctccaaagtcagataaagttaaggaatttgaaaggtgtttaaggtggaggtttccactaggaataattattccaaggagctgagttccaaatttgacatcctcagggtaagacgagaatctaacacatcatagcaataatgactgtctggtggtctgcaagcttcaccgctgggccgaagtgctctttcactgcacacagacttttagttgtttgggaattttagcagagcaaaaacaaggggaagagagaaaataaggtaaaaacaaggttcaagttgtcacaacagccatatattctggattttccatgatccgcatccatataatctctctgattgttcccataaaggtagtcatactcactagaattagaaaagttaaaagcataaacttggtatagtttataacaggtaagacacaactctattgttctttgagagcaatgattgtgccatatttatcttcgtgtttctaatgacttgcacatgacaaagagctcaatttatgttgaatgaatgaattgaaacataaatatgctaatgaaaatcaacagaaatatgggaggatagttattgtattaagcattattgttttacctctatgactgattttaacatacactaagaatgcaaagacataggttctaattgtggttctgcagaataccagggagaaagttacttatcctccaaagactcagttttgccatatagaaaatggagttaataacttccctgacttagcttatgttatggagttgttatgtaaaccacctgagacactgaatgtgaaaacgcttgataatcggaaaagatgcgtaccaatgtacattttcatcattatcgttattattaccaatcatcacggctctggtactcagggatgctcagtcctctcaaatcttgcaaaaagaaaactgctgggagccacaaaacatcttgtgccacatgtgagcttactttccaaaatggcttcgtttttatagtcattaaaacacaactcaaaacctgtcattctttgtccctagtgagccaaccaggacatgatcaaatgtggagaattatggagcatgaatcccaggaagaattcttttacaacacacacacacacacacacacacacaggctcacacacgtgctcacacatacatgctcacacacaatatcacacatcctttcagcactgagaatggttaatagtaggtgtgaagactcacccacagaaaactgagaaatagtgtgtgactatttctgtgactaacacactttttatatcatcttcctcttcaataccatccttaccccagatgtccaggatcttcaagttacttaggacccagcatacatgttgctaaacttctaccacttctgtaagtcatttaattcaagcccattcactcaatgcccagaactggagtgacaacgggtgggatgagaagtcatcaccttcttcatcaccatctttgtgatcttcatcatttcatgaacacttactctgtagctttacattcatcatctctgtctattgtgacaacatcttatgaaatatatactattaaccccattttgcagatgggcaagtcgagactcagaatgattaattttcccaaaggcacacaccctaatgtgacagactctggatttgaaaccaattccacctgattctaaagaccatgtttttaaccacctcactgtaatgctgagtgttcttaatcacaggaaatctttggtgtgctaggacagaggtttgcaaggccttccgggagcttctcaatgtacattctctactctgtttatttttgtctgtataccaacatatatttttgaacccttttttatatatggccaatgatgctaggcctggaagaatattaaaaacaattatttctataatgtaagtgactaccagttatttaatttccgttttttgggttatttgtattttaaaagaaaggctatatgctataagccaagtgaatgaatccctaatggtacgatttctgacactgagactagcagatggagaaggatctttgtttctgtggtggggtgtgtgtctgtgtgtgtgtgtgtgtgtgtgtgttaagggcgcagtcaagcactgcactactcgtaccataccatgcagacaaccatctaatctgatctctcaaaaggtttgacagtattggcatcattctcaatatcctcatcctacacgttaaaattgctaattaatattagtatttggttgctttatcttaaaacaatacctacctctgttaataggaaaattagaaattatatctattgttcctaaagatacaatttgtttctctaactccaagggaagtgaatgaatatgtttcagactatacttgtctgtgtattatttgtttttgtaaggtggttttttcttttgcttcaaattgagagcatacaaacaaaattccactgtataagcagtcaattttggtaataataacacatgcctagagcactcagattaaattattacacatactaataaaattattcacagtagtactccttggtaatgttggtattagggaacaggatagaacccatcttcaaagtcaaccctattacttcaagcctttgcagggtcctgctgtttccaaggatacaatccaatgcttaatttacaggaatccgaaatcatttgctgtgttaaaaacttgagattagcccttgctgcccccttccaggttggcctttggaagcgaaaggtctttaagcttaagtaaactggagaatatttctgagtaagcaggctccaggtggagggtacactccaagataccttcacttgccaaaacaacactccctgcaaggttatcagcgaaaaggcagtagaaagagccctcctgctgccagaaggtcttgttttgcaaggcttctcagcctgcctgcagccattgggtgaggagaggaaaggacacctcacctggcagagcagcacaaaggtcaggcatgtttccctcctgacctggaagctgggtcctgctccttcacatgaactgtccagggcttggtcatatacccaggtccccctcagtcctgcccagagtgactccactggtctccccagaaaacaccaacagcagagagaaatgaagtgtgtctgttttctggtttcatattgcagctcctcttgctcttcttaggacagaaataacatctgcaatgccagagacctgtgaagtaataaacaacctttcccccagctcttgacaagcattaccttgctttgaggtgcaatcagttctgacaagtttatggctttgtgtccttcaacccaatggacattaccctctgggggagtttaatgacccctctcagcttcacactcacttgaaggaaagagctagaagtcagtaatgatgtgttatgacttgcatggcttcaggtagttcagaacctgcaacctgtagttcagattacaggagaagaactcagacgataaattggcttccaaagaaggccaaatagaaaaaaaaaaggcttcttcagaccaatagctgagtgacctgaaatttaaatgcaaaaaatgcattaaaacccacaaaaccacttcctttaaaattcttgataccaaacatgttacagcattaagtgaaccttaatctaagcaaaattcagagaagagcattcacacctttgatagaagagccagccagccagggtgctggggctcagctcttgagaaaaatgttgatgtaaaagccttggtggcctggttcagcccctgagcctccctggtaagcacatggcaggctcagaacatccataactgaatgctctgagccctgtaaaaatgcagttacaatgggaaatcaactcttaagtatgctatgggatgctgtgataaaatttgagtttctctaccttctgtttgcactttggttcatttagaaaagagtccataattgtgtgcttcaagagtgcaattccatggctgtaacagaatagagtcctctttcttctggcctttgcctctttggggatattccaactctgtggaaggtgatcatttgcgattatgatcagttatttatatttgactgtaaatgaaaacttcagagtcagtttcaaaaaacaagagatggacataaggacatgtgcttatgagtaggggacaaataactagagacaagaaataaaaagagacaagatatgagacaagataacctttgatgccgtactgcacacacacacacacacacacacacacacacacacagaatctacattgtttctgtcactctgcggggctgctggaaggcagaaatgagaagcctcggccctcatcttgtttagagttttgcctgggccaggctcttctgctgcattggaattcaactttgcaaatctcagtgtttccaggttgacctcgggagaaaggggaccccagaaaaaattagaacaaaaaggaacaagtaaggagcagtgtctagaatgggaacactgacaaaaagaagcaaagtcagaacacatggtctatttggggggctgttagacagacctggactaggctaattccagggttgcctccatgtactcacgggccctcagaaggcactcttccctctcttccctctccagatccttgtcttcccattagatcaatgaggatggaggactacaccagggacacccaactaggggcaattttgcctcccaggggttatttgccaatgtgtagagatatttttggctgtcaaaactgaaggtggtgggtgctactggcatctaatgtgtgcaggccacggctgttgtgaaacatcctgaaatgcacaggatactctccaacagcaaagaattatccagcccagaatgtcaatcatgccaaagttgaggaaccctggctccaccatttgaaggatctgatgcaggtgatcgatggtcccccagaagagtattggtctgggaccaagagtccaatggccatactttacatttttccagggcctgagtgccaaagtgacctacaatccttataaatgttaccctgttttctggcattcatgagcattggaggttgaaaaatgattctctaagagaggcttggcctgcagtcaagttgaaaggtgagtgagagtgggtcagcctacaaatatgccatccacatggggctgctctgagtttgcacaaaggacagaatgtcacctaaatcaattcacatctactgatacaaacagcctactgcaaaggctctattgaatccagggtttgtaataagtatatcagaattcgaccgggcagggtggctcacacctgtaatcccagcactttgggaggtcaaagcaggagaatcgcttgaggccaggagtttgagaccaacctgggcaacatggcgaaaccctgtctctacaaaaacaaatataagaattagccaagcacggtggcacgcacctgtagtcccagctactcaggaggctgaggtgggaggatcacttgagccggaaggtccacactctagcctgggtgacagagtgagacctgtctcaaaaaaataaataaataaaaattaaatactaataaattctgtgaaagagataccacctacgcttcttggtaattgtttggtgaatacagccaacaagagcagaggcgcctctgtggtgttagagtgggctggagtgtttccacaagtttgccaaatattacagaaatatcctgccctcctgctgcacatacacctggcaggagaggaaccaatgggagaaggtctcgccgggaagattccagccagatgggggccctgccttggcaggtgcttggcatgggaaaggtggttctgaagcaccaaggcaggtggcttgtgaatctgcctacattcccctaactctctgaggcttgaaatatcccctcagggctccagagagttgctgttgttcagttatgatgccccatgccctaccagcctctagcaaaaaccatgcatagtgacttgggaaattcttttcactttgctgggccaagacccagatgctctgtgggcatgctgatgggggcctagtggtgttactcctgtattcctccgtagcaaaaaaatagtattaggagagatacagggagatcaggagaatacagcgtcccttcaacttctgcccaaatttctgcagtagcctcctaaccagtttccttatagctctctggttcccttccaatctctcccctcctatgcagccagagggattccttcacactgaaagctaatttgttacactcctgcttaaatacataaagtgattccatagtgctcagggattaagggaaaaatccttaacagatctcaaaaggcctcgcatggctccagcggctatgtggatccatgcaaggccttttggggtctgttaaggaattttctgcctctcaagcctaacatcccaccatgcgccaagcttgctttcatttccttggatgccccaagcttccttctgccacggggccttcacacatgctgtttcagctaccttagatcttctcctcccaggcccccaccacctcttgtcaccagactaattctattctcctcagtccttacctctctcacaaggccctggccaacctccctcaccagatcatgcctcatacaccacctatcatggcaacgcgaatttcttttacgtagttctttacaaaattgcagttttacattaatttatgcattggaattcaataaatatctactgaataaacaaatgaatgaatgaatcacccccttctggggtggaacagagaatccctccgaccacacattcttacttccatctctttggtggttctgtcctctcagcatggttagctgttgatttgtatctctgcccataagattcttcctttctggccaatcccattcatccactcatttctccatgaacccttctctcatctcctactcctcacagaacttatttgtctcactctatgaatcctgttgcattttctctatttttccacactttgccttgaatagcatcagctgtagacatgctagtcttccctttggggctctgaactccttgagaaaagagactcaacccaacatattgttctgcaaagcagcatgtacttaataaatatttgttgaactgaaataccacttgtgaaagctcaggtgataggaataatcgcaggtggcaactttaagatcacaccaaaacaccaatgccactttcattccacccactccgacttctaagagaggatgtagaatgtagctgggaagagggtctctctccatggggagagagcagctagaaatgctgtgagagttttctaattagcagtaagttaccaccacctttggggcccagtgggatttctcctcttgctccagatggctgtcatggcagtaactatttctctgcatgtaagatggtcagatttagcaaataaaaatacagggttttaggtacagtttacactgtttgggtgacaggtgcagcaaaatctcagaaatcaccaccaaagaatgtatttatgtaaccaaaaactacctgttccccaaaaattattgaaataaaagtttaaaaatagaaatatttaatttttaaaaatacagggctcccagttatatttaagcttcagcttcagaaaaacagccaggcttggtggctcacacctgtaatcccgggaggctgaggtgggcagatcatgaggttgggagttcaagaccagcctggccaatatggcgaaaccccatctctactaaaaatacaaaaattagccgggcatggtggcacacacctgtaatcccagctactcaggagtttgaggcagaagaattgcttgagcccaggaggcagagattgcagtgagctgagatcatgccactgtactccagcctgggtgacagagcgagactccatctcagaaaaaaaaaagaaagaaaagtttcagataaacaacaaatacatttttgcacaaatataacccaaatatttcatggcatgtacttctactaaaaagttgctcatagtttatctgaaattcaaatgtaattggccatcgtgtattttatctgtaatttcatgcttttagcataagcttgaagatgccataatattaattggtggctccaaatgaaaattcatttaaaaaaaaataccagtacaaaatgaccagacgtgtgcaactccttctcactgtatccttgtttgtctgcctgtctataatatcactgcctgagtcattattgtcttagagggtgggtgctggatctattttattctttttatagaatcctgatgttgcattcacatatgcacttaaagtatatttgtcttgctgcctgtgatgtccagaagaaggaatggactttggtaatagtttttataatgttcccacagaagatttaaattccaaaatgataccatagtttcccacacttaaaattttacatttcaaaaaacaccataaaatttaaacgtggaaactagttttgaacatttgaaataagttaacataaaagttcaggttttcattcccatgcggtgtgagtttgtcctggggcacggggttgtgcagggaaagaaaaggcaaatattctccagcaattttcctggagatgtatgacttttcaagcaagaggaaataaaagtgaagaatgagacatatccccgatcaaattttaccttcagaaatattaactgctacagtacacttactccccgcaacctcaatggaggaggccagattcctacaagcggggaggccttgtctgatttcattatatcttttcctcctttgcaatcctgcaaagtgatactttctcttttttatcaacatgggttgtaagttcaacgactgcgcacattcatgaaagtgccaaagagatgggaacctgttaggactaaaatccaagcgttttcttttgaccgtaccctgatccttgtctagatgttcttaaaaaactatgacctgacttttttatgactcagatgtttgtaagacccctagatcattaagacatatttaaacattctcgtgcccctactcctctcccacaagataatgttttgttcttaggcaactgccaggaaagcattaaaaacatctagcacaagcccaattttcccaaaagaatgatttcttgtttgaagtttaggagaaaaaaaaaatacattcctatcacttccatttctgtgtctaatttttatttatttatttttagaatatgtaaagtatgtattttcttagaatagttaggccctggggcatacaaccaatttactcacaaacaaaccctatatttaagagacagagttgttttttttttctgggaaaatgaaactgcaggctaggaattcatttctgtcctctatttgtcattttcaactttgattaggataataatgctttgcttgtgcagaaggctctatataactaaatagtgtaagtgacatggacctaagatgtctatttcctaccagctcctttctgctctctacagggtttctttgaccatggaagggggtgcttccaggaggcatgggaggtagctgtgggctgtgttaatttgtttaaaggatggagagccatagagaattctattaacatagatcttgctgaagcattcaaaataagcagagataatacatgagttactgtgaaatcgggacgtgagagctggttccgatattgcaataggaaactactattcttttgcttgactggcatcctcttagaccctccaataactcttctcaatttttatgttcatctgtattctcagctcccagtgagccagaaagttcatgacatgctcaggctggtagaaaatgagaataccagtcagctctccagagggctctgctggcatagctaagagccccaggacagacatgaaatgaagatctggctgagagagcactacagcgcccagctagaagatattaacacaagctctgattcacatgggacagcaaaatataatctgtgtgtgacaggaatcgacacagccttcaaccctgaggtggagcgaaagcacccagatatgcttttgcattgatgggaagtgcaagcagaaggtgaggggagaattttgcccatcactcaccatccccccccacacacacatacatagagtcatgccaaagcatgaagcagcacagaatccccagcattcagccatccctggcactgagccacagagaaattagtcaaaggctctgagggcagctagagcacaaagggtcatttgtttttagaaacaccagaaaaaggacaatattctccagctaaaccttgccagctccttgttttgctttgttttcctcttgtagctctgattctaaatccctgaagtggttgaacactgtgtctgaggccagaagctttcgtgggtcactagaaaagagcctagtgagggggaggaactggactggaacgtggaaagctggaatcgggtctgacctgccctgccgccttggcaaatcactcctacaggtaatgagtgggcctcagctttctcacaaccaaaactgagatcctgatgtgagtcccgctcaccttagagaggagagagaaaaccatgaccgtgaccgaggaagatgcctcaggacataacttctgcacaggggaggttgtcaatttcctctgcagtatggatttatgctcctcacctaaccagcctggactccagtatccctatctgtttaatattaagctctctgaaatgtctccaccataggtatctcattagtagaggacaagagacaaaggtgatttaatcaaaacagccaccaccccgacagcaaaacacatttactgattcctagaaccactatctttcctgaaatgttagtatggggttgaccctattggttacatttgaattgacttttccatgttgagagaattaaggtcaagagaatgaactaacagccagccagtttttatacaacaacatttttgtattctttccattgtaggttatatttctttaaagctcaaattaaacagccacttatcctataccccatcatctctttaagtctccttacagcagaaaaattctggagacattttcaaaggtggaaaatccaggcccagtacctagagaaattaaaatatggaacattggctcaaagttcataattaaaggtagtaaggaatttgcaggtgtgtagttttatcccgaagtcagtaaaaagaatcattttaatgttgttaatcagtggttcagcctgggaccttgttaaattgatttgcaaatgggaactttgaaacatcctggagtggccaagtgtaaaggaatgagagacgggatgtggggctctgcgcctaagccacagtacatttccagctcctttatcccaaaggaacagtcattgtcaagctcaaaagccaggtctggactcagcttacaggtgtctcctggggacctggggaggagcgattcccactgggtgaatgtcagcagagaatggtatgccggcaaagggacaccagagaactctctggtcgtaggacgggcagcaagactgcttcggtagattcaggacatgattctgggcagttagcagcctctctcccctgctgtgtgttaagaacacttgaggatgttttcccttagcatttatgatgctgaggaaaagagattttggaaactaccttgacaaagaaattaatggagggtgacatggggattccagcaaggccaacatacaattgcctcattttcatggtatgtcaaattagatttaggttttggctactgtgcttgtcatgggggctctaactctcacccagggccagcatctcacaaaattttatgactttacactgactttgacctccaaggacaagggccagtggggagaaagaccagcagaggctcattcctcctctagtctcaacgtctctctccctccctctttctggaacttgtgctcctgaggtggatgtctgactgtgtctttggccacagccagccatttgcacatctgttcctgtggagtgacaggcagtgggggagctcaccgcccacttcaggacccagacagccatggtccaggcactgctgtgggctggagaaagctggaaaggacctgcctgtggcaggaatctctgggccccttgaccatgatctccacactcaccacgtgtgtaccaggagggcagatccagacacaggagccagaaggaagcccacgcgagccaacagaacataacctctgggcaggaagagggaaatgcactctattgcccagtaccctagcatgactacctaccatgagcagaggtctatccaaacaggcagaaaaaacctggcacatgtacatttatcaaacagttatggagcatctactgtacatatttacctagtaggtacttgtggccaacactagcagtcatcctctaatacccattctcctcttccttagtcatgaaatgaccacctagaatagagactacacctcccagcatcccttgcagctagctgtgaccatgtgaccaagatctggctaatgggatgagaatggaggttctaggagcacctttcagggaggaggcacttttttcacctaattcttctttcctgctggctggaagatgttatttagaagtgatgtctagaatttgagccaccttggaccttgtactgaggatttcaaagcacaagagaggagaaacctgggtctctacagactttatagagccctgaaccaacccaggaattctaacaaataagaagaaaattaacttctttttaaactcattcatctagggtttttctgttactcacagtcaaacttaaccctattggactcaatatatatttgttttatttaggccttcaactgattggatgaggcccaccaacattatgaagggcaatctgctttactcaaagtccattggtttaaatgtaagtctcctcccaaaaaaccctcgcagaaacatccaaaataatgtctgaccaaatacgtgggcattgcagcccagtcacgttgacatatgaaattacccatcatggggatgaaaactggtgagtcactggcatatgaatagctggcatgactgtggactctggggagagagaagagaaggagaaggcagggcctaaggaacatcactattcaatgatcagatggaggagagggcaggtagctggcaaaggagacagctgacacttcatcaagtcctcagataccagtactgtagggagagccgtgtgcaggtagcagagccatcccagggccaaggtggggcctcagtttcccatcgagcaagtttccagaaccaagtgagatcagggtagcactggtgtgctgggggcttagtgccaatcagtgcttgaccattctggatgggcctggccttggggacgtgtcaggccaaaggctccgatgccttctacaatgaagaatggagggccacagaagccaggaccctgagcagccagcagaacagccaagccccttccctgtccagctgttctccaagaccagaagatgtaatgcctattgccgttttctgtacaacatcaattttcttattaggatacttttggggaaccagtttgagaatatatagaactgcaattttgttcaaaggcagtaacaaggttataagcatgaggtttgaagccaggtgggccttggttagatccttgctgtgatcctgagcaaggcagtcactccctgagcatcaggttccatatgtaggattactaacccctccctgattcaccattacggagaagagatggcgcacttagctgtatctggcacatgacttctacatggtaaaggctttcctttctttctttcttttttttttccttctcaaatctattgtttttattttttttaagtaagcagtggtatatatgtcatctttttaaatgtttcttttgggaagatcttatagaaaaatggcaccctgaaactttcagctctatatcccaaaaattgtctttcaagagttaaaaaactctttaaaatgaagagctttttttaactctttatgagttttaaaaaaacccttaaaaatgaagataatatacctggcctaaatcaaaataatctgaaaaatagatgtgtcccagtggaaagcctacaaaggaataatctcccatcttcatgggaccttctttctcctttctttctaaaagccttctaaagcatcaccaacacaccccaaattttgcttttcttttctattttattaccattttttggctgttatcactccatgttcccttgcatgtgttaaatgtatacatgtgttcatgcgactgaagtcatcttttgaaatacatacaaaaatgtaaatagccaatctcgtgtttgtgttagcctttgaaatcaggctgaaaataaaaatgcatgaagtcagttataaattgctattgccaaacagaaatgagatgagtatttgccagaggtctggggcctggggggaaatggggagtgatggctgatgggcatggtgtttctttctggagtgatgaaaaagttctggaattagatagtgatgatgttgctatagctctgtgactatcctataaaacaccgaagagtacactttaaaattgtgaattttatgtaggtgaattatgtcccaataaaaacaaatttctatcgcttgggtcaaatagtggatcgcctacttctaaggtcaagtgttatgaaaggcggggcagcattagggattcatacatggcagacaatggcaccaggactccgtgttgaactagcagaactgactttgagcatagtacaaattcaggaaaaaggactcatctagagaggctggcgtcaattttaggaggacagacttgagctgagtatgcagggaggaaagaatggactggaagagcaaagtaaaagacattccaaagaggaattcagaaggagggagagatcatgatgctctctttacttggttactgttttaaactttcatttcatgtggcagtgttttcaaggggagatgggaagattggacttctaggcaagggagttgggagcacaaatcttgtttggctgggcagggaagagccacattagagtgtcccttcacaagcagcctttatcttgatgtgggaggttgcagggcagtcgtctgaagccctggagccatgaacagtcacatgtcgttcattctgatgcgtctgaactcctgcatcctaagtcacgtaactggaggcaacgagagcctgttggataggaaacatgtcgactggcccagcctttgcagcctttcctttgtaagagatgtctaagctctgtttgaaagaaatgaggtttctttgttttaaagaaatagaatactgcaagggagagggagagtttcccgggctgccatcttgttttctgtgggtgggaagtgaaaaacctctcatttttggtaagctgagcaaagcccaaaagcaggagcaaaatcagtccacactcgagcttcaaatgccactgtgaaaattcgaggcaggcttcattggttaaaccgcagcctgtcagggaggcttcagcaaaaatgctggcatgagatcttgattcttctatgataggccacaggacagtggccgtactgccctgccaggtaactggtggggcccggggcctgggggaccacgtcgtgatggttcattcctgggccctgggatccatctgcctttgcctgtcactggaacccatgacagcagtggactgagcctgtcagggaggatgagagagatggaagcagcccaggaactctctcaacctgaggcaagttgtgcctcttcccggctgccctgtgccaggccccgagccagtacagaaatggcacttaggttgatatcttacattcagtccattttgctggaatgttctgtaagctccctcttggaattctgggtccatgacattcttttatcctttgctattaacattatcattgtgttagcagtatagctcagtatgactgctatttaaacatccatccccatccctgcccgctcccccacccgaaaaaaatactgtctgcactgaaaagaagtggtttggcatagtgaaagtttttaaacatccattttccagatggatatccttgttaaatttaaaaagaaaaaaaaaaactaaaccatgtggaatgctcctaagtgaatattattgtttactagacttattccatcttatggcattttatgacaaaatatcagcaagctcataaagagggctttttttaaggtccataatctttctaaccataacaaaagggtggtaaatatattgtacaagagcacgatggaaaaatgtgctaaagtatttccacaaatcaaatgtagcactttggcattggctctaaagcattaaatttagtaaattagaaccagatgattttaaaatagaaacttacataactttacggtgtgatttttttcccccaacgcaagtttatcttcctgcagccgcgttggctgctactgtaataggtatttaagaagtagggcagcctctaggtattattcatctttgtagctcccaaggtgcctagcattatattgggcaattagtaagtattggtggatgggtgaatgaaatctcagcagggattaacaagtactagttaactggcaaggaaatgtaatataaatatttatacagatctacaggtagacaaaacactgccgctatcacacacataatagtgaaaatatgggttgcttttcctttcattgttaaagctgtggattaaaatcaatgaacctgaaataaaagggtggatctgcttcgcctttgggtcaccatgcttcaaaccaccatcaccctggaatgttcctaatacataagtctcatttctatttctgccatcatagcagccacagaaaatgctccttttggtcatgtctccctctcctcccacacacaagttcacaatgtagctaataccttaaagataagctgggagttcaacacagcatattgactgagtgcctataatctccaagaccctgtatgtgctgccacagggggtgcaaaggaataaggtatagtctttgccttctaggaaaatactttccagtagagggttagtcagcacactgtcattgcatgtaaaagaaatctaacttatactaggttagtcaggaaggtgtatttatggccttctgaactgagttgtctaagagtagacttcaggcatggctagatccagaggcacagacaacaggattagggttctctccatctctccactctaaatgcctttgcttctttttgcacatggactcattctctcttgctattgactctctctacaaggagaaaaacatattcaccaccgagcaaacatttacagtctatgatccaaagacagagaagttgtctctctcccaggcttcatatacaaatctcaaaaagatcttggattgactctgagttacatgtcaagttctcagattaattactgtagaaaagaggatgtattctatgaccaatcaggcctgagtggtggttgggactctccctttgtggatgaatgaaaaggaggcgatttatgtcttaaatattgatatttaaatattgatgtgccttggcagctgattggatgtgggaagtaggtgggagaaagaaataaaagatcagtctgaggttttgattctaggtgactggtagggacataaatagaaagagaatggtttaaaacagacactgttttaaagggaatttatcattcataggtgtattaatcagggttctccaggacatgtgtgtatctatgtgtgtgtgtgcgtgcacacacgtgtgtgtgtgtgtgtaaagagaaagagagtaaaagattggtttgttttcaaggagttgtctccaagtccaaaatctgcagggtagacccacagcatgtggaccctgggaagagctgatgttgcagcttgagtctgaaggctggtggaacagaattccctcttcttcagggaacctcagtctcttttccctgaaggccttcatctgattagatgaggcccacccacatggtggagggtatctactttactcaaagtctactgatttaaatgttatctcctctttaaaacaccttcacagcaacgtctagactagtgtttgatcaaatatctgggtagcatgcatggcctatccaggttgacacataaaattaatcatcccaatatttgactataaggagcttatgacatgcctctggaatatttaggtgcagtagaaaatgagggcttggaactcagaacacaggttgggagatgtgattgtcatcagagtagacgtcattggagagcatgagatagataagggagaaaatacacaaggaaaaggagctgagaatggaaccttgaagaaaggctcctgaaaagaagactgaaacacattggcaagagaagtagaagaaccagaagagcccactgctttggaaaccgaaggagttgatttcataacaggggaaataacaaggagtttcaggagttgaggggagatcatagagttggcaggcagagaagagtccccggcttggacaatggaggctgggggttcccctggagcaggactcctcaaaatgtgttctgcagacctgcaccaggccacacactggacaggcccaccaacaggtaggtgcagaaattgagagctagtgcttagaagctctgacagccattagacaagagtgattttttatcagctgaattcaattatcatcatgatcatcatcatcatcatcaaggcttgtattttgccagtctttttcatttcttttttctagtaatttcaacactactcctattctatgcatcaatggctttgatggttattgatggaacaggggtcagaagcagatgcctggaggactgagcaggaggccaggatgctggaccacccactctctggtcatggcaagtgaaagatagagggcacttggtcagtgttggggaaggagaggtggcaaagggaagatcctgaagacccagagaatgttgtttgtggctcatatttgctcatccacagtaacaaaatgtaaaaatctggagtattttgatagctcactcagcagcacagcctgattggagttggcctgagtgatatgtattcttttacccacttggcatgactctttgtagattcaattgctgaaacatgcatgcctttgctcatgggacacagccatggatttcactgggagtgtcttgtaatatgtggtatatgctctaaatctctttctaaaatctgaaatattctgaattccacaagctcatctggcctccaggtttttgaacaaggaactgtgaatctgtttttagggtgaggaaggccagaacttacttgcagagagcagggtgggaaagattagggggcacatcagagaggggatggttagggagctgagtcccagagtgggcttgagaggagagaaaaaaaatgcacagagctgtctggataaaaaggaaagacagttttttttttttgcctggtgaccagaactgcacaggtgatgacttttgaaaatgtagagtgattttaagatggcaaaatgaaaactgggggaagacatggcctctatcagctagggccaggagggcacagcctttcttcttgtcactactctccacccctcctaagaccagaagctccaaaagcaggttagagcatgaatcaggagaactgcatgccctgggttcaagaacacccttgcaacactcccttgtctacatcgtcaagtctgaaatcacagggtgccaggccttcagcaagttaagagaacttatacttagtgcctgtaaagctcaggggtaccagtgagcgagacttcaagtcttgtgcatgctcattgccagaccccctttggctttttgtataaagaagagagctgctctttatttccgggctcagtgggcagaaaggaatgctccgtccatactccgttcggcaagtcaagggtggacactggtgtctttatcaccacccagtcctcggcccacactggcaaggcattcctctagcagacaaaataaaagattgctgatagctggagcactttgtttgctttctaaaacgagtcaaactcttcaaaagcttggcttgaaccgtgcagggtgtgctgtgttcccgccacattcctctcacccgcctctccaccaggccttgtattatccggattcctttcatgcgctcacgagcgccagctggcggctgcttgggctggccggacaggccagaggctctgggcccggggcctgctggacattggccggcctcagctgatgagggcagcggggcacgggagggaggccttcttggagggctgggtcagctgggctcttttaaggcacaagggggagaaaatgcatctccaacccctgaagaaatgaggtaccctgggcattactagtggccatttggtgtttaaaacactcccttctcccccattgtgtactgtccctacctccgcccccggagctatgctggatggctggtgtggaagatggcttccggaggccagtgtgcgctggagaatggcaaagctcggaagtagattggaaacagaaaatccagcccatctaggaagctagggcacacaatccataagccttttctgcttagtccaactagacaatagcaagacgtggagaggggaagagggctacaaagtcgcatcatatcacatgatgtcatgccatggcaagtaggaaagatcatgtcttataccacatgacatcacatagaaagtgtatgccagagaagtcaggaagacttttcaaatgtaagaacatatagaggaagcacaaaggttagcaagaagaagacctgatgcctttgctccccttcatttaataggtagtatgcaccaagatgattgtgtttgggcagtgcctccggaaagaggagacggccactctcatttcagccatgagagtccattcctgtttatttgatgttggcagatcacttcaacctttgtaaaaatccacagtgtgaagtttctatcagcagaaaagatttccatgacagtttcatataacaagttgtttatttggacaaactaaagcatgtaataacagaacacctcacggctagagaaaacaggagagagaggctttgccaggcagcctgcacaattttactattaaactccttttgttccactgaactctatgcctttacctagctggggacacataaatagtagaaatgtgaaccttgcacaattatggagataagcctaaatctttatgcatttctaatttttcttatcacttcacctttaagttaattcatccaagtctttcatgtaaagaaaatgctaaaatggagcgtcacaattgcttgtcacatttcactagagtcgagtgaatttatttaacacctaatttaatctgtcaacgtttttcaattctttgaagaaaaaaaggtagtaattaagtattccaaagttataataacactaaacatcaaaacttcacaatcgcacagttttttaaacatcaagttaagatattagccatagtcactccacttaaggtggtctggctaggtttttagtagcacggtagtgacacggttttacgtgttctatttcatggtttatcaagaactaagaggggcctaagacatcccattttagcgcttcacccttgggataattaaaagccacctcaaagagatggaaggaagcaggaagagggctcagtaggagtggtggttgtaaggggctgtacagtgacagcctgctcaagctcagctaagtggtaagaggcaccaggtcctcgtcaagtcttcacagtgtggagacccaccgcgtcgctgtaacctagaagatctagagaaactgcttccattctctgctgcctagcgccccacccaccccaggcagcttgtccttgagagcgaaatgagttaggagggaaccaaatgagaagaaattcagggatcacgagtcaaggagcttttttagaagacactaccctccacctccatctgcagaaacaaatttctttttttttttttttttttttgagatgaagtctcgctctgtccccaggctggagtgcagtggctcgatcttggctcactgaaatctccgcctcccgggttcaagcgattctcctgtctcatcgtcccaagtagctaggactacaggtgtgcaccaccatgcccagctaatttttgtatttttagtagagatggggtttcaccatgttggccaggatggtctcaatctccttacctcatgatccacctgcctcagcctcccaaagtgctgggattacaggtgtgagccaccgtgcctggcctattattttttttaatacgaacttaacaagtctttcagaaaatagaatgtattcctaggacactgttgctaacgaggtagttcggggtaaggtcgggtagccttcatgaggtctcttgtgccaaaatattagtggagggaaagtgaatgaaagccctatttcacagtatataaagaatcaagcattaaaactcttttgggcttttctctaataatagactttcattcattccaagagcttgaccagttcaacagataaaagaggtttattgccttgaagtgagaggagctcattcccttgccttctgagaagtggcttatttgtccccctgttgaattcagtgaaggcagtgtgcacagacaagacacaggctttgagaggacaaaagatggggttcagtcacctacataagtgcaaaatgggctacaacaaaagaaaagacagaaccctcttctataaattgctcaaaatctcattgcggaaaagaaactctcacaaaagaaaccatgtaagggaataccaagcactaaatggtgtgttatatacataaaactgactagagagcatatgcagattttttttatttttatttttttagagacagggtctcactctgtctcccaggctgcagtgcagtggcacaaacatggcacactgcagcgttgacctcctgggctcaagtgatcctcccccctcagcctcctaagtaactgagactataggcatgcaccaccacacctggttaattttttttaatttttatttctgtagagttggagtcttgctatattgcccaggctggtctcaaactcctgggctcaagcaatcctcctgccttggccaaccaaagtgctaggattacaagtgtgagctaccgcacacagccatgaagatcactttaaacgggtagattccatagcctcatactaagcctactgcggctcatacttaaaggagagaggcctaagcatttctaattgtttcttaagggaaattggatttgggaagcatagacttaggccacaggtgacgggagtccagagatacagaggaagattggagggaggagagcaacaatggagagatttttctaggaaaggttttataaagaagatggggtacaagcgggaggcacgataggatgtaggtaagcagagccacgaagtggggcagagtgatgaaagaagaactacatacgcacaggctccaacgtgcacgtgagtaaggggtgtgtgcatttgtatttacacggctgcatcagccctcctcacaactcaagaacaatacctgtttctcagttgagcttagtcccacgagggtggagactcgaccttattgagcggacaaacatgtgctcagataacgaagtgcattaattcattcattcatatgaagagaatggcagcaatatagctccatggtcagggccacacagactcagaaaccagaaagcctgggttcataaacaaaatgggccatcaccctgtaagttggcgcatgctgtagaacttctccagtcttggttttgtgaagtgtaaagtaagaacaatacaagctacctcacagggctgttacgtgagatgaatattaaatggactcctgcttgtaaacatctggcacagggcctggcacctcggagggtttcggtgaaggctgaatgaaccaagagtcagttgtattgaaggagaaaactctcaatggctggtctttgaggaggtttctggagacttgtaaaagactggaaaagttgctgcctccaattatttttgaaataagcttggtatatgtagattgtttttaaaaactaatgtcaaactagaaatgataaaacatggccctagaatggttcctttttaggactgggcttgttcctctggtctagcactcactcagcttccagattgttcccctgtagatgtggaaagatctatactttattctgaactcaggcatagatgtaccttgcactaatctagagtgtgggtcggcaaacttctagagacaaccaaataatactttttcttcttcggctttgggggctttgccatctctgtggcatgtgctcagagtctgccattacagctcaaaagacatccctacatgaatagggatggctgtgttccaataaaattttatttatagacatcgaaatttgaatttcacatcattttcatgtctcatctttggtttttttcccaaccacttaaaaatgtaaaagctattcttggctcatagatgcagaactagcaacaggccttgagttggttctgaaaaggtgcatcctaacaccattttaaataaatggaaaactcactgctaaactcaaacacacgggggaatatgtcttccctgttcccttcctgggcaccaaacagaacctcatgataaacatacgttctttgaagttacatttatcttcttactcattgatgctgcaagcatttatgcacctctaaggtatacaacaggacaggggacacagatgaacaagataccaccctgttccccaagaacacacatcggagctggggaaacagacatcaacaaatcattatgagacaacgtggaaagcccttataatagggccgtgttccagtacaatgggggcatagtgaagggagggaggaattagttctgaaagggcgaggtgggcagggtgggggttgtagacaaggatacacaaaagggttagtgttgaggccaaacttgacagcagaagagtgaaggggggtcattctcagcaaaggggcctgcctgtgcaagtcaggaaggtgcaagtccgtcttggaatcagtaagttcccggcaaccccacactcccaagtatggctagagggtgggatgggggtcggcggtagagggagaaagaaagggtgggttcagatggtggtccatgccaaagtgtccagattttgcttgttaagccattgaagtgtcactagaggtttttaaacacggtagtaatgtgatcgactctgtattccaggaattaaacacgtagtgagcaacgtggaagatagatgacagcagtgagagagttaggcaaagaaactaaaaagaaatcattagaatagaccagaccaagagattcaggggcctgacctcaccaccaattgctgttataactcaaactggtggggccctgtgtgaggcactcaatctctctgagcgacagacagctctgccctctctatgagtggctggattaggtgatttccaaagtcatttcctgccctcacatgctcttcactctttgcccttcactcttagagagcagtcacgtgggttcattccaagttgtcaacagaagtatttcttctttctagcctcctcttgattttttgctgtatttatgccagtgcccagttgcagctggaaaatcattagaatggcatccggtgccatttccctcactcctgcctgcacaagcatctggaaggaagagtgcttggttgaagagcaggcaggcggcaaggatgacaggaggggatgcccaccggagtgctggcaagtgcaggaagtggaaccggaggcccagagttctagccaatttcaggagggtctctatgggaatcctagggctgctgcataaatcaattacatagcccagtttaaacatcatttttgcatctgatagtaataaatgaggaagggaattgtttctgtattcactgagacaatttgtgtttccctgaagagttttaagggcaacatactaaatgacactaataaagtaacaactatctgcattatttaagctgcattaagaccagagctcaatattttaactagtagcctgctgtccttgagtgtttaacaaaccggagagaaacagattactccctggtcaaaacactgcagaggcttcatgtcacactcaggaaaaaaatccaagctccctaccacctacctctctgagctcatcctctccatccagccctgtgtaccccacgctaagcacactagacagcttgctgcgcttagacacactaagctcgtgcctactgcgggcccttcccctgggtcacttctgtccggaatgctcatcccctagatctctgagtggctggatccctgaaactattcagatttctgcttaaatatcatctcctcagaggagcttccctgaccactttatctaaaataatacacctcctgtcccaccctggtctgttttcctccagcaattttccctgcttaatttttcttcatagcatttatcactgcaaatcatattatacattcatttaattattttcctcaactctcactagactgtaagctccatgaagatgggaactttgtctgggctactgctgtatcctcccctcctagaaaggtacctggcacatgctaggtgctctagtgataacagttcagtgagaaagctgccttatgaaagaatggcacacagagaaggggttcctccaacttcttctgaatgcctaccacacttatcaacagtagtctaatattaatactagttataattaatacaataattaaataataatctatagaatatagcaataatgtcataaaatattaacaaaatatcataaatctgatattaattaaaataataactaataacaacagtaataagaacaagcaaccatttaaggtcttacaatgtaacaagtactattaaattctatccacattatcttatttaatcctcattatgaggctagcaggtattattattttctctatttcatactgaaggacatcaaaattaagaagttcaactggccaggcacagtggcccacgcctgtaatcccagcactttgggagactgaagcaggtagatcacctgaggtcaggagttcgagaccagcctggccaatctggtgaaaccccgtctctactaaaaatacaaaaaattagccaggtatggtggcagacacatgtaatcccagctactcgggaggctgagggaattgcttgaaccagagatgcggggattgcagtgagccgatattgcaccactgcactccagcctgggcaacaagaatgaaactttgtctcaaaaaaaaaaaaaaaaaaaattaaaaatgttttgaggttccagcacaggtttacctgattccaacacccttgtgctttcctttaggcagctaactatatactgacccaagccttcttgaaatgaacttcgggtagattacatgtgtcttacttaccttacaggacagaaacaggaaagcaggagggccactagctagagaatgaaattacaaaaaaaccccagcacaaactttaggaaactgtttgaaaacattaaaataggatgggacagcactcacttactcaatgatattcatcaaacaaaacagaaaaaggattcagcttgaccacttaggaagccaaaggaatgttatctagatctcttggaggccgcaagactcatcttacagatgggaagggctttgaatcattgtcctcctttatccaggtagacaccaaaaacaatttcctgcaaactaacgactctccggtcagtctgcaggattcttaaggagatcgttacaatgcaatatgctgcgtgcttaatttgtgttcagaaaggccttgcacaatcactcaggcttatttttgctctaaggacaaatgaggagaagcaaggcctaatacaggctggaacaggtatgtcaacctcattaggatggcctggggggtcatgtccctggaatcagtgccacactgaactgcaaactaacctgccaaccctgtatctggaaaccacttttgtaggacagctgttctctcattccttttgcttagatcataaaagtagagttttcatccattgggaatttgtgtgttagacgcgaagggaatcagattctgatccaacttggtcaggaaaaaaaaaaataagggctgatttttccatccaagtcatgtagtctggttggagtgcatcccactcagggacagctattgtctggattcaccgagtctcagtcttgcccgggaaaaaggaatttttcgcctcactgctctgtccgtgagaagagttgcagaaggtgaccatttctgttttctgggtgattctctttctctatagaaatcctaaaatggaacctttatagaaattatgttctgtgcttcgctggagagagactggtctttttaaccaggctcatcaaacagtgggcattttcgttctcctggataataagtgttggtgggttaatgggtcatcctcaggacagaggtcagaaggaaaaacactgcagtgttcaaagctggagctagaaatgccagccgtcaaagaacacagaactcagtggacggtgatgatgtatagggcgtgcactggccaaccccatccgagaggtcacatctaacctttatcctcagcaaagccactgaaggtcgctcaatatgtgtgacccgcaactctgaggccctggtgagaagctgtccaggaaaacgctggtgcgtgtgctagagggttccttttcactaagggagaattgtcttccagctccttgcagactgacatcgcaaagtactttgaacgttgaaaagaacaaaaaaagcaaacagtcacacacacacaaaaagtaggcgggaggagggggaaagaaaaagggacagagagagagagaggtatcagcaggggtggttagtaaaaaggggcccggagacagaaaaccttttgttcccggagttcgtttcatgtagagattgtgaggtgaatggctttgaaacgaaatgggtttatgaaggagttgctaggtcacaggaagcgcgactgtcagactgcttttgtgaattcagtttctttaaaatttgggttaatcttaaaaagaatgtatctccttttcctgttctttctctttctgtcttcttttttggcgggggcgggaggacagagtaaggttcaggacggttccccactttctgttttattttccaccgtctgataaagcaaaaagaagcgatcacattacaagttctttgtcagtttttcagaattaggggtgggcagggcctgagcattaccttgtcccactagccaatggcggggcggcatgcaaatgaggtccgcgatcagcctgcctcagtcacaacagtgagctcagagacttgagggaggcgctgcgactgacaagcggctctgcccgggaccttctcgctttcatctagcgctgcactcaatggaggggcgggcaccgcagtgcttaatgctgtcttaactagtgtaggaaaacggctcaacccaccgctgccgaaatgaagtataaggtaagagagtgccttttacaggttaccttgcaagctgaaagctgtgcctgcgggtgtgtgcttgtgtatgcgtgttccttactgtcagtcccttgtgtgtcccggagagttctaagatgagtctcggtcactgaggttgacatgcaagcagacaagcaagcagagacccggtctttgagacccactccaggggttcacagtacacccgagtccatctgctctgaaagttgccggggaaatacctcggtgagaagttaagacttggagccgcttcacagcagccactggagatcagagggtgtctgacttgaatcgcggcaggcattggctcaagtctccttggcttccccaggcctggcttccactgccctggggaactgtaatgagaggaatgaggactgcatagtctgtctcagactggctcttagtgcaaagttttccagactttgctttaatcgtttggtctcggaaggagtatgccatatgcacttttggtgggagaaattaaaagcccagattacacagctgaggatggaaaattttgacatccttatgttatattggatgtaggaataaataagtatgagccatttcttgaaaacatttttattggagtttgaatggggtgagagtgcgaaggctcaggctggctcattgtgcctgaaagcttacagagtgtcatagtcatagtacttcagcagcattattttccaatgcattttacaccattgtttgtggatttttcttgccaaaaggatttttgacttgctccgtatattcccccctcccctttttcttttaagtcactcccatctaaggaggcaagcagcttccaggggacacaaagaaagcagactgcaatgaattggacatgaatttttcttgaatgatgaatagacatgagtgctagtgctactattttattttatgctattttaaacaaaagtgttattattaagatggatttgggcaagggtgctaggcttgtggattgacaatttatattaactgtacactagctggaagctacttcgctttttttctaaatttttctggtccatccttttttgatgtaaggttgtaaatacttggtctaactgatagccactgactagcctcagtaataaagcttttgttcaaaaactatgaatcttattcaaaagctttaagtctaaatgtcaaaagtctttatagtaatgcctacgttaccactgtctgaagacacaggtatcagctatttctgtttcatcagctttctattatcttcatcagtagggaagatcagaggaaagggtcatcctgaagactattaatatttgactttaggatgcaaccagaaacaaatccctctacttggcaggaaagttatcttccttaaagtggctcaccccatatttccttatttagaacaatgataggaccagatattactcagcctggagtgacttttttgctcctcctttccctgttgttgaataagaactggcttgcagaaaaaagagaaagtatgttcatatgtctattattggaaagtataaatggctgaaattaacattgagtgctataatctagaaagtgacgaaagcgacaaagtctcaagtcacttttattcaatgatctcatcgtggttagctttactctttatggaaagaaaatctaaaggcaactgataaagtgactgacagcgtaaactgcgattggcattcatggagaaacctgcttctccactgggccttactggtgttgaacaccttgccaaatgatgtaaatacatgatttttattaccttgtaggcaccttcaccagcaaaaaagctaacttctccgaccgaacacatgacttatgccctatgatgactattaaatcaaccaatagctgaagaaatccactttccttttttataaagttttctttctctctagttaataatgaacaactttacttcaggaaaggattttgttattgtaagtagaggagagacacaaaagtaatgaagtaacattaattgagacttactgtgacaacacaagattgtcatattcaactctcccaatagctctacaaggtgggtattatttttatactcaatttcaaatgacacagagaggctaagtaatttatctaatgccacacagctagaaagtggtgagctgggattagaactaaggcgatctggctccagaactcatgactttaaccactattaagagaaagagaaagagctatcgttgacctctctaaaatatggccagtgttttcttctcccagaaagtttaagactatttcatcccaagtattcctgcaggataatttctttttaagatagtaactctacaaagcaaaatgaagtgcatgtttggcagttatttgtttaattcgagccacttaggtagtaaaaccagataattattagatggtaaaatcccagagacaggaattatctctaaaatactacgttgctctatgcactgtaaatttagcacaaaccttaaaatgtttactgaaagacttatgaatcaggccctataagattgtcgttgttaacctgattatctggtttggctgccccagggatcacaactacggaacaacaaaccttcacttattttgcacttaatatacatagcttcaggccaggcagcaaggtacttgcagtaatcctgagaactgtggaatgtaagctattactccggacagacatttctggttagcacttatctaatctgtctttatttccctgtatgtttttatttgtccacaggaaggttgcagtcactgtcatacgtacttaattttccatttctcttagaagggattcagtctgtggttatgtgatagtaaattacgggggcttcatttattaagaattttctacaaaatccccttcatatacagagcatgttcttaattgggcgggggctggcggggttaggtgattgcctcgatggccttggtttgcttacccagtgaaggctccctcctgagggtctggaggtgtatggttgtgctgtttcccaggagggtgatggaagggtctctgcgcagctgtgtttgagcagaagcccccgagaccccaccccgtttgtgcctgccaggcccgaggccccgcccacctcaggcccagcccgggcgggggctcagcggccccttggcctggctgctaatggctgagcagagacgcttttgtggctttgccaaatttctgagcccttacgtgcctacattaaaattctaaattatttatctcgtctaccatgcaacaaattcattctttaacgttttgactgaagaaaaattacagacggaacttacaatgccattaagaaaggtgcattctgaaagtcagagtcctgtgttctggttgaatggggtaggtcagggaaaggagaacctgtgtgccgtgaaacgctttggaaaggactttgaaagtattcgtatttcctcaagcaagaccgaggaaaataatgacagaggatctttaatttagtcaatatggtcatgcataagctattaaattcccaattatttccttgctttgatattttggtttaaaatgctttatttttctctgtatgatttttgcaaccaatccaaatgtaggactcctgtccttttcctttttaaaccttgtatgagatctatggatttaaaatcactaaaacatgctttgaaaaatatcaacttggttatttatgtatttatgcatttatttatttatttagtaaacccatttgcagagctaaatggcttacctacacagagataaaagcctttagagtactgaaggtgcctgataataccaaatttagcaagttgtacagtgcgtaacatgccaaggattcctttagcatcctttccttgctgggatacacgtcagtccctgttctcagaattcagtggttccctgtctctcccttcactccagtcttctgaaaaaaacaccttcctctccacttttctttttttctttttttgagatcaagtctcactctgtcgcccaggctggagtgcagtggtgccacctcagctcactgcgacctctgcctcctgggttcaagtgattctcctgtctcggcctcctgagtagctgggattacaggtgcccaccaccatgcctggataagttttgtatttttagtagagatgggtttcactgtgttggtcaggctggtctcgaactcttgacctcaggtgatccacctgcctcagcctcccaaagtgctgggattacaggtgtgagccaccgcacccggcctttttgcaaattctctcccactttcgtgcttttatgacctcattggttctccttttatcttcttcttcttcttttcaggctttccttacgcttctttaatactgacttccgtagatcttacttccaaccccctactccccagccccccacccgcacctatctactgccgcccccttgcctcccacacacagatgtgacacttttaatgcacattctgtagccctcatttttccttctccttagactctgctatgggaaatcttggtccctcactgcccccattcatctgcctctctgtttgcgtttacatgacttgagtggcctgtcagtcccgctagtaaagtctcctcatccatccactctgtttaaacaatcaaactctgaaacctgtgtctcctggaccatcctataatccctaaaataggctgttatgcttttcacctctgccctactctgttagcactaccttacttattgacctctttcaatcaaatcgttatctaaaggatacctgtaactcagataggttgcctactgggcctgtttagttttaagtaaaccccactgaatatgagagacccaccctctatttgtatgtagaggcagattgatcgaaaagtccttgaataaaaaacatgatctagggtctgtgaagttttgagggggccaagacttggtgttttatgctcttgtgttagagacatgatagagcatgggctttgaagaaaggcatttctgttccttatggcttatagctctggaccttaggcaagttaagctctctaagcctcattttacagcattgtctgtaaaatagggataagaataactgcctcatactattcgaagacctgggataatatatgaatgaagtacttactatggctcttggcatatagtaagcagacaatgcaagctggctccagctctctttgtatggtagatgctcaatagatgttgaaaggatggtatgtactcaagacttggtgacagaattatgtcaaaatcccagttactaggttgagatggttgaatattgttgagtattctgtgggcctggatgtgtattgtaagcatagggccctaacagcatatgaccccacttgctaatatactaatgacttgattccttcattattgttcattggactcagtattcctgaaattacaagactttgctcatagaagacaaaatgtatacacaaatagccatttaagaggatcttaatactatatggcatagtaaaaaaacaacaacaacaacaaaaaacatgggctttgtttcagatcccacttttgttactttctaacagtatagttttatgctagctactttaaaccttcttttcctcatttatcaaatgagaataatacctgtcttgtcagatagttataggatataatatatgacaattgtcctttctagcagatattaggcatttaataaatggcagctattatatgatgttatatacacatacccacaaagatatacagatatatagatatggaatttttatatagataaaagtgtttaaaggagacattcactagaattgtttacccataacagaaatatcagtgaggaagagaaagtcgtcaattcaaaaaaccaaagataaaatccaaagaatgtaagttgggagtacatgagaagttcagggtgaactctcttatccaattgcagtcaattagaatgacataaatgtaaagtaagaggtcttggttgtctatgtttagatcattttagggtcagaaagaaatctgaacaaattggtttgaaatgccaaccactaggaccaaggcaatactctgcaagaacatataggctgaattaccaggacttctcgccaagacaaatgaaacagggccattgggaagaaatactatatttctaacttaaaatgccagagagtaactgacggtttcctaggtgatagatggttgcaaagagtacgggcatgaaaaggggacacacacacacaaaaaaaaaccctgtttatactttgccaacaacacccccctccatcttatttactttgaacattccagccatctctctgcagtaattcctgctggctaatgaggattccacacagctagggaacatgacagcctgcaaaggattattttcctgaacaatctgcattttaagataagtcaccttgttggtaaccttttgtacccttcattggaaagggtgactctctttgaagacagtttgaccaaacaatgagatctaggtgaatttgaggaagatagaacgggcactccagaaatatggatagtggtggagctgacagcagtttttcatggttgacgtagggagtggaggcagctgtcatggagatattaaagttgccagtggaatgttttccaatacatattcctgggccccacaatggactattaaatcccagttattctttaaaaaaaaaaaaaaaaaaaggccgggcgcggtggctcacacctgtaatcccagcactttgggaggccgaggcaggcggatcacgaggtcaggagatccagaccatcatggctaacacggtgaaaccccgtctctactaaaaatacaaaaaattagctgggcatggtggtggtcacctgtaatcccagctacttgggaggctaaggcaggagaatggcttgaacccgggaggcggagcttgcagtgagccgagattgcaccactgcactccagcctgggcgacagagtgagactgtctcaaaaacaaaacaaacaaacaaataaacaaacaaacaaaacagctagtctctttctccctaatcccctcactaaccactactagtgcttctggtgcttacacggtgtctaagtaggtagttcatgatccttattcaaaggctggatccagtgatttgtaagtgtcatgtttctttgcaaatctcagtcttgcgaattagaattccccctgatatgtctaacatatcaaggtaatagttatatgatgttactaaaaatgtccctcacatgaaatgttatgtttatgcccacaggaaacaaagatttagcaacaaatatgtaaaagtgaaaccatttcaagcaacaaaaatatttgatagcccttttgaaattaatttgaattcctttttttactgtgtgtatgtgtggttggggggcaggggggcggtggatggattaattatctgtgaaacccagtagaaagttgcagtaaccaaaacacgtgtaaagttcagatttgaaccagatctcctgtctacttcttaaggcattgtgcatttagatagtatatgtcattcatgtttttcctaggttttattggtcaggcagaaacactgtgctatctcttggtaactatgagttagccttaatctcagtgattcatgacagtccacttgttttccttaatttaatgcctcactcccacaggagatgaggctaactgaggactcatctagaggactctttaagaatgagctgggcttttctgccccccaacaccctccgcctcccaaaataaccataacaggcaaagccagcacacagaaaatggcagtaagtggacttctagacactccagctacttctgagtcttcagtgtcaggacacatcagtcatctgtcgatgagattttttttttcttttccttttgttctttcgttcttgttactagtcactgtggcatgactgagagtttggcaggaaatgggttcgtggacctgtggtacagtcgcactaccacagcagcattggcctagcaaaatgttgagccctctttcccttgcatgctcccctggggcagaagtccagtgctatctccgcttccctgaccctctccactcagagcccagcatgacaagcacacctttaaatgggttcaaggaagggaatagcagaaatgaacgcagcccgacagcctcctttctcttgataacccctgtcactgtggagctggacttctaggctatctcacagaggcccagaggcactggaatcgatctcatttccttacagacatcaccttgtcaattagagaacacataacgttgattgaatttaagattcttatcagtgcctagctctttttctcccaaatccgaaattcagccatggcagatccataatcaagaaatatacttacattcccatcctttgttgttggtttcaaaaatatttcttttttgtgagtatgtatccatgttttacaaaccaaaaaaatgggacatatggtctgacaaagggaaggatatttgaacctggggactgcctgggagagtccggaagcacatggtcactctagagactgtcatcaagggctgctcctgagattaatccactgtcgaaggcattatcccatctcccttacagcagccttttgcaggaaactgtctaagatgttgtgctttttttttcattgacttgtaaataacaaggtgctctctttccttttctttgcagaaataggcatctttagaaataaagccatgcccattttgaaataagaacttgtttggaacacctgagagtgttaagcagtgcgggggatttgcatccaattgttcttgctttaaacctggcatgggcgctctcgcctcatagcccgcagcacctgaatcaagcctcctgcctcccttattaagatcttaattacagactcagcttagttcattgctgaagggaaagaatttcatttctctgaagtgtgtctgttttttggtgtggcaggtgtaatcatgataagatcatttctgggttttttgttttgttggtttttttttcctagaggaagtttttttttccaaggggaggagtacagttcttaagacacaatttcatgagctcatcttggcgcagtaataataactgtgctttgattttatagagactctttttcctgaagaaatcagagcatttggagtaaataatctcatgattcctcatatttttataaagaagaacatgtctattaatatttattttgcagacagggaaacagaggcacaaaaggcagagatttgatggtcattagtcttcaaatgtgaagtctgaagctagaccctcctaattcagtctggtgtccattcctctatccagggtttctcaaccttggcactattgacacttagggccaggtcattctttgtggtgggggctgtcctgtacactgtaggatgtttagcaacatccctggccactctacccactagatgccagtaacacacgtgtgcatgcatgtgcacatgcacacacacacacagtgacaaccaaaaaatgccactaaacattgcccgtacccagaggggacaaaaatcctcctagttgagaagcagtggtctaatctcttctactccttctccttaaaaataactgccctactcaaaaatacccccatagaactgactgccataattttatcattactgatattgagcttaatgtaacaggtcctaaccaaaaagcaacttcctcttacaggcctagccccagtttgtttcagtgaataccacaaaatactaagaagcgcagagtttcattcaagtcaaatgtaaaacccatcaaaccatctctaaggcaactttaaagtatttctctggcttctctctctacaatatgtacctcatcatggaacatgcatttagagctgggtctttaagaaagctattttattctcataaactggtgtataacatgtgcgtgtaagagcttgtctctccacctcggcactgaacaatttcacaatgaaggttttttgttccctttgctcctgccaccttttccctgtcttctaactaagaagctgcagcttcaaaaactcttccttgagacagcttagtggctgcattgctgacagtgtatgactgtaaacacctctcagccaagtgtgtgaatctgttttctaaaactctctgaggacctcacaagtgaagtagataataccaatcaggcaccaaatccaggtcaagtgacatctaaaagagttccagggagggttgcatcctatttacatcaactcggttctggctgggagatggacaacagttgccaggatgtgtatgcatttgtattggtgggtttagatataaccttgggctgcatagcttggtgaaggaagataagatagacaggaatggaaaaataggaacctctttttcttctttcaaacaccttatcagatgttataacttgtgcattttgactttgagaaatgacatcatttttggaagtatattgtaatatagtagattggggtctcctactccattaaaacttaattcttatttctcttccctgagtacctggatgttagagggatttgtctagacaggcagatagatatgatccagtgccaacactgtaatgctggctgaaatccagatggttgttttattgttaataaaatctatcttgtgggtgggtgggtgtcaggccttcatcattatatggtgcctgtcagatttatctacagacagaaccctgaaaacagcttgtgcctgccccgcatttttgaccccttgccaagatactgtactgaaatctatcaaaatcaggcaacctgggacaaatgcttcgagattccaaggcttaatagcaacagtgctgacttctaagatggagaagattctcaggaagggcatccttgtccggtggggaaaaattctagattaagaggtgaaccagatgctagctctggctctgccgctaatctgagaccctctgggctgtaaaataaggagattgggttagaatggttccttcttactctgaaattctactctaatcaactctggtcaaggtatgggtgacttctggttctaatacctataaaaaacctaggtgttcttcccccttctttttttctttttctttttctttttttttttttatgacagagtctcgctctgtcacccaggctggagtgcaatggcgtgatctcagctcactgcaacctccgcctcccaggttcaagcaattctcctgcctcagcctcccgagtaactgaaactgcaggtgcacacctccatgcctggctaattttttgtattttagtagagacggggtttcaccatgttgcccaggctggtcgcaaactcctgagctcaggcaatctgcccacctcagcctcccaaagtgctgggattacaggtgtgagccaccgtgcgcggcctccaccttctttaagattctcaggagttgcttcggtaaacccaaagaccacagatgagtgaaaaagaactcagcagtcaaattcatcttccaccgtgggccaggaaataatagaagttgactgtgacattgcacgtatacacacatatatgcaaatctgcctactaactctttgccctaagattttgttggttacatagtaaacaaatcctagcatatgaatgtgtctgtccagcacgaaccctaaatcaagcaagaatagatggcattcattcaagtatggggaaggagaggaacccagcttttgaggaacccctttgtaattgcacagctatgctgtccatatcatgttaccaaatctggtcagagagagatttctttctgagatccaaatatccaaatttgcagtgagcatcagatcttttcaccagtcctcaaaaagtaacttcactttggtatatgagccaccaaaatagtgctgggttccaaatgatccttcatcagacaggattggccagtgtggaagagatgttaagattccaagccctggatctacaaccacacacagggcgctgccccacagcacatccagggagtattaacagcttctcttgccatgtcaaagagtaccttcgggaggcaagtatttaatgtcacatttctcaaaccttctcccactcagacatgctcaaaagagaatgctatagctaaagttcacaaagctggaaaatctaagaaaacttgaggactcggggcaaagtgaatgacgtcaagattcggcgggggggtccaagatactcctataagctttgtaactgtcataggggtctagaagaagcacttcccagaaaataaaaattactgcctgaaatgcagtctgggtgccacaggaggccttgtgggaaatgttgaacacctctcagcagtgggcagaaggatgccagggattagtgggacaaagtggggtcctgcttttgcctttctgtgagctccattcagctcacctagtgaaaagtgtgtcagaacacagtcgacaaatagtactgggaaaaaattagcatatcttatattatatcataacttatcatatcttctgtctcctgtattgaaagcttcatgcctgtgacttcataatctcaagaggaaccaactcaaaaaattcgacattccagatcttcagatgcaagaacctaagtgtaaaccaagtattctgagaattaaaatcctgacacttacagatatccatgttttctgactatggctgtttccttctctggggaaagcccacatccccctctatcccaaaggtgatggtgggaaggaaaggagaaatgtagccaaaatggtttgcagttctcagaccaaagccggttttcgtcagtatgcacaaaagcacgtgagcctttctttctcttccctgttgtgccctgagactgaccttgacaatgttcatccctcagctgcctgccttaggactgacttccttgatgatggccatttccttgaatgtgtctgtttctcagggtctgtcctctgcatgcatgcatttgcgcatgcaggcatgcaaacccacaagagtccaggctaaagttttgggggattgggtacaggaaaatcatgtcattgagaatggggcaaccctgaggccatggcaggatcccctgcatgacaaatatagaatgaagtaaaaataatcagaggaagccgggccattgatgatgctatcagtcttagtggggtgatacaccagacattctgtctcatttctcttcaaacgaccgcatgagtggtcatggaaactacaagtcacacctctccgtatttggaaaagcagatcgtttctctgacataggagtaataagctttcttgacattttgatagcagtgagggaagggaaaaaaggcagggaggagttggaggtggggtgaggggtagaagccgtcatgtgtcctagagctctctgtaccagcgttctggtcaactgtacagtattttcttcccactcctcaggcatagcttgggaaccaggaacagcagaacccaagtggtctggcaaagtgtttgaatggtgctctgtcacctagtgccaaaagcagattgctacactgaagggagaaaggctcttaaaagagaccattgtgtttaatctcactgggatggtcagttcctcttggccttcctgtttgctccgtagttgcgaacactagtttcaggggggtcaggctcccgatctgcgtcattatcctgtttaaatagggaggggcaggccctttcctgctgtctgtctcccatagtctctggctgtgaggcttgagtgacttggacatgacatttctctttctggttcattcattttccccacttccatctgaaaattctaaccaaatgtcttgctgaattctctaagtacaacaatttcaccctccctgcagacaatgaggaaatcagagtccagaatccatttcaacttagcaaacatttactgagtctatattttgtttcggatactggggtaaagttctggaaatgcaaaaggaatttgcatctctgaacttaaggagttcacagtcttgaacagggcaatccaagttgtactgtaaagaaatagtatgatcgagaactgggaaaggaaacagcctttgaatagatacccattctggttaaatggaagatgggtttcgagggaggaaggaatttaatgcaggaaagccaattgggaagcaatttctgtgctacagaaaaaaaaaaaaaaaaagttgctgaagacctgaatgaagggtggcagtgaggtggaaagcagggccccagatgggttgcaggtcatgaagagacacagcaaacctctgcggctcttactgcacagctgtgtgcatgctgttaaccaagcaaagcaaagcaggagaaaaaggtgtttgcacttgcttttagagaggaagatgcccattagactggatataagggactggaatgcagaagaaatatccagcgaagactatggctttaggaattatctgtgtgttcagatgccatcctcctgtagagcgtaagcacatagctgagaagaggaaagtgcaaaggacaaatctctttggaacatgatcactttagggatgggaaaaagatttagtctccagtggagaataaggatgagagtggtcaagagaagacagagaacgaaaaagtggtatcgtggaggccagaagaagacagtttcaaggaagcttgggctggggatcaaggctagaggctgctgcaatcagggttccctcagatagggctcatgatcctaaatgctgatttgcaatcctgattagagccacagcttgtgttgcacctgtatttcacttgactaaattctgtcctaattctagacctgaagacaagaggcctgaattcctgtctcagctctaagactttcttgccaggtgagctggcaaatcattaacttcttgaggctcatttttttcttttgtaaagtgaaagggttggacggtaattgtttaaagttccttctggctttcaagttctgtgccctaactgttttggtgttttgccaagctctagctgcactgctaactgccagcctttggagactaaccatccaagtgaatatagagttacatagctctcttatctctccttgatttgtttctgtgttgaccttccctaccctggagataaatatccaagggggtgagtgggcaggagaaagagtacatcttgagtagattaaactgcctctctggggtttttctaagatagcagatcatcagcttctgactttgtggctcaaggaatcacacctttgcactgaaggagaggatccctccacttccttgccagaagaattcattcttgattttcctattacgactgatgtgcacttttgaatgagatggtttatggtccagctgaaattcatttggctgttatggtcttactgaaaccttgcaccaacaccaaatcttttcgaaagtccaactcctgcctcatgccttttcctacctgctgatgtattatctgtgttggaatctgatgacatttatccataatttatcaagtagtatcattattaatatgttgtctcagaagttcccttgaatgcaaccaatggtttcactattgctgtttgtaggcagatactcaacaagaggttgcagtgacaagaactcattcataattcagaaatatactgctttaagataacagttcttctgaaatgtaatcctgagcaagataaatatcagataggtacaaaacatatataatagcatcattggaataggaccaagcctggactgcaaatggaaaggaggcaaggcggggagggagcctgaagcccaagggccatctagcaaattaaataaaacatcaccatagcttaccaaagaccgggaaactaaggcccaaagggatgctgttgcctggcaaagtaacacagctagaacctaagaccgcaaatatccaatttattccatagacacaaaaagaagaaccgctcctcttcagaactttatcatataatggaactgagcccagtaacaaggatgctgcgtggctgagctaaggtagcttaaagttctggaaagaggattaaactgaaagaacgcaattctctttccatcgctgccaatagtgtggtcttgggcaaatgataaacttcaaatctatttcctcatctgtgacacaagggcattgtgtccaggtgatctctaaaggtccctggagccgtaagcttcggtttaggagagtggctggatgtagacattggctctctgtagcttgcgcagatattaaataactcatactcctgttcggccaaggctgagaatatgtatcggtgtgtgaataggctggtgccggggtcctggctactaacagcactgacaagctgtgcctgaaacctaatctctatgggcactgaggaggactgctgggaagtcctgacaaccagtcaggaggactcacctgcggtgcccacattagcccagactgtggggctctgagagtttcccccaagaagcagctcacaggccagtgtagaaacattagccagctgctcaccaggtggtaagaaggttactggggcaggagacaaagaacgcccaggacgactctcgcacggggatttctatctgcctctgatcaagcatgctccggtgctccacttcagtgcctcatggtgctcttggagttggaagtggcccaattccgaatgccttgagctgatttatgctgattagatctgtagccctttgcctttctactgttttctgtttctcttctttcccttctttgtagccagtataattgcacagctaccaaccctcagctcccatacaactagcccgactctgttgcttctgatttcatgtgggggcttcccgattgctgaatgggcccagaagaaagggacagacagaggccagagtggtcagctatctcctcacttaataatctcagtacagctctggtggagtcatttcctggaggtcattttagtaaaaggaccagaatcttgtcctctgtaactctatgacttctcttgtaaaatacagaatacccaaaagatgggagaagagaaacagagacaattttaggattatgacaccatccttaaatggttccatgaacaggggaaactgctgcctgattttttctttatgtatgtgaacttttcattgttagatgaaacccagcgcctcctggaatattaactacccagtgaaaccttcccctgaaatatgcactcctcagtttccctttagcttccctggccgctcacctctctgtgtctcacacttcctggatctcataactgtcaagaaaaaggacttcaaccttattcttgaagagtatcacaaagcttcctgaggactgtcctctatggctttatctcttttaattgccctggctaagaggaacctggctcacagcagcagaactggacccgtcccaactactgaatagagggcagatcccttccattgcacagccctccagagcggaaaacacacaggacccgtggcaatggggctagcacaaggggacgcgagtagtgcaagtcagctgcaaagaaatgaaaagcacgaggctgaatgatcaagtccacgttgctagagaagaaaatagacagcaaaagctcagacaatgacagccgaaaatcccacgaatatgtcatggtataaaataaagtcatgaacctgccccatccaatccgtaatcctttcttccataaatgagccccacctcaatgacattaagtgcatccaaacatcttaacaaagcattagagttcacttttagtgttccgagggcttgtgctgaatcaacaacgtccccgacttcgctgtgctctgggaagggggcagacatgcgggaatggctgcccgcgtgctgggaaactttactaatgccaagaaatgaaatcttccgagcctttgaaaggcctccaagaatgtcagcacgtactgcctgcccactctctgctgaatgcctactttggctgtctgcttagtactgaatgtgccagacaggccttcatacaaagacggagagtgtgttgggcccatgaaaggggaaggcacagcttttctgatgtgaatggtgagattcaagaagtaggtgacgaaaggggagggcgaggaggggccctcaggaaaggtatgcataaaagaccgagagagaagagttggcatccacctatgtgttaataaatttgttgtcaaagctggagatgtatatggctgctggcctatgctccacgcttgatggcatgtctacatgccttgcttgtggattctctctggatccaaggctcctgtcatctgagaacaagaatttctaagccctgccaaggcatatatatgtgtacttctattggcttttcaactccaaatataaatgctatttgtactgtgtgttatttgggatttttcttttactcttttcacctccaatatagaacaatattgagaaatgttcattgtcgaacatctgaatatctcgggatttttttttccttaagctcactttgaaaaaggaagaaaaatgttttgtatagtgaaccatgctctaactctgtaacactgctactcataattccttggcacggcatatcctgctagaggaaagaactcttctggtgttttgagcttttccaaggaggcagtctgatgtcactggtggcagatgcagtgtatatgtatctgtcttttgtctgcaccatctgtttttctccttacagtctattgttcagatttatgcttctctctttccaggaagtgtgcctttccataagagcacgggccttaggtgataaagggaccgacccaatattctaacacggtttccttctcttccttccctcctagaatcttatggcaagggccttatatgacaatgtcccagagtgtgccgaggaactggcctttcgcaagggagacatcctgaccgtcatagagcagaacacagggggactggaaggatggtggctgtgctcattacacggtcggcaaggcattgtcccaggcaaccgggtgaagcttctgattggtcccatgcaggagactgcctccagtcacgagcagcctgcctctggactgatgcagcagacctttggccaacagaagctctatcaagtgccaaacccacaggctgctccccgagacaccatctaccaagtgccaccttcctaccaaaatcagggaatttaccaagtccccactggccacggcacccaagaacaagaggtatatcaggtgccaccatcagtgcagagaagcattgggggaaccagtgggccccacgtgggtaaaaaggtgagtaaatgactaactaaatttttgttcctacttatttttttttcccattacacttggagcatttggaaatgttcccaaattaataacttgaagctgccaagaagtagatataaccaataccttagctcaggcatcatgtttgcatgattttgccattcatccatcattcagcaaaacttctttgaactaccatgtgctgagtacagttgatttccagccctcctaagttcctgtgtcatcctgggttacatgggttattaaactgtttctctccatctttctcatatatcagcttctaagccttcactctgtgctcagatcgtttcctatcttttctgtttcttcattgagtggaacaaacaccaaatctcgtacaagcctgatgatgcaacaaggatcctcccttggccaaaagctgaatcatgacctcagtggcctggctggacaaggaacccacccaaagtagcgagagtgaggaagctgggagtatgtcatgctgaccaactcgttctatagagttatcagcttagtttgactcatttaaaaatgcacagatactagtggaattggaatgaagccatcctcctgtccttcaagtcattcttataataatgcctgaggcagtgggtgaaaacagtggagcttggatatttaggaaggaattaatttaaaaatacagtgtggggagctctgcaacaccctgtgtaatcccaaatactttagcaatttgaggtcaatagaaattcactaattgaacaatgaatgttgagcatctaatatatttttgatgcttgtgatacagtgattaattaaagataaacaaagccctggtgatgcttacattgccgtgggggagacagaagcaaccaagagaatgctaggtagggacacgtgttatcaggaaaataatgtcagtggactgatcgggggtaacacccacaaccaaggtgatgcttatgtgagcatcacaaaggagggattttctctttcatttgctggcaaattccaatgggtcctacaaggtttggtattaggaatgaacaaatttaactggataagaagatatccctgaattacaagaggaaagatgcaattacataccagaaagagcttgttgacccttagaacactaactatagatgtgtcctgccccaagtaaatctaatatgaagtctgattttacaaacctctgtaaattagggaatatctatttgatgtattagaatcctctgttgaaaaaacaaaggattcctttaaacaatgaaagcactaatgcatttttgggtacatggaaagaggcagcctagagaccctgtggagagcccttagtgtttggctggggaggtgccagggccaccctcctgccctccccatcctggccatgtcaccaccccagaccctgaccctgtgtgggtagattcctttaaacaacaaagcactaatgcatttttaaatcacctttgatataaaaagtatgttttacaaaatacttctcaagagcacgcgtgtggcatgaactgagcgtaggttcgttaagagggattcctcaagggtggtgcacagcttttagacttgtactgcccacgacaacgatgctgcctagaggtgataaactgacttgtggcttttcagtcttccttgtcctaggaattgtagattcaaagggaaaacaaaacctggcttctatctccagaggggaaaaataacagttgaaaggtgtaactataaataagtaacttcactcattcttagtcctggttgtttgcaccttaaaaatagctctcccacatctgagccagtgtgaggcagaaggggaggccagagcaggaaatgcttggctgggaggtggtgggctctaaactttcatcacagttgactttggcaggaaggtagcgtgttttcctttttagacccaaccttttcagctccaagtcagagaagcctaagccttcagacttcttccccttgtatctgctgggactgccctgcaggctttccccatggctccccgtccttccagagggcagagatacggactcatcttcccttggattgatgtcaaagggctggggtgctggggtgaccctcgggcactcacattccatgttttgttttgctttttttaagtctacactcagtagaacattttctgtttagcaaaaggtagatgagtcctgcaggaggaaatcaacttctgaaaatgacctgtgccagcccttccaggagttgcagccagggctgaagagtaggccgtgcctaaagcatcacacagtcagggtctggggtagtgacatggccaggatggggagggcaagagggtggccctggcaccttccctgccaaataccaagggcttctccacagtatcctgatcctgggtctctaggctgcctctctccatgtaccccagagcagtggttcacatccatgggagtgtggttgcctcttcctttcttttcactcccttcctcacttctcttttctatctctctctctctctctctctctctccccccatccctccctccttccctctccctcccttcctcccttccttcctttctttcatagtggagatggcttagctgctaggaggtgattttagccttccaggcaattgcaactgctttaaaaaacatctgtcaacatcttcctgggtataggatattctcagtgggtgggaatcattctaatgacttaagcctaggccctaagagataatcccagcacactggggatcaggcgtggctttttcatttttctgagtttgcattttagtagttttactgactggcttaataaagcaatttgctcattttctctttaaatttttcatctgtaagataatatgagcccagaactagatatgcctggtagtttaagctatggtctttaaaagctcttgaataagaaaataaggaggcagtggaatcttattctgagccaccggggtggggtttaaaaatgttaatgggcatagaatcacccagagaggtagggcagtgagtttaaatgcagattcccaggtctttccctcagagaaattaatccagtaggtctggttgggggcccaggaatctgcatcttattgagctccttgcatagttttgtgggtggtggcctaggactagactttgagaaacactgtaaagggaccatgaaggggctgggacatgctccaatctgattatgatttgggactttccatagttcaaaattcccttgatattgctacagactgtgggcttccgaagttttacccagcactgcttttttctactaatgaatcacttaaggaaaaaaaaaagacagtgaattctgccttctatcacttcaactttgctctcttggaaactccaacctctacccaccctcttgcatcccctccacactaactgacattcatcacatattaaatcagcatttagagaaagaaatatagtcataaaatccccacccttttaggaaacaagcagacagtgtgagaattgtggagagagtaaggccttcagggttcagctgatgctgggttgtttctccatagctgtatatcctttggtaagttactgaccatctctacgccttggtttcttcatctgtttaatgggaatgatactaactacttcataggctgtcgtgagaattaaacagaagcatacatagaaagtccctggctcagtgcttagcatggcaggggcttaaaagaatgcattcctctcaccttgcgtttcctttctcagagtttatttcctactacatcagccctgttgtgtttcttacgacacaccgaaggtacaagtgctttcttgctaacacatatgctgtgttttttgagtgtgtggctttctctttggttctgcaagaattctgcaaagggtggaaaaaaactctccaagttatctgaaaaccatatacgctgacacctttacttaatttcattggtctttttcactctgtgttttgtgcacagggccgttttatccattaggcgttgtaggcaatatgcccagtgcctataagaatgtttgggagctgaataaaagatcttttgactccaaaatatgaaacacaaaaactgcaaaatagaaattaataaacatttaggtcaatgtctaggaaaccatatcatgtctgccccattaattgttttatttagggcttataactatttcatcatattagaaaacagtatgtaggttatatttttctcactttgcaaagatttctaaatatgcatcatggttgccaagaacccacaggcaatcctaaattaaataagttactcatagtcgaataatttgaaaaactgaattataaaggaagaaaaaaagttttcaatttttaacagcaaaaattctacttaatatgggattatggtttggggtaaatgaaatctacaaatgttcaaaaccaaaagcctaaaaagatctaaaatagtctcatttctctgcttcaaagatcagtgaaattgctacctgagttcatccatttcacagttgatctgcatgggaaattatatgtgcttctctgatttttctttggatgtgtcgcttttattctaactgctggaactatttgttgtacctctttctgaagatcagtttggggctaaattacaagctccatcagcacaggggccatggctgcctcctgactgctgtaggctgagcacttggtagagcatcagcccacagatagcagcccagtgaaccaatgaacaggtggaagcaagaatcaaagtgttaaatgagagttaacctttaattaactgaaaggtggttctgatcttatcacacatccaccctcacacgctgctgctcgaatcccatggttcagctcattaccatctggtatgagaggtgtcagattatatacagtcatttccctcgctgaaggaccttccagaatgtcactgcctgtgtcctgtaagggtaactattcatatacaatcaatgagcaccttgatgcaaagcatgagtgatgtaaagaagggcttatctgagagtttaacttctgtgcattttgcccaatttagacaagattagttaactcctctgtggtcacctaaggaggaaaactaggctttttttttttttttttgagtcagggtctcgctctgtcacccatgctgaagtgcggtggtgccatctcggctcactgcaacttctggctcctgggttcaagcgattctcattcctcagcctgcccagtagctgggactataggcatgcgctaccaagcctggctaatttttgtgcttttagtagagacggggttttgccatgttggccaggctggtcttgaactcctggcctcaggtgatatgcccgcttcaggttcccaaagtgctgggataataggcatgagccactgcgcctggcctaactttttctactgaggggcagaacttcctttgcatatgttatgatttacctagaatgcctttcccttctattttccctgtgaactcctatccattctttaaaacccactccaaggttcatccccctcatgaagcttcctctctgcaacccagcagtttctcccttccctatggtcccagaatgtgttgtatattccattgatctcaagggcttcttaaaaatggaatggtctgccattgcaatgtgtgtgatggtctggactggggtaagtattgctttgaggtggcacttggaaaactgaagtaatattcagatttaccaagatcctatgacatcatctttaaggaccattttctaccttccaaaatgggtcacggccaaatgttggcaggaaatgattcaaaggttttagccaggtcttccaggcccattcctgaaaggtaatgtaagaaacagaaatagattagctacaatgtttgtaccttcctagacactgagtcatcacaaattacacacatacacgtacatacacatacacatacacacacacagacacccataagctgttggctaaggaacaaggacttcccttattggaatttgaggcattgtgcaatctggttgcccagagcgacactcagatactagccaactaagtgctatatattagcagcatgacttgtctaacaacaagcaaaaaataggtttagaggaaatgaaagcttccagaaaagttaaattctgacttcacctcactttctcctgttccttgcctatacacacacaaaatacgtacacacccaaaaaatactcctagggcagagggtacttcggtttcctcatttataaatcaataaagtacaactatgttccagaattgtacatttctacataaagataatcctaatgtatatgaattgtttgcctcgatacatgggttttggggctatgcagagaactgtacttgccatctaaaatgtcacccctgaagtttcaagatacattttaatattacacaaaactggaggtcattcagctcttgaagggcaggactttatgagctcactttgaaaatgagaagttatcttttctcagacaagtcacccgagccaaagcaatgagcaaactctaacacccctccttaaaaattaacaaaggtcctttttgtttggccagtgccaaagccttcaaactcagttgcacttcgttctaaattttatagataatgcatatttctaagagtgcattagtaacttcttataaacccacaccaaagcaaacagaggttaaccctcctttttcaatgatttcatgctaaatgactgtgcttatcagagtgaagaggtaagagactgctttaatatgatgtctggctaagtaggagaacactgtgagagagagaaaacagaataaatttatttatttaatttcatgataaacaatattcgttgaacacatctttttttttatttttgagatggagtttcactcttgttgtccaggctggaatgcaatggcgcaatcttggctcactgcaacctccgcctcccaggttcaagcgattctcctgtctccgcctcccaagtagctgggattacaggtgcccaccaccttgcccggctaatttttgtatttttagtagagacggggtttcatcatattggtcaggctggtctcaaactcctgatctcaggtgatctgcccacctcggcctcccaaagtgctgggattacagacatgagccatcacgcccggcctggttgtacaaatctttaaaaaaagacttgcttgactacattgtgcaaaatgcagaactagaaactgtcagcaatcaaaagcacttcattctaactagctgtgccttaaacgttgtcaagataacttctagagagatgtgctgctcctgtttaaagtgtgtcagtgccactcacataggacaatgtgtgttcctcaaaagtcggatgtaggtcgggcgcagtggcgcatgcctgtaattccagcactttggaaggccgaagtgggtagatcacctgaggtcaggagtttgcaaccagtctgactgataccatgaaaccccgtctccactaaatacaaaaaaattagccaggcatggtggtgcatgcctgttaatccgagttacttcggaggctgagacaggagaatcgcttgtacctgggaggcagaggttgcagtgagctgagatcacgccattgcactccagcctgggcaacaagagcaaaactctgtctcaaaaaaaaaaaaaagtaggatgtaactccagtaacatttgaagagtgccaaggagtcctctctttaaagggatcctacagtatatcagttttttgaagcaaagaagcctttagcaatgccacaatcgcctctgatttatttgattaatttttgtaatacttggttttcttaaagcatggcacacttaaaccagttatttattggaatagtttttgttttcaaagtcactaccaattgaatgtgcagccttcactggtgtcattaccccatgcttccgtctcattttgcaagatagtgttagaactaaagtgggggtgaccccaaggcgccttgagccttggctccatgttagggatcccatagaggtactaccacctgatcctctccacagcctcgtgaggtgcacctcacagcatttgctgttcagaggagggaactgaggtctgagaaggaaattcacttgctgaagttaacttgctgcctccagtgagaggcaggattgatatttgagcccacgtctgtctgactccaatgctaatgatttttacatcccggctgaaggatgatattgccaagcccttaaagaagaaggcatatttggacacctcattagcaatttgggcgctaaatcataccctgttggccaggaagaattaaagttgctgcccagggctcccacctcaggtccagggagtagcctcaatactgagggaatctgaattaaggagcttggaagttccccccacctagctgtagtgggcagtttcagagtgggctgatccaggagtcctgaccaggtcagtagggtgatgtctagactccagtaccactgagaatgttgctatgttggctttctctgccacacagaaaagtcttttctttccttttcttttctttctttctttcttttttttttttttttttgagacggaccctccctctgttgaccaggctggagtgcagtggcacaatctcggctcaccacaacctccgcctcctgggttcaagtgattctcctgccttagcctcccgagtagctgggactatgggtgcgcactaccatgcctggctaatttttgtatttttagtagagacaaagtttcactacgttggcaaggctggtctcaaactcctgacctcgtgatctgcccacctcggcctcccaaagtgctgggattataggcgtgagccaccacgcctggcctaagactgtctttccaaatgacttcaaattccttcaaatgggtaacttcatttaaccaggtgggggcacctcccaaaacacaagttacccagctttcaagttgtggctctcatataaggaagtaactttctttgagagtatttacttgtgaaattataaaagtagtaaatttctggaaaatgtctaacatgtattgctagcgtaggccgcagggcattgagaaacgtataccgctgcactgctggcccagctaaccaagggtctccttcacttctttgtcattaatagcctgagtaactaactccactttagttccctcaactgtgaaatggcaagtgatgctagattatctctaatgatctttgctaaaattttatgatccagatatccttatctgattctttctcagaatcactttaacagtttaataaaaacggcctgacatcaagagtttttttttttttaaagaaaagatactcaagcattgattataaatttcaacttgacccttaagtttttgcaaatctttcctactcttcctttaggatccagcccaccatcccatccagaaccacagtgccctttggaagacagagctatgccaaaagacagcaggagcaggcagggacacaaggaggcagggactggagtgtgctgagccagtgagaatcagtgtttgacagacctgggtcctgtacccaaaaaaacttccagagttccccattaaggagcactctcatccctgttttgttaccaagagctaagaaagcacttcatcctggaactcattgttttctgcccattttcccctatgtaatcctcttggattttgcagacgttttaggcctgttgtctctggacacgacaaccaccttcagagctggcaccgagttctgccttgtgagtggtttgccccatcagccactgcatcccttcttccaactaaacctgagcgttctcctctttaggaagaaatgataccaatcggcatttgggtcccaaaattctcatctctcacctcctcttcacagtccctttccccttagggcagtctgtgggcatctctctaaaatccatttcccaatctagatgtagcgctcagagtcctgttgaatttatttggacatcaaaagagccacaatacttgtgcttttttatagttttctttcaaagaacatttcagtccatgagacagaaaaaaaatggctttgctgtatccaacttgtcacaggcttgtatttggcattgttctgagaaagacctcaaccactcgtgaaacccagacgtcatttcccgtcgtgttctttcatgttaaatgcttctagctgctcgctggtgcttggtcactctataactaaatattgctttagcactggctacacaaagagcttcctgaaagcagcaggggggacatgctaggggcttaacaataggggcactgtttccattgagcgggtttgctgcccaacgctgtgtcaaatgaaagtgacccaggagcaccactgctccacttctgagcttccacttgtgactttttcctcactggggaaagaagctggctgtgatttagatgtggctagcaaaaggtttagttctggcataaaatcaggcatcagaacgactttgaaagaaagtaattcaccttcaaaaatacatggggaaaaaacttcatgagcaccagagaagcatttggaagagttaaccttggacatggcttacgagggtgtatttttaaggccagactcagttttcattatattgttgctatgcaagtaaataaatgagctcactgctacacccaagctgggcagaatgaatttacagagaattaataaatccagggtaggcaacatgtggcttttcttctggtcatagagaagcaactagtactcttggattttaagcaggcaaacctctgtagctttacagtttctgaaaattggatcccagttctaatgggcaggcagtgataatggtaatgtttcttttcctaaggttttctttaaagggaagggatcaaatagttcatttaagacaaagaggttattataaagtctaataaatactgtggtagctctgttaatgcttttcaagggcatttaagtgaaagaagccctttccaacaggcagttttggaaagctaaacactcttgttaattcatgaaacgcaaagagagataatataaataaatcaggggctggggaggaattagagatagacaggaagcagtcaaattttacttcccacatatgccaagaaaagtgcaaatacatggctgttacttagtaaaacctacttttaaattcagagaatcgtaggtactatgaatggtgaggttataaatctgtaatcattacagcacggggacactttttaacttctcatcaattacccattgttatttcctgagcacatcctgggttacctagctcctgactaggcattagggaaggacacaagaagctgactccacacattagtactctactaaattcatgggtaaactccactggtcaataatcaagtcactatctctatattggaggcaaaggattgcacaattcaggctatttgtaatgttgctttggattgtagagacttagactcagaggaatcacgggacatagaatctagaacaggtctgtgtcccatcattctcttaaaagaaaacctttcaagtaatatttcttattatcttttaaaatcttgttaaaatgacaaaatatatatatatttgtaatttttaaaattttgatgcatacaaagatagacatagatagatagataatgtagaagtataaataataataagtcactagagcatgactaactagtgaagttacccagtctcctctccatcccatctctctgtctcccatccactctacccaactcttcctttcaaagagtaggatttttctgcttcgtttttttactgctttgttcttacttagggttgctggaagcacatggaaggagggaagtagtcaaaacaagacagtgttgtgaggggagagatgagaagtcatgataagtaggtgggtgggtgacccacagggctggcatcagaaggaaacatagcaaaacatgatggatatgaggcttgctgtggggagggggattggcctttgtgagtggcagccgtctgctcccttcccgcttcccttagtgctccattgagctagcagcatgcagctgagaagttgaagttctgaccacatggcctctgctgccgctgctctgccccatcccaggcacctagccagctctgcattaaggaggtgaagtggatgcccaaggaaagaagtgcccccaaggagacttgctgagaccttgaacaagtgacacaatgtgagcagaacttgtcttgacagaaaatgctttgtctctaggtgttccagagagatgggcaagtgtcctatttcttagtgagagcctctaaacaaaccagcttgtgaacctccactgaaaagatctcatctgatgagcattttaataaagtgtcctgagtttggaggcttgccgtctttctcttggataaatatcttcatctcctagacttggaaaaacacattttctcctggggtttcccattggcgtgtcttgagctgctctggtgataaccgtaataatgccaatactgatacgaacagcagaaaacagtaaccccaagaactctacagatgatcatcaaggaccactgtctcttaccatttgctgctttggtttgaaattctcactgcctcgtagatctcattttgagcactatacattcctaaagattgatttctttctatctgacttaaatttaggaatgattaaatcttcatttctcccatgatttgatcctaaaacattttgaaaggaaacagccttgagatctgtgattactaagacatacataacattcttatcacattagaaagcaagaattgactgttgcttgtcttgttcctgttgtcttgtcccctgaattcctgtttatctttgattgtatgtgggacattgtattttcagtacatttgtagaaataatgtgaagcctataaagatgttctctgcctccagagagaattttgtttccttctgccagcctcataggcaagcatacatctgattccatgctttgagctgttctggcaaccctgatgtcttcagcctgtgcaagggtgggtttacttccagttaatccttattttggatacagtccttagggttccaacccaaagtcgggggtggtttggggtccctgccttggtgagccctatagtccaatgttcccccttacccaaagaagctgtagaaaacccagcacagcctcccaggcaccagtttcagatcagcaaaaaatagcaaatgcccccaggcttgaaaagcaatctcacctctattaactcttctcccaaagtttgacctagtaattctttattatccttgaactcttgacactattaagaagatcttttcggctgggcgcagtggctcacgcctgtaatcccagcactttcggaggccgaggcgggcggatcacgaggtcaggagatcgagatcgtcctggctaacacggtaaaaccccgtctctactaaaaatacaaaaaattagctgggcacggtggcgggcgcagtgggcgggtgcctgtagtcccagctactcggaaggctgaggcaggagaatggcgtgaactcaggaggcggagcttgcggtgagccgagatctcaccactgcactccagcctgggcgacagagtaagactctgtctcaaaaaaaaaaaaaaaaaaaaaaaaaaaaaaaaaaaaaaaaagatctttcctagcttttcttcatttttttaagttgtcttcagcaagatggttaatctcaattacctagtccatgatttctggaagtcaaagtcaaaaggtaaaatctatatagcctaggtgacaattacaataacaataacaatagctaaggcttattatggctttatgccaggtactttatgcacttgatctcatttaatactcatatagcctatgagggaagtataatttccattttacctatgagaaaacaggcttagaatggaacctttgttctcatagcttgtgagtggtagaaccgggatttagatccagctctgcctgagtccagcttctgtttgtcaattacttccctcttcagacctaattcttccaataagcaacagaaaaagacccagtggggccatggcctctggcacacagcttctcataaacgagcctatcacacatccccagaactaaagcaatcgtatgttccttctgatgttgaggtaaaaagcagggtttgttttggtttcccttttccaaaacactcccccacatgtttctggcttgtggttaagaagaacccaggtgttcatgtcacatacgagctcaactggggaaaaggaaaccatccagcagccctccttgcctgccaatagtggcttcacccaacttggggtgcattcttctacagtttctgatttctcaacttcacctaacattcccttgccttcttggatccctctcttgcccaacactaccatgcatggctgatagggcactgttctgccccatatcccatgggttctacttaacccagagctggcttacctggaaaccaagcttattctgtagtggcagacctcacgccatcttgcttaatagccttcagttttcctttagttgattaatgtatcactcaatagattatgcaagacctactctgctaggcactgtactaggccctgtggtttatatttaaatgaagagggaatgatctctgactttaaaatgctggaagaagagatgagatgcatcaagaccgtcaaaccacaagtgataagtgctgtcagagatgtgtggatcactggctcagggagttccaaggatagagacatattatctgtttgggaagggcttggtgggggaaaggcattcagccgggccttgaaaatcaattaaagtttgaatatgaggaaagaaagaagagcatctcagacaaggacatggcatggatgaaggcacagaggtatgggcgtgcagggcatctgtggaaatggacagctcagttctcgccgagggagggagttggtgcagagcctgggggccctgccttcagaagatttccaagaggaaggagggcaaaaatacacagatgaaggcaaagactggcagcccggaggccaaagacgcgtttagtttggccaagacactgtttttaaaatttaagtcaattttgaaaaccaggtttcacataaaattccaaatttctggcttctgaaaacgtgaaagatctggcaacacagggcgcaatgtcttccctctttcggtagaaggagttctgtctccccggcaccaaagcctggcttgtttcttccctacaccctgcttgctcggtccgtgagcatctgagtataggacccttgctctgctatgggtaccagctcagggaacacagatgcagaaacatcagaaagagtcccaagggcctctcatccaacttgctgactgtcatcatgctggttctcagacctccctatctctctctgctatccaaacacagaccctcctctttaaaatttcagcatacatggctttcaaaattatgaggcatgaaagtgtcaaaagcatctccagaaactcatgccgccaggatctgagactcaaaacagtgtggatcaaacaccatcaaagtgtggggtggggcaattcgagtttgtttccttgtttttatgtaagcagattaattagagaactaacataacgccagtctttgggcttttgatcctatcctgccaggacccagacttggagatgtattaaatggattcttccttttctaaatggaagaatctgcccttctcggcttcatagctcttctcaaagtctctgtcttggaccctcccgttagttactgagaatggtatactaacatctgagaaaggttggattcctcctagggacagaaaatccacatatggaaagtgcaaatcctgtgccgggtaatcacgaaagcagttgcagtagcattggatcatagagccccaggagacctcacaattcagcccccttcctggcaacactaatgaattaagaggtcagtttggtaattccaaaggctaagcctttgtaactataaataaatgcacagaatgaaaggaatgtagaaaaaaaaaaaagcaaacagagggggaaaggaaatgaaaaacctgacttgatttcattgagaaaattagtttaaaaatgtcctttgtgtagcaattcctttaatgcctcaccgaacaaatgcctaggagaattcttccaaacttgaggtccccttaaccagaccttggtgtgcgtcttcagctgaaattcagcagttctgggaggtggaatgaggagagatcgttggaaggtttttgtgtacttatgtcacgcagcaagaaaaagccttaatgaaccacaaaactggagactttgtaaggtacagctcagtcagcacttttcctccgaggagaggacacacaattggcatgaaagtgacccaagcaacaggtcgaggcagagaatgtccaaaagtagaagacttcgagctccctgatcttccacacgtcacaatgcggattgctgcactggacttggcatttaaatgggaccagcattttgcatcctggtcccatttaaatgccatttgtggaccaacgtgaattagatggtaatgtcaggaaggctggaatcggtggtggcgggcggggggtgctgtattcggttggcgtttcccccctgtggttttcaccatctgtttctttgaatgcataaacaaggaaaatgactggtttggaatgcagagttttaaaaaaccagaagaccacaggcatcctctaaatgagaaagagagagcaagttggggttctgtgacatttgtcaggaagtgaaatgttaaataccgggaagcattagcgctttctgccagggaagatccacaaaggcaaggaaacactttagcggtgaacctgccttccttttctgaggtcgtgctatgtgtttatatgtcacctagtgctattttcagacaccaacgccacccactctagctcccaatccccttctgggttttttgtttgtttgtttgttttgttttgttttgagacagagtctctctctgtcacccaggctggagtgcagtggaacgatcttggctcactgcaagctcctcctcccaggttcacgccattctcctgcctcagcctcccaagtagctgggactacaggcgcccaccaccacacctggctaattttgtgtatttttagtagagatggggtttcactgtgttagccaggatggtctcgatctcctgacctcgtgatccgcgatccttgccctcccaaagcgctgggattacaagcgtgagccaccacgcccagcctgtttgtttgattgtttgtttgttttttgagacggagtttcactctttttgcctaggctggagtgcagtggcaagatctcagcccactgcaacctccgcctctcgaattcaagtgattctcctgcctcagcctcccgagtagctgggattacaggcacatgtcaccacacccggctaattttatatttttagtaaagacggagtttcaccatgttggccaggctggtctccaactcctgaccttaggtgattctcccgccttggcctcccaaagtgctgggattacaggcatgagccactgcgcccgacatgcccgcttctgttttttaaacgaaagatgaacagttaagctggacttagccttggttttccattagcattattgctaagttggcaaccttggataaaatccactcttggaaacttttaagctgaacaaaagctgcactatgagcaggtgctatgataaagccaagacagcgctctaagtagaggggctgatgaaatagactaaggggagatcttcatttctctcctggacaatagcgagtaaaaaaaaaaaaacaatcatataagggcattaggaacacattgtgtttttctttagcaaagggcatcctgctttgaaaaggaaggtttgctatgcacaatacagtggccattctataaagtggttccgtatgctccatgccaacagacctcaaagcaataggttccttttttaaacccaagacagtggagagacttgatggaaattttgagtgcatactaatctcttttacttcgttgcaagaaacaatcagttgtaagcactagggattaaaagccaaattgaactcaggcattttgagagcgcctggggagaaggcattggtgcatttggctgagttccacccatttcagcataagatggacgtggagcatttttcacatagttctgtaggcagcctgacgccagagttttcacttcagagaaaggataaaagttgacggtttcttagggaacaaccaactcttcctcatttgcaatgtctgttctcctcaaagatgtcgtgggcaacgcttgagatgggcactcaatgactcaaagggtgggggttaggcagaaacaagaccctgggcatttagaagcccttggacgattacatatatttcaaaatgagttaagttcaaataattttttgctggtgcttagcacaccaatgaagtatgtagatatgaaaacaggaggctgctaggtaagattcattttattggcactggttccagatgccagcatcgtgatgaacgctatttgacttctgatatcccttgacgtaggtactgttggggatgttttctttcctggtggaaatgggaaaatgattagagaccagaggtcaggagacctgaattctgttcctggtgcctccctgactcagtattttgtttgtttgatacgttagaatgaaagctcccagaggtttctaaggacagcacagtttgagcattggctttgtaaaagtactctggtgacctgtggaattacagttataatcatcataataatgtccaatgaagaggcatactgaggaaggcatgagaggaattttaagtggctaaactctatttgcattattcattttacaaattgtttcagagccttaaagcaaatttcagtatgcggtactttagatgcaaaatgctcctctaggactttcataagttacacacaagtatcccttaaagtatatttcagaaatatgcttgcagtgcatcaactctatctgatgaactttgagatgatcacaattaagggtgatagagatattttagggattttttttctcattgggattcaagagggatttaaaagtttactaacctgggccagatgcagtggctcacacctgtaatccctgcacttttgggggctgaggtgggtggatcacctgaggtcaggagtttgagaccagccaacatgatgaaaccctgtctctactaaaaatacaaaaaattagctgggcatggtggcgtgcacctgtaatctcaactactcaggaggctgaggcaggaaaatcacttgaacccgggaggcagaggttgctgtaagctgagattgtgccactgtactccagcctggggagcaagagcaaaactccatttcaaaaaaaaaaaaaaaagtttactaacgtggtgtctacttgtctccttcctgttatgtcttctttctttggtttctttctatctttttatgagggagagttgagggatgagtgcttagttaggaggcaaggagattcaaggactcaggcttggaaatttacacctctgtgccttctctcccacaggtgataacccccgtgaggacaggccatggctacgtatacgagtacccatccagataccaaaaggacgtctatgatatccctccttctcataccactcaaggggtgcgtaccagaacatggtcacaagaggagaagcgcttctaagggtagcattccttcagggctgtagagaaaagggagttcacaaattatgcattaatatatgtcatatgaagctttgtttaggttgtctacccagtagccactttagccaatgctatttaaattatgttttctggatttgctttatcaggaaatcctagtatttcacccaagagagcttatgttcttctacaattttgcttcagaaagtagatttttcttttttcttttttttttttttaagacagaatctcactttgttgcccaggctggagtgcagtggctctatctcagctcactgcaacctccacctcccaggctcaagcaactctcctgcccctgcctcagcttcccaagtagctgggactacaggcacacacaccaccatacctgactaatttttgtattttgtagggacaggcttttgccatggtggccaggctggttttgaactcctaactgcaagtggtctgcccacctcggccttccaaagtgctgggattacaggtgtgagccacggcccccagctggaaagtagaaaatttaaactacactttaaagtacagacagcgtagatatttcacataagatctttttttttttttttttttttttttttgagacagagtcttgttctgtcaccaggctgggagtgcagtggcacgatctcagctcactgcaacctctgcctcccgggttcaggcgattctcctgtctcagcctcccaagtagctgggactacaggtgtgcaccaccacacccagctaatttttgtatttttagtagagatggggttttaccatgttggccaggatggtctcgatttcttgaccttgtgatctgcccacctcagcctcccaaagtgctgggattacaggcgtgagccaccgtgcctggccaaaatcatttttatattaaatgtaagttaaaaaccataaaatgtattaaaaaaaaaggcaataaatctgttataacatggagcactgccaaagatcaagcttgtacataacctggtaaataaatccataattaagtgcttaggagcataaaaaatgaccaagtataagacatttccattctgggtaactcacgggtttctcttcaggtatacgacatccctccctcatcagcaaaaggccctgtgttttcagttccagtgggagagataaaacctcaaggggtgtatgacatcccgcctacaaaaggggtgagtgagtgactacaaagcagcaaaaaggagtgtgtgtgtgtgtctgtgtgtcggggggtgcagggttgggagggtgggtaagtagttcactcgaataaaacaagaaaggcaaacccaaaaggggaaaatgtagtcttggtgagagtaaaggaaggaagcaaaaaaggaaaggcactaattaaagatagctctagggatttcatattgagaagccccaactaaaaaacactaggtggccaataaggataaccctttggcagggaagataattagttcagtttggcaagtactaatatatatttgtagagggtttgttttgttttgttacattttgtttgagacagggtctcgctctgtcacccaggctggagtgcagtggcgcaaccacagctcattgcagtctttacttcccaggctcaagcaatcctcccacctcaggctcccaagtagctgggaccacaggtgcacgccaccatgactggataaattttattttttgtagagacggtgtctccctatgttgcccaggcttgttttgaacatatgggcttaaatgatcctactaccttggcctcccaaagtgctgagattacaggctgagccgcgcctggcctgtagagggtttgacagtttcctcagtgtgtatgtttgagtgaactcgtttgactcactctgttaccctatggggtatgcctgcacaggaggcacagtaatccctactttacagacaaggggactgtgtttcagacgcctatgcagctcattcagcatcacacagctggtgtgataaccaaaaagaccgggggagaactctggtcttactctgcctctcggcacagatcagcagagaaaggatacccaggaggtggtcagaaacacaggactggaaacacagggtgagcaatttagccaggagggttgtacatacgagtctgcaccaagaacgtggggttggacacacttggcaaaggacaagggaagtgacagcagaataacggggaaccttggaagtgcctaacattggggcgggggagggcgaccgaaaaagtgccagcaaataggactgagcacatgggaccacaggttcccatgagccaactcaataaatagcatttcgctttctacttgctttgcaggtatatgccattccgccctctgcttgccgggatgaagcagggcttagggaaaaagactatgacttcccccctcccatgagacaagctggaaggccggacctcagaccggagggggtttatgacattcctccaacctgcaccaagccagcagggaaggaccttcatgtaaaatacaactgtgacattccaggagctgcagaaccggtggctcgaaggcaccagagcctgtccccgaatcacccacccccgcaactcggacagtcagtgggctctcagaacgacgcatatgatgtcccccgaggcgttcagtttcttgagccaccagcagaaaccagtgagaaagcaaacccccaggaaagggatggtgtttatgatgtccctctgcataacccgccagatgctaaaggctctcgggacttggtggatgggatcaaccgattgtctttctccagtacaggcagcacccggagtaacatgtccacgtcttccacctcctccaaggagtcctcactgtcagcctccccagctcaggacaaaaggctcttcctggatccagacacagctattgagagacttcagcggctccagcaggcccttgagatgggtgtctccagcctaatggcactggtcactaccgactggcggtgttacggatatatggaaagacacatcaatgaaatacgcacagcagtggacaaggtggagctgttcctgaaggagtacctccactttgtcaagggagctgttgcaaatgctgcctgcctcccggaactcatcctccacaacaagatgaagcgggagctgcaacgagttgaagactcccaccagatcctgagtcaaaccagccatgacttaaatgagtgcagctggtccctgaatatcttggccatcaacaagccccagaacaagtgtgacgatctggaccggtttgtgatggtggcaaagacggtgcccgatgacgccaagcagctcaccacaaccatcaacaccaacgcagaggccctcttcagacccggccctggcagcttgcatctgaagaatgggccggagagcatcatgaactcaacggagtacccacacggtggctcccagggacagctgctgcatcctggtgaccacaaggcccaggcccacaacaaggcactgcccccaggcctgagcaaggagcaggcccctgactgtagcagcagtgatggttctgagaggagctggatggatgactacgattacgtccacctacaggtaaaacagcggaactcataaaacacctacactcactcacatgcagggagcctgagaaagatgcctataaggatgtcgggttggactgccaaaggagagaacataattaatgttaatctacatggttcacaaattggagggagtgtcgtagagtagtaagaacgctgggctgagagtcctgagtactcactcagatctagccctttctctgacgtttactgtgtgaccaacttattcaacctccttgggccttaatttcctcatttgcaaaatgaatggggtaaggggttggattagatcccgttgatatacctcaggtaagaggagactcaccaagtaggataataggccctctaataataataccagctccacttctatttgtgttttatgtatagttccatgcaatattttatttgaaaaaaaagttttcgtcattaagaaaaagaatagaagacctttgcaccagagaatttctaaggcccctgctagccctactctgtgtatgtgtgtgtataattgctttaaaacttagccccatctcagacttacctagaggaccactgggcattagctagctgtcctaggagcttaatctgtgtatgggacattggatagtcacagttggcctcctacaattgggaattctaccaagctccaagttgacctgggattccgacagctttcccttccactttgagggattaaaacattctactggctgggcgcagtggctcacgcctgtaatcccagcactttgggaggctgaagcaggtggatcacaaggtcaggagttcaagaccagcctggccaatatggtgaaaccccatctctactaaaagtacgaaaattagccaggcatggtgatgcacgcctgtagtcccagctacttgggaggccgaggcagaagaatcacttgaacctgggaggcggaggttgcagtgagctaagatcgtgccactggactccagcctgggcgacagagcgagactctgtctcagaaaaaaaaaaaaaaatctaccaagatccattgtttaggactaggcttactatcttattctgccattcttttaatttgactgagagtcacagattatactgagaactacgtaactattatgccaaattccctcaagcgcaagaaagtgtggcaaggagaactgagccccacctgatgctgaggaaggaagtggagagagagaggatggaggcattgaacattcatcttactggttgtctgaccctgcacagtgggaactactgccttggagcagaaatctatagatgatttgagggaactagaagtgagaggtggaccacatttagacctgcatttgggggtttacaggttcacatataatctatgagaaaagaacccagagactataaaaagaacattatatatgagatttgaagggaatcatgagtagctctccgaaaattttaaggtgccccagaaagctggcaccctatatggcaatgggctttatttttctgccacccctgtcgtctagggttcacagtgcctcactgggcatttgagatgttgccaaggcagtggaaaataaagagtatttactcatccgtcaatgaaattgttagcataagtgaatcacagtgatgacataatatgttctttatgttgaaaattaacagggtaaggaggagtttgagaggcaacagaaagagctattggaaaaagagaatatcatgaaacagaacaagatgcagctggaacatcatcaggtaagttcaatcagagcaaaaactgcttggcattggaaagatttcccacctagcactaaggaaaggtatcacttcaagagattatgattttgattcttccagctcactggcaggaatcagctccaaagcacggaatggggtttaaaagcaaagagaaggtttatgaccttgttagttcaactgggtgtacctgggttccatctaaacggcaatttttttaaaggctaaacctgcatatctaacatatgaggactatttgggttaaggcatttggtctcaagaaacaagacccattcaagctagcctaagcaagcaggtttatagtaaagccacagtaggggaattcagtaacagaaagtgaagatagagccaggtctggggagaactagaactgtaaattatctctccttcttgtagttcctttgcttctttctatcagtctacttcactctcacctattttctggttttctctaattatctactcatttggctcccctgtaactttgcagaacccataaatggccactcagaacttctatagatggcttttcatctcggcttcctcttccgatggttagctcccttctcttgttcatcagattcccaagaaagagtctgattgggccacgttgattgggccatttctctttctctctctctctctctctttctgtctctacctcgctatttgtctctctttcgccagcaacacaagcctatggtttgcctggccttggtccaatctaaaggtaggagagcagaattcaatgttttcaacatatatccaggcctatctactgaggactttgggcagggcatgttcattcaaaagctgggtatgagtaggggagataatgacgactattgctagaacaagggcatacaaataaagagagatggattgaggatttatttacaagccttttaagatgaaatgaagtgaaatggcatgtaatgacatgaaatggcatgctatatttaggaaatctgagttctaatcctttctggccaaccaactatgtcaagtcaggtaacctccccgagcttcagttacttccctataaaatgggaaagtaccccccccatctaatgacatgatatattgatgaacatatttgcataaagcctaagatatataaaatataatccattatgattaaataccttggaatatcaccttgtacctatttatgtttgccttggcatctggcaaggtaagactgcagggctttggggaacttgtagaaaccatagcaatcgctaagaagaaaacagattctagaaaagtaaagctgttgaaggctgggcacggtggctcacacctgtaatcccagcactttgggaggccgagacgggcggatcatgaggtcaggagatcgagaccatcctggctaacacaatgaaaccccgtctcactaaaaatacaaaaaattagccaggcatggtggcgggcgcctgtagtcccagctacttgggaggctgaggcaggagaatggtgtgaacctgggaggcggagcttgcagtgagccaagatcgtgccactgcactccagcctgggtgacagagcaagactctgtctcaaaaaaaaagaaaagtaaagtaaagctggctgtgcatctctcagagaagctggggaagctgggtgaggtgatcactgctccagctcatccctacgtccaggtgggagattaactgagtctgaagctcaggtcacagatagtccttatctgcagaagagaggtctctcttgagtcttagtggaatccctagaaattattataattgcaatttaaataatacaccatttggtagcaatgaggaaagaaggaagaaagccagcacctgatgcatctgactctgggtaaaacccccttcttttaacagctctgggggactaaatattatgatgcacaattcccattcagactgccttagaaactttttttccttaagtgctcatatatttatatgcattaatcttcctgtagtgctggatcataacatgtctatcaatcttgacagaaagagtaggataaacagaaaggggtcatgaatggtcatttcatctgagcatcctgagatagtcgaggctttctccgagaaggagcaaactgtcagtgacttacttgacaaggaggtcactacatttggttttcccttgccacccctcaacattaataaacatttacatagagcctactacataccaaactattataagcattttgtaaacgttaactcatttaacctccataaaggtgtaggtaacagggctgcggtttaaacactatgctaccttctagccagagggtacaagagaccagtagtccaatcatagaaggtctgagcttgaggatcatctttcccaacgtctacattttacaatttaggaaagcaaggcagcttgacccaggctttacagctcacatgcatctgacagttactagcgactaaaatccctgtcttttaactccaaggcctagtgaatttccattgcaacacactcccttgctctaatgagatctgctttcgtcttccttgcagctgagccagttccagctgttggaacaagagattacaaagcccgtggagaatgacatctcgaagtggaagccctctcagagcctacccaccacaaacagtggcgtgagtgctcaggatcggcagttgctgtgcttctactatgaccaatgtgagacccatttcatttcccttctcaacgccattgacgcactcttcagttgtgtcagctcagcccagcccccgcgaatcttcgtggcacacagcaagtttgtcatcctcagtgcacacaaactggtgttcattggagacacgctgacacggcaggtgactgcccaggacattcgcaacaaagtcatgaactccagcaaccagctctgcgagcagctcaagaccatagtcatggcaaccaagatggccgccctccattaccccagcaccacggccctgcaggaaatggtgcaccaagtgacagacctttctagaaatgcccagctgttcaagcgctctttgctggagatggcaacgttctgagaagaaaaaaaagaggaaggggactgcgttaacggttactaaggaaaactggaaatactgtctggtttttgtaaatgttatctatttttgtagatattttatataaaaatgaaatattttaacattttatgggtcagtcaactttcagaaattcagggagctggagagggaaatctttttttttccccctgagtggttcttatgtatacatagaagtatctgagacataaactgtacagaaaacttgtccacgtgcttttgtatgcccatgtattcatgtttgtttgtagatgtttgtctgatgcatttcattaaaaaaaaaaccatgaattacgaagcaccttagtaagcaccttctaatgctgcattttttttgttgttgttaaaaacataccagctggttataatattgttctccacgtccttgtgatgattctgagcctggcactcccaaatctgggaagcatagtttatttgcaagtgttcaccttccaaatcatgaggcatagcatgacttattcttgtttggaaaactcttttcaaaactgaccatcttaaacacatgatggccaagtgcccaaaagccctcttgcggagcaaatttcagaatatatatgtggatccaagctctgatagttcaggtgctggagggaagagagacctgtgtgtttagaggccaggaccacagttaggattgggttgtttcaatactgagagacagctacaataaaaggagagcaattgcctccctggggctgttcaatcttctgcatttgtgagtggttcagtcatgaggttttccaaaagatgtttttagagttgtaaaaaccatatttgcagcaaagatttacaaaggcgtatcagactatgattgttcaccaaaataggggaatggtttgatccgccagttgcaagtagaggcctttctgactcttaatattcactttggtgctactacccccattacctgagggaaactggccaggtccttgatcatggaactatagagctaccaggacatatcctgctctctaagggaatttattgctatcttgcaccttctttaaaactcacatatgcagacctgacactcaagagtggctagctacacagagtccatctaatttttgcaacttcctgtggccagtgtgtataaccccttccactatctcacagatagtcacagcgtccattccatagtctgtctcctcacatctgttagtattgacacagcacagacaccacaagccatcaggttcttcatggggcaggtgaaatacttctaccccatgggtaaatgtattcacatattaccaagagaagaagcacattatctatgatcttttggcccagttcttatttagcatttttattccagcctacttggaaacatgtttttatttgcaatatatgcctgactgaattaagcttgcttgttttaaacaaccaaatcattggaacagaaaaggatttaaaaaacaagaatgcatgatctcagagtgattaaaaaaaaatcagtggaaataaatgatcatagaaggtgcttttcaaaacaactgctattataattctcaaagtcctactctgccaaaagaagattaaaagtcatacattacattacaaggaaatgttcatgtgggaagagggttgctgaaaatcaacaacgcttgaagttaaaaagtgtgtctttgtagatttcattgtataatgtgtatttcttaggagatggctgacttgattgatctacgctaagtggagacatttcacatttttaaaaccaaatgttcaatctgtattactctttgccgtcttgtatgtagaggctatttttaaatcattaaatttttagatctctgttttcata

SEQ ID NO: 5 - DNA, 4550 bp, Homo sapiens
acaacagtgagctcagagacttgagggaggcgctgcgactgacaagcggctctgcccgggaccttctcgctttcatctagcgctgcactcaatggaggggcgggcaccgcagtgcttaatgctgtcttaactagtgtaggaaaacggctcaacccaccgctgccgaaatgaagtataagaatcttatggcaagggccttatatgacaatgtcccagagtgtgccgaggaactggcctttcgcaagggagacatcctgaccgtcatagagcagaacacagggggactggaaggatggtggctgtgctcattacacggtcggcaaggcattgtcccaggcaaccgggtgaagcttctgattggtcccatgcaggagactgcctccagtcacgagcagcctgcctctggactgatgcagcagacctttggccaacagaagctctatcaagtgccaaacccacaggctgctccccgagacaccatctaccaagtgccaccttcctaccaaaatcagggaatttaccaagtccccactggccacggcacccaagaacaagaggtatatcaggtgccaccatcagtgcagagaagcattgggggaaccagtgggccccacgtgggtaaaaaggtgataacccccgtgaggacaggccatggctacgtatacgagtacccatccagataccaaaaggacgtctatgatatccctccttctcataccactcaaggggtatacgacatccctccctcatcagcaaaaggccctgtgttttcagttccagtgggagagataaaacctcaaggggtgtatgacatcccgcctacaaaaggggtatatgccattccgccctctgcttgccgggatgaagcagggcttagggaaaaagactatgacttcccccctcccatgagacaagctggaaggccggacctcagaccggagggggtttatgacattcctccaacctgcaccaagccagcagggaaggaccttcatgtaaaatacaactgtgacattccaggagctgcagaaccggtggctcgaaggcaccagagcctgtccccgaatcacccacccccgcaactcggacagtcagtgggctctcagaacgacgcatatgatgtcccccgaggcgttcagtttcttgagccaccagcagaaaccagtgagaaagcaaacccccaggaaagggatggtgtttatgatgtccctctgcataacccgccagatgctaaaggctctcgggacttggtggatgggatcaaccgattgtctttctccagtacaggcagcacccggagtaacatgtccacgtcttccacctcctccaaggagtcctcactgtcagcctccccagctcaggacaaaaggctcttcctggatccagacacagctattgagagacttcagcggctccagcaggcccttgagatgggtgtctccagcctaatggcactggtcactaccgactggcggtgttacggatatatggaaagacacatcaatgaaatacgcacagcagtggacaaggtggagctgttcctgaaggagtacctccactttgtcaagggagctgttgcaaatgctgcctgcctcccggaactcatcctccacaacaagatgaagcgggagctgcaacgagttgaagactcccaccagatcctgagtcaaaccagccatgacttaaatgagtgcagctggtccctgaatatcttggccatcaacaagccccagaacaagtgtgacgatctggaccggtttgtgatggtggcaaagacggtgcccgatgacgccaagcagctcaccacaaccatcaacaccaacgcagaggccctcttcagacccggccctggcagcttgcatctgaagaatgggccggagagcatcatgaactcaacggagtacccacacggtggctcccagggacagctgctgcatcctggtgaccacaaggcccaggcccacaacaaggcactgcccccaggcctgagcaaggagcaggcccctgactgtagcagcagtgatggttctgagaggagctggatggatgactacgattacgtccacctacagggtaaggaggagtttgagaggcaacagaaagagctattggaaaaagagaatatcatgaaacagaacaagatgcagctggaacatcatcagctgagccagttccagctgttggaacaagagattacaaagcccgtggagaatgacatctcgaagtggaagccctctcagagcctacccaccacaaacagtggcgtgagtgctcaggatcggcagttgctgtgcttctactatgaccaatgtgagacccatttcatttcccttctcaacgccattgacgcactcttcagttgtgtcagctcagcccagcccccgcgaatcttcgtggcacacagcaagtttgtcatcctcagtgcacacaaactggtgttcattggagacacgctgacacggcaggtgactgcccaggacattcgcaacaaagtcatgaactccagcaaccagctctgcgagcagctcaagaccatagtcatggcaaccaagatggccgccctccattaccccagcaccacggccctgcaggaaatggtgcaccaagtgacagacctttctagaaatgcccagctgttcaagcgctctttgctggagatggcaacgttctgagaagaaaaaaaagaggaaggggactgcgttaacggttactaaggaaaactggaaatactgtctggtttttgtaaatgttatctatttttgtagatattttatataaaaatgaaatattttaacattttatgggtcagtcaactttcagaaattcagggagctggagagggaaatctttttttttccccctgagtggttcttatgtatacatagaagtatctgagacataaactgtacagaaaacttgtccacgtgcttttgtatgcccatgtattcatgtttgtttgtagatgtttgtctgatgcatttcattaaaaaaaaaaccatgaattacgaagcaccttagtaagcaccttctaatgctgcattttttttgttgttgttaaaaacataccagctggttataatattgttctccacgtccttgtgatgattctgagcctggcactcccaaatctgggaagcatagtttatttgcaagtgttcaccttccaaatcatgaggcatagcatgacttattcttgtttggaaaactcttttcaaaactgaccatcttaaacacatgatggccaagtgcccaaaagccctcttgcggagcaaatttcagaatatatatgtggatccaagctctgatagttcaggtgctggagggaagagagacctgtgtgtttagaggccaggaccacagttaggattgggttgtttcaatactgagagacagctacaataaaaggagagcaattgcctccctggggctgttcaatcttctgcatttgtgagtggttcagtcatgaggttttccaaaagatgtttttagagttgtaaaaaccatatttgcagcaaagatttacaaaggcgtatcagactatgattgttcaccaaaataggggaatggtttgatccgccagttgcaagtagaggcctttctgactcttaatattcactttggtgctactacccccattacctgagggaaactggccaggtccttgatcatggaactatagagctaccaggacatatcctgctctctaagggaatttattgctatcttgcaccttctttaaaactcacatatgcagacctgacactcaagagtggctagctacacagagtccatctaatttttgcaacttcctgtggccagtgtgtataaccccttccactatctcacagatagtcacagcgtccattccatagtctgtctcctcacatctgttagtattgacacagcacagacaccacaagccatcaggttcttcatggggcaggtgaaatacttctaccccatgggtaaatgtattcacatattaccaagagaagaagcacattatctatgatcttttggcccagttcttatttagcatttttattccagcctacttggaaacatgtttttatttgcaatatatgcctgactgaattaagcttgcttgttttaaacaaccaaatcattggaacagaaaaggatttaaaaaacaagaatgcatgatctcagagtgattaaaaaaaaatcagtggaaataaatgatcatagaaggtgcttttcaaaacaactgctattataattctcaaagtcctactctgccaaaagaagattaaaagtcatacattacattacaaggaaatgttcatgtgggaagagggttgctgaaaatcaacaacgcttgaagttaaaaagtgtgtctttgtagatttcattgtataatgtgtatttcttaggagatggctgacttgattgatctacgctaagtggagacatttcacatttttaaaaccaaatgttcaatctgtattactctttgccgtcttgtatgtagaggctatttttaaatcattaaatttttagatctctgttttcataaaaaaaaaaaaaaa

SEQ ID NO: 6 - DNA, 1329 bp, Homo sapiens
acaacagtgagctcagagacttgagggaggcgctgcgactgacaagcggctctgcccgggaccttctcgctttcatctagcgctgcactcaatggaggggcgggcaccgcagtgcttaatgctgtcttaactagtgtaggaaaacggctcaacccaccgctgccgaaatgaagtataagaatcttatggcaagggccttatatgacaatgtcccagagtgtgccgaggaactggcctttcgcaagggagacatcctgaccgtcatagagcagaacacagggggactggaaggatggtggctgtgctcattacacggtcggcaaggcattgtcccaggcaaccgggtgaagcttctgattggtcccatgcaggagactgcctccagtcacgagcagcctgcctctggactgatgcagcagacctttggccaacagaagctctatcaagtgccaaacccacaggctgctccccgagacaccatctaccaagtgccaccttcctaccaaaatcagggaatttaccaagtccccactggccacggcacccaagaacaagaggtatatcaggtgccaccatcagtgcagagaagcattgggggaaccagtgggccccacgtgggtaaaaaggtgttccagagagatgggcaagtgtcctatttcttagtgagagcctctaaacaaaccagcttgtgaacctccactgaaaagatctcatctgatgagcattttaataaagtgtcctgagtttggaggcttgccgtctttctcttggataaatatcttcatctcctagacttggaaaaacacattttctcctggggtttcccattggcgtgtcttgagctgctctggtgataaccgtaataatgccaatactgatacgaacagcagaaaacagtaaccccaagaactctacagatgatcatcaaggaccactgtctcttaccatttgctgctttggtttgaaattctcactgcctcgtagatctcattttgagcactatacattcctaaagattgatttctttctatctgacttaaatttaggaatgattaaatcttcatttctcccatgatttgatcctaaaacattttgaaaggaaacagccttgagatctgtgattactaagacatacataacattcttatcacattagaaagcaagaattgactgttgcttgtcttgttcctgttgtcttgtcccctgaattcctgtttatctttgattgtatgtgggacattgtattttcagtacatttgtagaaataatgtgaagcctataaagatgttctctgcctccaaaaaaaaaaaaaaaaaaaaaaaaaaaaaa

SEQ ID NO: 7 - DNA, 4745 bp, Homo sapiens
acacatacatatgccactcacatccgacgtgtgtggttgctcagtagggaaatgcttacagctgcctctagaagcaagtccgctcgctgcatggagagggaaacatgagcatgcagcaggactagctgtcacctcccgcccgcctgcccagagagggccagagcgtcggggaggcaagatgatccaccagcggttccatcctacacttggattcagtaagctgtgaggtccgtaatgtcagacactggcaaacatcatatgttcttcaagtagagttatgaaaacgaagaaactggtcagaagagtaaaacgccggaattgtcctttccaacatccagagctgcatcattccttggggcaaaatgtggacaaggaatcttatggcaagggccttatatgacaatgtcccagagtgtgccgaggaactggcctttcgcaagggagacatcctgaccgtcatagagcagaacacagggggactggaaggatggtggctgtgctcattacacggtcggcaaggcattgtcccaggcaaccgggtgaagcttctgattggtcccatgcaggagactgcctccagtcacgagcagcctgcctctggactgatgcagcagacctttggccaacagaagctctatcaagtgccaaacccacaggctgctccccgagacaccatctaccaagtgccaccttcctaccaaaatcagggaatttaccaagtccccactggccacggcacccaagaacaagaggtatatcaggtgccaccatcagtgcagagaagcattgggggaaccagtgggccccacgtgggtaaaaaggtgataacccccgtgaggacaggccatggctacgtatacgagtacccatccagataccaaaaggacgtctatgatatccctccttctcataccactcaaggggtatacgacatccctccctcatcagcaaaaggccctgtgttttcagttccagtgggagagataaaacctcaaggggtgtatgacatcccgcctacaaaaggggtatatgccattccgccctctgcttgccgggatgaagcagggcttagggaaaaagactatgacttcccccctcccatgagacaagctggaaggccggacctcagaccggagggggtttatgacattcctccaacctgcaccaagccagcagggaaggaccttcatgtaaaatacaactgtgacattccaggagctgcagaaccggtggctcgaaggcaccagagcctgtccccgaatcacccacccccgcaactcggacagtcagtgggctctcagaacgacgcatatgatgtcccccgaggcgttcagtttcttgagccaccagcagaaaccagtgagaaagcaaacccccaggaaagggatggtgtttatgatgtccctctgcataacccgccagatgctaaaggctctcgggacttggtggatgggatcaaccgattgtctttctccagtacaggcagcacccggagtaacatgtccacgtcttccacctcctccaaggagtcctcactgtcagcctccccagctcaggacaaaaggctcttcctggatccagacacagctattgagagacttcagcggctccagcaggcccttgagatgggtgtctccagcctaatggcactggtcactaccgactggcggtgttacggatatatggaaagacacatcaatgaaatacgcacagcagtggacaaggtggagctgttcctgaaggagtacctccactttgtcaagggagctgttgcaaatgctgcctgcctcccggaactcatcctccacaacaagatgaagcgggagctgcaacgagttgaagactcccaccagatcctgagtcaaaccagccatgacttaaatgagtgcagctggtccctgaatatcttggccatcaacaagccccagaacaagtgtgacgatctggaccggtttgtgatggtggcaaagacggtgcccgatgacgccaagcagctcaccacaaccatcaacaccaacgcagaggccctcttcagacccggccctggcagcttgcatctgaagaatgggccggagagcatcatgaactcaacggagtacccacacggtggctcccagggacagctgctgcatcctggtgaccacaaggcccaggcccacaacaaggcactgcccccaggcctgagcaaggagcaggcccctgactgtagcagcagtgatggttctgagaggagctggatggatgactacgattacgtccacctacagggtaaggaggagtttgagaggcaacagaaagagctattggaaaaagagaatatcatgaaacagaacaagatgcagctggaacatcatcagctgagccagttccagctgttggaacaagagattacaaagcccgtggagaatgacatctcgaagtggaagccctctcagagcctacccaccacaaacagtggcgtgagtgctcaggatcggcagttgctgtgcttctactatgaccaatgtgagacccatttcatttcccttctcaacgccattgacgcactcttcagttgtgtcagctcagcccagcccccgcgaatcttcgtggcacacagcaagtttgtcatcctcagtgcacacaaactggtgttcattggagacacgctgacacggcaggtgactgcccaggacattcgcaacaaagtcatgaactccagcaaccagctctgcgagcagctcaagaccatagtcatggcaaccaagatggccgccctccattaccccagcaccacggccctgcaggaaatggtgcaccaagtgacagacctttctagaaatgcccagctgttcaagcgctctttgctggagatggcaacgttctgagaagaaaaaaaagaggaaggggactgcgttaacggttactaaggaaaactggaaatactgtctggtttttgtaaatgttatctatttttgtagatattttatataaaaatgaaatattttaacattttatgggtcagtcaactttcagaaattcagggagctggagagggaaatctttttttttccccctgagtggttcttatgtatacatagaagtatctgagacataaactgtacagaaaacttgtccacgtgcttttgtatgcccatgtattcatgtttgtttgtagatgtttgtctgatgcatttcattaaaaaaaaaaccatgaattacgaagcaccttagtaagcaccttctaatgctgcattttttttgttgttgttaaaaacataccagctggttataatattgttctccacgtccttgtgatgattctgagcctggcactcccaaatctgggaagcatagtttatttgcaagtgttcaccttccaaatcatgaggcatagcatgacttattcttgtttggaaaactcttttcaaaactgaccatcttaaacacatgatggccaagtgcccaaaagccctcttgcggagcaaatttcagaatatatatgtggatccaagctctgatagttcaggtgctggagggaagagagacctgtgtgtttagaggccaggaccacagttaggattgggttgtttcaatactgagagacagctacaataaaaggagagcaattgcctccctggggctgttcaatcttctgcatttgtgagtggttcagtcatgaggttttccaaaagatgtttttagagttgtaaaaaccatatttgcagcaaagatttacaaaggcgtatcagactatgattgttcaccaaaataggggaatggtttgatccgccagttgcaagtagaggcctttctgactcttaatattcactttggtgctactacccccattacctgagggaaactggccaggtccttgatcatggaactatagagctaccaggacatatcctgctctctaagggaatttattgctatcttgcaccttctttaaaactcacatatgcagacctgacactcaagagtggctagctacacagagtccatctaatttttgcaacttcctgtggccagtgtgtataaccccttccactatctcacagatagtcacagcgtccattccatagtctgtctcctcacatctgttagtattgacacagcacagacaccacaagccatcaggttcttcatggggcaggtgaaatacttctaccccatgggtaaatgtattcacatattaccaagagaagaagcacattatctatgatcttttggcccagttcttatttagcatttttattccagcctacttggaaacatgtttttatttgcaatatatgcctgactgaattaagcttgcttgttttaaacaaccaaatcattggaacagaaaaggatttaaaaaacaagaatgcatgatctcagagtgattaaaaaaaaatcagtggaaataaatgatcatagaaggtgcttttcaaaacaactgctattataattctcaaagtcctactctgccaaaagaagattaaaagtcatacattacattacaaggaaatgttcatgtgggaagagggttgctgaaaatcaacaacgcttgaagttaaaaagtgtgtctttgtagatttcattgtataatgtgtatttcttaggagatggctgacttgattgatctacgctaagtggagacatttcacatttttaaaaccaaatgttcaatctgtattactctttgccgtcttgtatgtagaggctatttttaaatcattaaatttttagatctctgttttcataaaaaaaaaaaaaaa

SEQ ID NO: 8 - DNA, 4103 bp, Homo sapiens
acaacagtgagctcagagacttgagggaggcgctgcgactgacaagcggctctgcccgggaccttctcgctttcatctagcgctgcactcaatggaggggcgggcaccgcagtgcttaatgctgtcttaactagtgtaggaaaacggctcaacccaccgctgccgaaatgaagtataaggtgataacccccgtgaggacaggccatggctacgtatacgagtacccatccagataccaaaaggacgtctatgatatccctccttctcataccactcaaggggtatacgacatccctccctcatcagcaaaaggccctgtgttttcagttccagtgggagagataaaacctcaaggggtgtatgacatcccgcctacaaaaggggtatatgccattccgccctctgcttgccgggatgaagcagggcttagggaaaaagactatgacttcccccctcccatgagacaagctggaaggccggacctcagaccggagggggtttatgacattcctccaacctgcaccaagccagcagggaaggaccttcatgtaaaatacaactgtgacattccaggagctgcagaaccggtggctcgaaggcaccagagcctgtccccgaatcacccacccccgcaactcggacagtcagtgggctctcagaacgacgcatatgatgtcccccgaggcgttcagtttcttgagccaccagcagaaaccagtgagaaagcaaacccccaggaaagggatggtgtttatgatgtccctctgcataacccgccagatgctaaaggctctcgggacttggtggatgggatcaaccgattgtctttctccagtacaggcagcacccggagtaacatgtccacgtcttccacctcctccaaggagtcctcactgtcagcctccccagctcaggacaaaaggctcttcctggatccagacacagctattgagagacttcagcggctccagcaggcccttgagatgggtgtctccagcctaatggcactggtcactaccgactggcggtgttacggatatatggaaagacacatcaatgaaatacgcacagcagtggacaaggtggagctgttcctgaaggagtacctccactttgtcaagggagctgttgcaaatgctgcctgcctcccggaactcatcctccacaacaagatgaagcgggagctgcaacgagttgaagactcccaccagatcctgagtcaaaccagccatgacttaaatgagtgcagctggtccctgaatatcttggccatcaacaagccccagaacaagtgtgacgatctggaccggtttgtgatggtggcaaagacggtgcccgatgacgccaagcagctcaccacaaccatcaacaccaacgcagaggccctcttcagacccggccctggcagcttgcatctgaagaatgggccggagagcatcatgaactcaacggagtacccacacggtggctcccagggacagctgctgcatcctggtgaccacaaggcccaggcccacaacaaggcactgcccccaggcctgagcaaggagcaggcccctgactgtagcagcagtgatggttctgagaggagctggatggatgactacgattacgtccacctacagggtaaggaggagtttgagaggcaacagaaagagctattggaaaaagagaatatcatgaaacagaacaagatgcagctggaacatcatcagctgagccagttccagctgttggaacaagagattacaaagcccgtggagaatgacatctcgaagtggaagccctctcagagcctacccaccacaaacagtggcgtgagtgctcaggatcggcagttgctgtgcttctactatgaccaatgtgagacccatttcatttcccttctcaacgccattgacgcactcttcagttgtgtcagctcagcccagcccccgcgaatcttcgtggcacacagcaagtttgtcatcctcagtgcacacaaactggtgttcattggagacacgctgacacggcaggtgactgcccaggacattcgcaacaaagtcatgaactccagcaaccagctctgcgagcagctcaagaccatagtcatggcaaccaagatggccgccctccattaccccagcaccacggccctgcaggaaatggtgcaccaagtgacagacctttctagaaatgcccagctgttcaagcgctctttgctggagatggcaacgttctgagaagaaaaaaaagaggaaggggactgcgttaacggttactaaggaaaactggaaatactgtctggtttttgtaaatgttatctatttttgtagatattttatataaaaatgaaatattttaacattttatgggtcagtcaactttcagaaattcagggagctggagagggaaatctttttttttccccctgagtggttcttatgtatacatagaagtatctgagacataaactgtacagaaaacttgtccacgtgcttttgtatgcccatgtattcatgtttgtttgtagatgtttgtctgatgcatttcattaaaaaaaaaaccatgaattacgaagcaccttagtaagcaccttctaatgctgcattttttttgttgttgttaaaaacataccagctggttataatattgttctccacgtccttgtgatgattctgagcctggcactcccaaatctgggaagcatagtttatttgcaagtgttcaccttccaaatcatgaggcatagcatgacttattcttgtttggaaaactcttttcaaaactgaccatcttaaacacatgatggccaagtgcccaaaagccctcttgcggagcaaatttcagaatatatatgtggatccaagctctgatagttcaggtgctggagggaagagagacctgtgtgtttagaggccaggaccacagttaggattgggttgtttcaatactgagagacagctacaataaaaggagagcaattgcctccctggggctgttcaatcttctgcatttgtgagtggttcagtcatgaggttttccaaaagatgtttttagagttgtaaaaaccatatttgcagcaaagatttacaaaggcgtatcagactatgattgttcaccaaaataggggaatggtttgatccgccagttgcaagtagaggcctttctgactcttaatattcactttggtgctactacccccattacctgagggaaactggccaggtccttgatcatggaactatagagctaccaggacatatcctgctctctaagggaatttattgctatcttgcaccttctttaaaactcacatatgcagacctgacactcaagagtggctagctacacagagtccatctaatttttgcaacttcctgtggccagtgtgtataaccccttccactatctcacagatagtcacagcgtccattccatagtctgtctcctcacatctgttagtattgacacagcacagacaccacaagccatcaggttcttcatggggcaggtgaaatacttctaccccatgggtaaatgtattcacatattaccaagagaagaagcacattatctatgatcttttggcccagttcttatttagcatttttattccagcctacttggaaacatgtttttatttgcaatatatgcctgactgaattaagcttgcttgttttaaacaaccaaatcattggaacagaaaaggatttaaaaaacaagaatgcatgatctcagagtgattaaaaaaaaatcagtggaaataaatgatcatagaaggtgcttttcaaaacaactgctattataattctcaaagtcctactctgccaaaagaagattaaaagtcatacattacattacaaggaaatgttcatgtgggaagagggttgctgaaaatcaacaacgcttgaagttaaaaagtgtgtctttgtagatttcattgtataatgtgtatttcttaggagatggctgacttgattgatctacgctaagtggagacatttcacatttttaaaaccaaatgttcaatctgtattactctttgccgtcttgtatgtagaggctatttttaaatcattaaatttttagatctctgttttcataaaaaaaaaaaaaaa

SEQ ID NO: 9 - protein, 834 aa, Homo sapiens
MKYKNLMARALYDNVPECAEELAFRKGDILTVIEQNTGGLEGWWLCSLHGRQGIVPGNRVKLLIGPMQETASSHEQPASGLMQQTFGQQKLYQVPNPQAAPRDTIYQVPPSYQNQGIYQVPTGHGTQEQEVYQVPPSVQRSIGGTSGPHVGKKVITPVRTGHGYVYEYPSRYQKDVYDIPPSHTTQGVYDIPPSSAKGPVFSVPVGEIKPQGVYDIPPTKGVYAIPPSACRDEAGLREKDYDFPPPMRQAGRPDLRPEGVYDIPPTCTKPAGKDLHVKYNCDIPGAAEPVARRHQSLSPNHPPPQLGQSVGSQNDAYDVPRGVQFLEPPAETSEKANPQERDGVYDVPLHNPPDAKGSRDLVDGINRLSFSSTGSTRSNMSTSSTSSKESSLSASPAQDKRLFLDPDTAIERLQRLQQALEMGVSSLMALVTTDWRCYGYMERHINEIRTAVDKVELFLKEYLHFVKGAVANAACLPELILHNKMKRELQRVEDSHQILSQTSHDLNECSWSLNILAINKPQNKCDDLDRFVMVAKTVPDDAKQLTTTINTNAEALFRPGPGSLHLKNGPESIMNSTEYPHGGSQGQLLHPGDHKAQAHNKALPPGLSKEQAPDCSSSDGSERSWMDDYDYVHLQGKEEFERQQKELLEKENIMKQNKMQLEHHQLSQFQLLEQEITKPVENDISKWKPSQSLPTTNSGVSAQDRQLLCFYYDQCETHFISLLNAIDALFSCVSSAQPPRIFVAHSKFVILSAHKLVFIGDTLTRQVTAQDIRNKVMNSSNQLCEQLKTIVMATKMAALHYPSTTALQEMVHQVTDLSRNAQLFKRSLLEMATF

SEQ ID NO: 10 - protein, 174 aa, Homo sapiens
MKYKNLMARALYDNVPECAEELAFRKGDILTVIEQNTGGLEGWWLCSLHGRQGIVPGNRVKLLIGPMQETASSHEQPASGLMQQTFGQQKLYQVPNPQAAPRDTIYQVPPSYQNQGIYQVPTGHGTQEQEVYQVPPSVQRSIGGTSGPHVGKKVFQRDGQVSYFLVRASKQTSL

SEQ ID NO: 11 - protein, 834 aa, Homo sapiens
MWTRNLMARALYDNVPECAEELAFRKGDILTVIEQNTGGLEGWWLCSLHGRQGIVPGNRVKLLIGPMQETASSHEQPASGLMQQTFGQQKLYQVPNPQAAPRDTIYQVPPSYQNQGIYQVPTGHGTQEQEVYQVPPSVQRSIGGTSGPHVGKKVITPVRTGHGYVYEYPSRYQKDVYDIPPSHTTQGVYDIPPSSAKGPVFSVPVGEIKPQGVYDIPPTKGVYAIPPSACRDEAGLREKDYDFPPPMRQAGRPDLRPEGVYDIPPTCTKPAGKDLHVKYNCDIPGAAEPVARRHQSLSPNHPPPQLGQSVGSQNDAYDVPRGVQFLEPPAETSEKANPQERDGVYDVPLHNPPDAKGSRDLVDGINRLSFSSTGSTRSNMSTSSTSSKESSLSASPAQDKRLFLDPDTAIERLQRLQQALEMGVSSLMALVTTDWRCYGYMERHINEIRTAVDKVELFLKEYLHFVKGAVANAACLPELILHNKMKRELQRVEDSHQILSQTSHDLNECSWSLNILAINKPQNKCDDLDRFVMVAKTVPDDAKQLTTTINTNAEALFRPGPGSLHLKNGPESIMNSTEYPHGGSQGQLLHPGDHKAQAHNKALPPGLSKEQAPDCSSSDGSERSWMDDYDYVHLQGKEEFERQQKELLEKENIMKQNKMQLEHHQLSQFQLLEQEITKPVENDISKWKPSQSLPTTNSGVSAQDRQLLCFYYDQCETHFISLLNAIDALFSCVSSAQPPRIFVAHSKFVILSAHKLVFIGDTLTRQVTAQDIRNKVMNSSNQLCEQLKTIVMATKMAALHYPSTTALQEMVHQVTDLSRNAQLFKRSLLEMATF

SEQ ID NO: 12 - protein, 685 aa, Homo sapiens
MKYKVITPVRTGHGYVYEYPSRYQKDVYDIPPSHTTQGVYDIPPSSAKGPVFSVPVGEIKPQGVYDIPPTKGVYAIPPSACRDEAGLREKDYDFPPPMRQAGRPDLRPEGVYDIPPTCTKPAGKDLHVKYNCDIPGAAEPVARRHQSLSPNHPPPQLGQSVGSQNDAYDVPRGVQFLEPPAETSEKANPQERDGVYDVPLHNPPDAKGSRDLVDGINRLSFSSTGSTRSNMSTSSTSSKESSLSASPAQDKRLFLDPDTAIERLQRLQQALEMGVSSLMALVTTDWRCYGYMERHINEIRTAVDKVELFLKEYLHFVKGAVANAACLPELILHNKMKRELQRVEDSHQILSQTSHDLNECSWSLNILAINKPQNKCDDLDRFVMVAKTVPDDAKQLTTTINTNAEALFRPGPGSLHLKNGPESIMNSTEYPHGGSQGQLLHPGDHKAQAHNKALPPGLSKEQAPDCSSSDGSERSWMDDYDYVHLQGKEEFERQQKELLEKENIMKQNKMQLEHHQLSQFQLLEQEITKPVENDISKWKPSQSLPTTNSGVSAQDRQLLCFYYDQCETHFISLLNAIDALFSCVSSAQPPRIFVAHSKFVILSAHKLVFIGDTLTRQVTAQDIRNKVMNSSNQLCEQLKTIVMATKMAALHYPSTTALQEMVHQVTDLSRNAQLFKRSLLEMATF

SEQ ID NO: 13 - DNA, 1001 bp, Homo sapiens
tatctccttggatcagccctgctgtcatctcttcacaactccctgtccttgttgctgcccattttggggaatttatttatcaactcctgctgtaaacgataataataacaatgataacacatattgaatattttgtgcctaacactgtacactttctcatgtaatcctccaataaccacgtgagataggtgctattattatttccattgacaggtgaaataacagatgttcagagagttaagtaatctatccaaagtcagacagctagtacctgacaacgcatatcagagcaagaaattctagctctcataacaggcaaactcccaaatcacagtatcttaacacaaaaagagtttatttcatgatcacatcttggcccctgggaattggtgactccttctagtcaggccatcatgaaacatatgacacccatggcttctgcatggggtaatgaaagaggcattgcaaactttaagggcctcagcccttcctgtcacagttcaatgacaagaatgagtattgtgacccctatctacttacaagggaggataggacacataggggaagacatatctatttagtgagcactaactgtactgctttaccctagcacccatgctcttatctagcttaactgtccttagttatctatctatctatctatctatctatctatctatctatctatctatcatctatctgcctacagttaactatcttaactgtccttaccaaggccccagttgcacattccctgatgccaccagggctctgctgacctttattacaactcctctacagattcaacagtctgcctttgctctgctttcctgctcatctgctttcctgctcatctgctttgctctttttactctttctccctcccatctccctttcctctgcttctcactgtctttcttctgcataaccctactctgtgtgttgagtcttctatcacatctttctcctgtacgtgccttctctgatcttctttcagttgc

SEQ ID NO: 14 - DNA, 1001 bp, Homo sapiens
tatctccttggatcagccctgctgtcatctcttcacaactccctgtccttgttgctgcccattttggggaatttatttatcaactcctgctgtaaacgataataataacaatgataacacatattgaatattttgtgcctaacactgtacactttctcatgtaatcctccaataaccacgtgagataggtgctattattatttccattgacaggtgaaataacagatgttcagagagttaagtaatctatccaaagtcagacagctagtacctgacaacgcatatcagagcaagaaattctagctctcataacaggcaaactcccaaatcacagtatcttaacacaaaaagagtttatttcatgatcacatcttggcccctgggaattggtgactccttctagtcaggccatcatgaaacatatgacacccatggcttctgcatggggtaatgaaagaggcattgcaaactttaagggcctcagcccttcctgtcacagtccaatgacaagaatgagtattgtgacccctatctacttacaagggaggataggacacataggggaagacatatctatttagtgagcactaactgtactgctttaccctagcacccatgctcttatctagcttaactgtccttagttatctatctatctatctatctatctatctatctatctatctatctatcatctatctgcctacagttaactatcttaactgtccttaccaaggccccagttgcacattccctgatgccaccagggctctgctgacctttattacaactcctctacagattcaacagtctgcctttgctctgctttcctgctcatctgctttcctgctcatctgctttgctctttttactctttctccctcccatctccctttcctctgcttctcactgtctttcttctgcataaccctactctgtgtgttgagtcttctatcacatctttctcctgtacgtgccttctctgatcttctttcagttgc

SEQ ID NO: 15 - DNA, 8718 bp, Homo sapiens
cctcccctcgcccggcgcggtcccgtccgcctctcgctcgcctcccgcctcccctcggtcttccgaggcgcccgggctcccggcgcggcggcggagggggcgggcaggccggcgggcggtgatgtggcgggactctttatgcgctgcggcaggatacgcgctcggcgctgggacgcgactgcgctcagttctctcctctcggaagctgcagccatgatggaagtttgagagttgagccgctgtgaggcgaggccgggctcaggcgagggagatgagagacggcggcggccgcggcccggagcccctctcagcgcctgtgagcagccgcgggggcagcgccctcggggagccggccggcctgcggcggcggcagcggcggcgtttctcgcctcctcttcgtcttttctaaccgtgcagcctcttcctcggcttctcctgaaagggaaggtggaagccgtgggctcgggcgggagccggctgaggcgcggcggcggcggcggcacctcccgctcctggagcgggggggagaagcggcggcggcggcggccgcggcggctgcagctccagggagggggtctgagtcgcctgtcaccatttccagggctgggaacgccggagagttggtctctccccttctactgcctccaacacggcggcggcggcggcggcacatccagggacccgggccggttttaaacctcccgtccgccgccgccgcaccccccgtggcccgggctccggaggccgccggcggaggcagccgttcggaggattattcgtcttctccccattccgctgccgccgctgccaggcctctggctgctgaggagaagcaggcccagtcgctgcaaccatccagcagccgccgcagcagccattacccggctgcggtccagagccaagcggcggcagagcgaggggcatcagctaccgccaagtccagagccatttccatcctgcagaagaagccccgccaccagcagcttctgccatctctctcctcctttttcttcagccacaggctcccagacatgacagccatcatcaaagagatcgttagcagaaacaaaaggagatatcaagaggatggattcgacttagacttgacctatatttatccaaacattattgctatgggatttcctgcagaaagacttgaaggcgtatacaggaacaatattgatgatgtagtaaggtttttggattcaaagcataaaaaccattacaagatatacaatctttgtgctgaaagacattatgacaccgccaaatttaattgcagagttgcacaatatccttttgaagaccataacccaccacagctagaacttatcaaacccttttgtgaagatcttgaccaatggctaagtgaagatgacaatcatgttgcagcaattcactgtaaagctggaaagggacgaactggtgtaatgatatgtgcatatttattacatcggggcaaatttttaaaggcacaagaggccctagatttctatggggaagtaaggaccagagacaaaaagggagtaactattcccagtcagaggcgctatgtgtattattatagctacctgttaaagaatcatctggattatagaccagtggcactgttgtttcacaagatgatgtttgaaactattccaatgttcagtggcggaacttgcaatcctcagtttgtggtctgccagctaaaggtgaagatatattcctccaattcaggacccacacgacgggaagacaagttcatgtactttgagttccctcagccgttacctgtgtgtggtgatatcaaagtagagttcttccacaaacagaacaagatgctaaaaaaggacaaaatgtttcacttttgggtaaatacattcttcataccaggaccagaggaaacctcagaaaaagtagaaaatggaagtctatgtgatcaagaaatcgatagcatttgcagtatagagcgtgcagataatgacaaggaatatctagtacttactttaacaaaaaatgatcttgacaaagcaaataaagacaaagccaaccgatacttttctccaaattttaaggtgaagctgtacttcacaaaaacagtagaggagccgtcaaatccagaggctagcagttcaacttctgtaacaccagatgttagtgacaatgaacctgatcattatagatattctgacaccactgactctgatccagagaatgaaccttttgatgaagatcagcatacacaaattacaaaagtctgaatttttttttatcaagagggataaaacaccatgaaaataaacttgaataaactgaaaatggacctttttttttttaatggcaataggacattgtgtcagattaccagttataggaacaattctcttttcctgaccaatcttgttttaccctatacatccacagggttttgacacttgttgtccagttgaaaaaaggttgtgtagctgtgtcatgtatatacctttttgtgtcaaaaggacatttaaaattcaattaggattaataaagatggcactttcccgttttattccagttttataaaaagtggagacagactgatgtgtatacgtaggaattttttccttttgtgttctgtcaccaactgaagtggctaaagagctttgtgatatactggttcacatcctacccctttgcacttgtggcaacagataagtttgcagttggctaagagaggtttccgaagggttttgctacattctaatgcatgtattcgggttaggggaatggagggaatgctcagaaaggaaataattttatgctggactctggaccatataccatctccagctatttacacacacctttctttagcatgctacagttattaatctggacattcgaggaattggccgctgtcactgcttgttgtttgcgcatttttttttaaagcatattggtgctagaaaaggcagctaaaggaagtgaatctgtattggggtacaggaatgaaccttctgcaacatcttaagatccacaaatgaagggatataaaaataatgtcataggtaagaaacacagcaacaatgacttaaccatataaatgtggaggctatcaacaaagaatgggcttgaaacattataaaaattgacaatgatttattaaatatgttttctcaattgtaacgacttctccatctcctgtgtaatcaaggccagtgctaaaattcagatgctgttagtacctacatcagtcaacaacttacacttattttactagttttcaatcataatacctgctgtggatgcttcatgtgctgcctgcaagcttcttttttctcattaaatataaaatattttgtaatgctgcacagaaattttcaatttgagattctacagtaagcgttttttttctttgaagatttatgatgcacttattcaatagctgtcagccgttccacccttttgaccttacacattctattacaatgaattttgcagttttgcacattttttaaatgtcattaactgttagggaattttacttgaatactgaatacatataatgtttatattaaaaaggacatttgtgttaaaaaggaaattagagttgcagtaaactttcaatgctgcacacaaaaaaaagacatttgatttttcagtagaaattgtcctacatgtgctttattgatttgctattgaaagaatagggtttttttttttttttttttttttttttttaaatgtgcagtgttgaatcatttcttcatagtgctcccccgagttgggactagggcttcaatttcacttcttaaaaaaaatcatcatatatttgatatgcccagactgcatacgattttaagcggagtacaactactattgtaaagctaatgtgaagatattattaaaaaggtttttttttccagaaatttggtgtcttcaaattataccttcaccttgacatttgaatatccagccattttgtttcttaatggtataaaattccattttcaataacttattggtgctgaaattgttcactagctgtggtctgacctagttaatttacaaatacagattgaataggacctactagagcagcatttatagagtttgatggcaaatagattaggcagaacttcatctaaaatattcttagtaaataatgttgacacgttttccataccttgtcagtttcattcaacaatttttaaatttttaacaaagctcttaggatttacacatttatatttaaacattgatatatagagtattgattgattgctcataagttaaattggtaaagttagagacaactattctaacacctcaccattgaaatttatatgccaccttgtctttcataaaagctgaaaattgttacctaaaatgaaaatcaacttcatgttttgaagatagttataaatattgttctttgttacaatttcgggcaccgcatattaaaacgtaactttattgttccaatatgtaacatggagggccaggtcataaataatgacattataatgggcttttgcactgttattatttttcctttggaatgtgaaggtctgaatgagggttttgattttgaatgtttcaatgtttttgagaagccttgcttacattttatggtgtagtcattggaaatggaaaaatggcattatatatattatatatataaatatatattatacatactctccttactttatttcagttaccatccccatagaatttgacaagaattgctatgactgaaaggttttcgagtcctaattaaaactttatttatggcagtattcataattagcctgaaatgcattctgtaggtaatctctgagtttctggaatattttcttagactttttggatgtgcagcagcttacatgtctgaagttacttgaaggcatcacttttaagaaagcttacagttgggccctgtaccatcccaagtcctttgtagctcctcttgaacatgtttgccatacttttaaaagggtagttgaataaatagcatcaccattctttgctgtggcacaggttataaacttaagtggagtttaccggcagcatcaaatgtttcagctttaaaaaataaaagtagggtacaagtttaatgtttagttctagaaattttgtgcaatatgttcataacgatggctgtggttgccacaaagtgcctcgtttacctttaaatactgttaatgtgtcatgcatgcagatggaaggggtggaactgtgcactaaagtgggggctttaactgtagtatttggcagagttgccttctacctgccagttcaaaagttcaacctgttttcatatagaatatatatactaaaaaatttcagtctgttaaacagccttactctgattcagcctcttcagatactcttgtgctgtgcagcagtggctctgtgtgtaaatgctatgcactgaggatacacaaaaataccaatatgatgtgtacaggataatgcctcatcccaatcagatgtccatttgttattgtgtttgttaacaaccctttatctcttagtgttataaactccacttaaaactgattaaagtctcattcttgtcattgtgtgggtgttttattaaatgagagtttataattcaaattgcttaagtccattgaagttttaattaatgggcagccaaatgtgaatacaaagttttcagtttttttttttcctgctgtccttcaaagcctactgtttaaaaaaaaaaaaaaaaaaaaacatggcctgagagtagagtatctgtctactcatgtttaattaaggaaaaacacttatttttagggctttagtcatcacttcataaattgtataagcacattaaatagcgttctagtcctgaaaaagtccaagattcttagaaaattgtgcatatttttattatgacagatgtttgaagataattccccagaatggatttgatactttagatttcaattttgtggcttttgtctattattctgtactctgccatcagcatatggaaagcttcatttactcatcatgacttgtgccatataaaaattgatatttcggaatagtctaaaggactttttgtacttgaatttaatcatgttgtttctaatattcttaaaagcttgaagactaaagcatatcctttcaacaaagcatagtaaggtaataagaaagtgtagtttgtacaagtgttaaaaaaataaagtagacaatgttacagtgggacttattatttcaagtttacattttctccatgtaattttttaaaaagtaaatgaaaaaatgtgcaataatgtaaaatatgaagtgtatgtgtacacacattttatttttcggtatcttgggtatacgtatggttgaaaactatactggagtctaaaagtattctaatttataagaagacattttggtgatgtttgaaaaatagaaatgtgctagttttgtttttatatcatgtcctttgtacgttgtaatatgagctggcttggttcagtaaatgccatcaccatttccattgagaatttaaaactcaccagtgtttaatatgcaggcttccaaaggcttatgaaaaaaatcaagacccttaaatctagttaatttgctgctaacatgaaactctttggttcttttatttttgccagataattagacacacatctaaagcttagtcttaaatggcttaagtgtagctattgattagtgctgttgctagttcagaaagaaatgtttgtgaatggaaacaagaatattcagtccaaactgttgtaaggacagtacctgaaaaccaggaaacaggataatggaaaaagtcttttaaagatgaaatgttggagccaactttcttatagaattaattgtatgtggctatagaaagcctaatgattgttgcttatttttgagagcatattattcttttatgaccataatcttgctgtttttccatcttccaaaagatcttccttctaatatgtatatcagaatgtgggtagccagtcagacaaattcatattggttggtagctttaaaaagtttgtaatgtgaagacaggaaaggacaaaatagtttgctttggtggtagtactctggttgttaagctaggtattttgagactacttccccatcacaacaacaataaaataatcactcataatcctatcacctggagacatagccatcgttaatatgttagtgactatacaatcatgttttcttctgtatatccatgtatattctttaaaaatgaaatttatactgtacctgatctcaaagctttttagcttagtatatctgtcatgaatttgtaggatgttccattgcatcagaaaacggacagtgatttgattactttctaatgccacagatgcagattacatgtagttattgagaatcctttcgaattcagtggcttaatcatgaatgtctaaatattgttgacattaggatgatacatgtaaattaaagttacatttgtttagcatagacaagcttaacattgtagatgtttctcttcaaaaatcatcttaaacatttgcatttggaattgtgttaaatagaatgtgtgaaacactgtattagtaaacttcatcacctttctacttccttatagtttgaacttttcagtttttgtagttcccaaacagttgctcaatttagagcaaattaatttaacacctgccaaaaaaaggctgctgttggcttatcagttgtctttaaattcaaatgctcatgtgacttttatcacatcaaaaaatatttcattaatgattcacctttagctctgaaaattaccgcgtttagtaattatagtgggcttataaaaacatgcaactctttttgatagttatttgagaattttggtgaaaaatatttagctgagggcagtatagaacttataaaccaatatattgatatttttaaaacatttttacatataagtaaactgccatctttgagcataactacatttaaaaataaagctgcatatttttaaatcaagtgtttaacaagaatttatattttttattttttaaaattaaaaataatttatatttcctctgttgcatgaggattctcatctgtgcttataatggttagagattttatttgtgtggaatgaagtgaggcttgtagtcatggttctagtgtttcagtttgccaagtctgtttactgcagtgaaattcatcaaatgtttcagtgtggttttctgtagcctatcatttactggctatttttttatgtacacctttaggattttctgcctactctatccagttgtccaaatgatatcctacattttacaaatgccctttcagtttctattttctttttccattaaattgccctcatgtcctaatgtgcagtttgtaagtgtgtgtgtgtgtgtctgtgtgtgtgtgaatttgattttcaagagtgctagacttccaatttgagagattaaataatttaattcaggcaaacatttttcattggaatttcacagttcattgtaatgaaaatgttaatcctggatgacctttgacatacagtaatgaatcttggatattaatgaatttgttagtagcatcttgatgtgtgttttaatgagttattttcaaagttgtgcattaaaccaaagttggcatactggaagtgtttatatcaagttccatttggctactgatggacaaaaaatagaaatgccttcctatggagagtatttttcctttaaaaaattaaaaaggttaattattttgactaaaaaaaaaaaaaaaaaa

SEQ ID NO: 16 - DNA, 8718 bp, Homo sapiens; identical to SEQ ID NO: 15

SEQ ID NO: 17 - DNA, 8833 bp, Homo sapiens
cctcccctcgcccggcgcggtcccgtccgcctctcgctcgcctcccgcctcccctcggtcttccgaggcgcccgggctcccggcgcggcggcggagggggcgggcaggccggcgggcggtgatgtggcgggactctttatgcgctgcggcaggatacgcgctcggcgctgggacgcgactgcgctcagttctctcctctcggaagctgcagccatgatggaagtttgagagttgagccgctgtgaggcgaggccgggctcaggcgagggagatgagagacggcggcggccgcggcccggagcccctctcagcgcctgtgagcagccgcgggggcagcgccctcggggagccggccggcctgcggcggcggcagcggcggcgtttctcgcctcctcttcgtcttttctaaccgtgcagcctcttcctcggcttctcctgaaagggaaggtggaagccgtgggctcgggcgggagccggctgaggcgcggcggcggcggcggcacctcccgctcctggagcgggggggagaagcggcggcggcggcggccgcggcggctgcagctccagggagggggtctgagtcgcctgtcaccatttccagggctgggaacgccggagagttggtctctccccttctactgcctccaacacggcggcggcggcggcggcacatccagggacccgggccggttttaaacctcccgtccgccgccgccgcaccccccgtggcccgggctccggaggccgccggcggaggcagccgttcggaggattattcgtcttctccccattccgctgccgccgctgccaggcctctggctgctgaggagaagcaggcccagtcgctgcaaccatccagcagccgccgcagcagccattacccggctgcggtccagagccaagcggcggcagagcgaggggcatcagctaccgccaagtccagagccatttccatcctgcagaagaagccccgccaccagcagcttctgccatctctctcctcctttttcttcagccacaggctcccagacatgacagccatcatcaaagagatcgttagcagaaacaaaaggagatatcaagaggatggattcgacttagacttgacctatatttatccaaacattattgctatgggatttcctgcagaaagacttgaaggcgtatacaggaacaatattgatgatgtagtaagttgtgctgaaagacattatgacaccgccaaatttaattgcagagttgcacaatatccttttgaagaccataacccaccacagctagaacttatcaaacccttttgtgaagatcttgaccaatggctaagtgaagatgacaatcatgttgcagcaattcactgtaaagctggaaagggacgaactggtgtaatgatatgtgcatatttattacatcggggcaaatttttaaaggcacaagaggccctagatttctatggggaagtaaggaccagagacaaaaaggcagatcctacaggaggtattccagataaaggcattattgtcataggagatggcagctccatggatgttattgccccttaagaccttccagtgggacaagatgtataggtggaagacagtgatattgatgatcctgaccttgtagaggccaaggctaaaggagtaactattcccagtcagaggcgctatgtgtattattatagctacctgttaaagaatcatctggattatagaccagtggcactgttgtttcacaagatgatgtttgaaactattccaatgttcagtggcggaacttgcaatcctcagtttgtggtctgccagctaaaggtgaagatatattcctccaattcaggacccacacgacgggaagacaagttcatgtactttgagttccctcagccgttacctgtgtgtggtgatatcaaagtagagttcttccacaaacagaacaagatgctaaaaaaggacaaaatgtttcacttttgggtaaatacattcttcataccaggaccagaggaaacctcagaaaaagtagaaaatggaagtctatgtgatcaagaaatcgatagcatttgcagtatagagcgtgcagataatgacaaggaatatctagtacttactttaacaaaaaatgatcttgacaaagcaaataaagacaaagccaaccgatacttttctccaaattttaaggtgaagctgtacttcacaaaaacagtagaggagccgtcaaatccagaggctagcagttcaacttctgtaacaccagatgttagtgacaatgaacctgatcattatagatattctgacaccactgactctgatccagagaatgaaccttttgatgaagatcagcatacacaaattacaaaagtctgaatttttttttatcaagagggataaaacaccatgaaaataaacttgaataaactgaaaatggacctttttttttttaatggcaataggacattgtgtcagattaccagttataggaacaattctcttttcctgaccaatcttgttttaccctatacatccacagggttttgacacttgttgtccagttgaaaaaaggttgtgtagctgtgtcatgtatatacctttttgtgtcaaaaggacatttaaaattcaattaggattaataaagatggcactttcccgttttattccagttttataaaaagtggagacagactgatgtgtatacgtaggaattttttccttttgtgttctgtcaccaactgaagtggctaaagagctttgtgatatactggttcacatcctacccctttgcacttgtggcaacagataagtttgcagttggctaagagaggtttccgaagggttttgctacattctaatgcatgtattcgggttaggggaatggagggaatgctcagaaaggaaataattttatgctggactctggaccatataccatctccagctatttacacacacctttctttagcatgctacagttattaatctggacattcgaggaattggccgctgtcactgcttgttgtttgcgcatttttttttaaagcatattggtgctagaaaaggcagctaaaggaagtgaatctgtattggggtacaggaatgaaccttctgcaacatcttaagatccacaaatgaagggatataaaaataatgtcataggtaagaaacacagcaacaatgacttaaccatataaatgtggaggctatcaacaaagaatgggcttgaaacattataaaaattgacaatgatttattaaatatgttttctcaattgtaacgacttctccatctcctgtgtaatcaaggccagtgctaaaattcagatgctgttagtacctacatcagtcaacaacttacacttattttactagttttcaatcataatacctgctgtggatgcttcatgtgctgcctgcaagcttcttttttctcattaaatataaaatattttgtaatgctgcacagaaattttcaatttgagattctacagtaagcgttttttttctttgaagatttatgatgcacttattcaatagctgtcagccgttccacccttttgaccttacacattctattacaatgaattttgcagttttgcacattttttaaatgtcattaactgttagggaattttacttgaatactgaatacatataatgtttatattaaaaaggacatttgtgttaaaaaggaaattagagttgcagtaaactttcaatgctgcacacaaaaaaaagacatttgatttttcagtagaaattgtcctacatgtgctttattgatttgctattgaaagaatagggtttttttttttttttttttttttttttttaaatgtgcagtgttgaatcatttcttcatagtgctcccccgagttgggactagggcttcaatttcacttcttaaaaaaaatcatcatatatttgatatgcccagactgcatacgattttaagcggagtacaactactattgtaaagctaatgtgaagatattattaaaaaggtttttttttccagaaatttggtgtcttcaaattataccttcaccttgacatttgaatatccagccattttgtttcttaatggtataaaattccattttcaataacttattggtgctgaaattgttcactagctgtggtctgacctagttaatttacaaatacagattgaataggacctactagagcagcatttatagagtttgatggcaaatagattaggcagaacttcatctaaaatattcttagtaaataatgttgacacgttttccataccttgtcagtttcattcaacaatttttaaatttttaacaaagctcttaggatttacacatttatatttaaacattgatatatagagtattgattgattgctcataagttaaattggtaaagttagagacaactattctaacacctcaccattgaaatttatatgccaccttgtctttcataaaagctgaaaattgttacctaaaatgaaaatcaacttcatgttttgaagatagttataaatattgttctttgttacaatttcgggcaccgcatattaaaacgtaactttattgttccaatatgtaacatggagggccaggtcataaataatgacattataatgggcttttgcactgttattatttttcctttggaatgtgaaggtctgaatgagggttttgattttgaatgtttcaatgtttttgagaagccttgcttacattttatggtgtagtcattggaaatggaaaaatggcattatatatattatatatataaatatatattatacatactctccttactttatttcagttaccatccccatagaatttgacaagaattgctatgactgaaaggttttcgagtcctaattaaaactttatttatggcagtattcataattagcctgaaatgcattctgtaggtaatctctgagtttctggaatattttcttagactttttggatgtgcagcagcttacatgtctgaagttacttgaaggcatcacttttaagaaagcttacagttgggccctgtaccatcccaagtcctttgtagctcctcttgaacatgtttgccatacttttaaaagggtagttgaataaatagcatcaccattctttgctgtggcacaggttataaacttaagtggagtttaccggcagcatcaaatgtttcagctttaaaaaataaaagtagggtacaagtttaatgtttagttctagaaattttgtgcaatatgttcataacgatggctgtggttgccacaaagtgcctcgtttacctttaaatactgttaatgtgtcatgcatgcagatggaaggggtggaactgtgcactaaagtgggggctttaactgtagtatttggcagagttgccttctacctgccagttcaaaagttcaacctgttttcatatagaatatatatactaaaaaatttcagtctgttaaacagccttactctgattcagcctcttcagatactcttgtgctgtgcagcagtggctctgtgtgtaaatgctatgcactgaggatacacaaaaataccaatatgatgtgtacaggataatgcctcatcccaatcagatgtccatttgttattgtgtttgttaacaaccctttatctcttagtgttataaactccacttaaaactgattaaagtctcattcttgtcattgtgtgggtgttttattaaatgagagtttataattcaaattgcttaagtccattgaagttttaattaatgggcagccaaatgtgaatacaaagttttcagtttttttttttcctgctgtccttcaaagcctactgtttaaaaaaaaaaaaaaaaaaaaacatggcctgagagtagagtatctgtctactcatgtttaattaaggaaaaacacttatttttagggctttagtcatcacttcataaattgtataagcacattaaatagcgttctagtcctgaaaaagtccaagattcttagaaaattgtgcatatttttattatgacagatgtttgaagataattccccagaatggatttgatactttagatttcaattttgtggcttttgtctattattctgtactctgccatcagcatatggaaagcttcatttactcatcatgacttgtgccatataaaaattgatatttcggaatagtctaaaggactttttgtacttgaatttaatcatgttgtttctaatattcttaaaagcttgaagactaaagcatatcctttcaacaaagcatagtaaggtaataagaaagtgtagtttgtacaagtgttaaaaaaataaagtagacaatgttacagtgggacttattatttcaagtttacattttctccatgtaattttttaaaaagtaaatgaaaaaatgtgcaataatgtaaaatatgaagtgtatgtgtacacacattttatttttcggtatcttgggtatacgtatggttgaaaactatactggagtctaaaagtattctaatttataagaagacattttggtgatgtttgaaaaatagaaatgtgctagttttgtttttatatcatgtcctttgtacgttgtaatatgagctggcttggttcagtaaatgccatcaccatttccattgagaatttaaaactcaccagtgtttaatatgcaggcttccaaaggcttatgaaaaaaatcaagacccttaaatctagttaatttgctgctaacatgaaactctttggttcttttatttttgccagataattagacacacatctaaagcttagtcttaaatggcttaagtgtagctattgattagtgctgttgctagttcagaaagaaatgtttgtgaatggaaacaagaatattcagtccaaactgttgtaaggacagtacctgaaaaccaggaaacaggataatggaaaaagtcttttaaagatgaaatgttggagccaactttcttatagaattaattgtatgtggctatagaaagcctaatgattgttgcttatttttgagagcatattattcttttatgaccataatcttgctgtttttccatcttccaaaagatcttccttctaatatgtatatcagaatgtgggtagccagtcagacaaattcatattggttggtagctttaaaaagtttgtaatgtgaagacaggaaaggacaaaatagtttgctttggtggtagtactctggttgttaagctaggtattttgagactacttccccatcacaacaacaataaaataatcactcataatcctatcacctggagacatagccatcgttaatatgttagtgactatacaatcatgttttcttctgtatatccatgtatattctttaaaaatgaaatttatactgtacctgatctcaaagctttttagcttagtatatctgtcatgaatttgtaggatgttccattgcatcagaaaacggacagtgatttgattactttctaatgccacagatgcagattacatgtagttattgagaatcctttcgaattcagtggcttaatcatgaatgtctaaatattgttgacattaggatgatacatgtaaattaaagttacatttgtttagcatagacaagcttaacattgtagatgtttctcttcaaaaatcatcttaaacatttgcatttggaattgtgttaaatagaatgtgtgaaacactgtattagtaaacttcatcacctttctacttccttatagtttgaacttttcagtttttgtagttcccaaacagttgctcaatttagagcaaattaatttaacacctgccaaaaaaaggctgctgttggcttatcagttgtctttaaattcaaatgctcatgtgacttttatcacatcaaaaaatatttcattaatgattcacctttagctctgaaaattaccgcgtttagtaattatagtgggcttataaaaacatgcaactctttttgatagttatttgagaattttggtgaaaaatatttagctgagggcagtatagaacttataaaccaatatattgatatttttaaaacatttttacatataagtaaactgccatctttgagcataactacatttaaaaataaagctgcatatttttaaatcaagtgtttaacaagaatttatattttttattttttaaaattaaaaataatttatatttcctctgttgcatgaggattctcatctgtgcttataatggttagagattttatttgtgtggaatgaagtgaggcttgtagtcatggttctagtgtttcagtttgccaagtctgtttactgcagtgaaattcatcaaatgtttcagtgtggttttctgtagcctatcatttactggctatttttttatgtacacctttaggattttctgcctactctatccagttgtccaaatgatatcctacattttacaaatgccctttcagtttctattttctttttccattaaattgccctcatgtcctaatgtgcagtttgtaagtgtgtgtgtgtgtgtctgtgtgtgtgtgaatttgattttcaagagtgctagacttccaatttgagagattaaataatttaattcaggcaaacatttttcattggaatttcacagttcattgtaatgaaaatgttaatcctggatgacctttgacatacagtaatgaatcttggatattaatgaatttgttagtagcatcttgatgtgtgttttaatgagttattttcaaagttgtgcattaaaccaaagttggcatactggaagtgtttatatcaagttccatttggctactgatggacaaaaaatagaaatgccttcctatggagagtatttttcctttaaaaaattaaaaaggttaattattttgactaaaaaaaaaaaaaaaaaaa